European Patent Application EP 4 613 865 A1, published September 10, 2025. Title: Animal collagen from non-animal sources. Applicant: The Cultivated B. GmbH. Application EP. The sequence listing filed with the application follows.

SEQUENCE LISTING (34 sequences)

SEQ ID NO: 1 - protein, 1463 aa, Bos taurus
  PROPEP 1..161
  PROPEP 1217..1463
  PEPTIDE 162..1216
MFSFVDLRLLLLLAATALLTHGQEEGQEEGQEEDIPPVTCVQNGLRYHDRDVWKPVPCQICVCDNGNVLCDDVICDELKDCPNAKVPTDECCPVCPEGQESPTDQETTGVEGPKGDTGPRGPRGPAGPPGRDGIPGQPGLPGPPGPPGPPGPPGLGGNFAPQLSYGYDEKSTGISVPGPMGPSGPRGLPGPPGAPGPQGFQGPPGEPGEPGASGPMGPRGPPGPPGKNGDDGEAGKPGRPGERGPPGPQGARGLPGTAGLPGMKGHRGFSGLDGAKGDAGPAGPKGEPGSPGENGAPGQMGPRGLPGERGRPGAPGPAGARGNDGATGAAGPPGPTGPAGPPGFPGAVGAKGEGGPQGPRGSEGPQGVRGEPGPPGPAGAAGPAGNPGADGQPGAKGANGAPGIAGAPGFPGARGPSGPQGPSGPPGPKGNSGEPGAPGSKGDTGAKGEPGPTGIQGPPGPAGEEGKRGARGEPGPAGLPGPPGERGGPGSRGFPGADGVAGPKGPAGERGAPGPAGPKGSPGEAGRPGEAGLPGAKGLTGSPGSPGPDGKTGPPGPAGQDGRPGPPGPPGARGQAGVMGFPGPKGAAGEPGKAGERGVPGPPGAVGPAGKDGEAGAQGPPGPAGPAGERGEQGPAGSPGFQGLPGPAGPPGEAGKPGEQGVPGDLGAPGPSGARGERGFPGERGVQGPPGPAGPRGANGAPGNDGAKGDAGAPGAPGSQGAPGLQGMPGERGAAGLPGPKGDRGDAGPKGADGAPGKDGVRGLTGPIGPPGPAGAPGDKGEAGPSGPAGPTGARGAPGDRGEPGPPGPAGFAGPPGADGQPGAKGEPGDAGAKGDAGPPGPAGPAGPPGPIGNVGAPGPKGARGSAGPPGATGFPGAAGRVGPPGPSGNAGPPGPPGPAGKEGSKGPRGETGPAGRPGEVGPPGPPGPAGEKGAPGADGPAGAPGTPGPQGIAGQRGVVGLPGQRGERGFPGLPGPSGEPGKQGPSGASGERGPPGPMGPPGLAGPPGESGREGAPGAEGSPGRDGSPGAKGDRGETGPAGPPGAPGAPGAPGPVGPAGKSGDRGETGPAGPAGPIGPVGARGPAGPQGPRGDKGETGEQGDRGIKGHRGFSGLQGPPGPPGSPGEQGPSGASGPAGPRGPPGSAGSPGKDGLNGLPGPIGPPGPRGRTGDAGPAGPPGPPGPPGPPGPPSGGYDLSFLPQPPQEKAHDGGRYYRADDANVVRDRDLEVDTTLKSLSQQIENIRSPEGSRKNPARTCRDLKMCHSDWKSGEYWIDPNQGCNLDAIKVFCNMETGETCVYPTQPSVAQKNWYISKNPKEKRHVWYGESMTGGFQFEYGGQGSDPADVAIQLTFLRLMSTEASQNITYHCKNSVAYMDQQTGNLKKALLLQGSNEIEIRAEGNSRFTYSVTYDGCTSHTGAWGKTVIEYKTTKTSRLPIIDVAPLDVGAPDQEFGFDVGPACFL

SEQ ID NO: 2 - protein, 1056 aa, Bos taurus
QLSYGYDEKSTGISVPGPMGPSGPRGLPGPPGAPGPQGFQGPPGEPGEPGASGPMGPRGPPGPPGKNGDDGEAGKPGRPGERGPPGPQGARGLPGTAGLPGMKGHRGFSGLDGAKGDAGPAGPKGEPGSPGENGAPGQMGPRGLPGERGRPGAPGPAGARGNDGATGAAGPPGPTGPAGPPGFPGAVGAKGEGGPQGPRGSEGPQGVRGEPGPPGPAGAAGPAGNPGADGQPGAKGANGAPGIAGAPGFPGARGPSGPQGPSGPPGPKGNSGEPGAPGSKGDTGAKGEPGPTGIQGPPGPAGEEGKRGARGEPGPAGLPGPPGERGGPGSRGFPGADGVAGPKGPAGERGAPGPAGPKGSPGEAGRPGEAGLPGAKGLTGSPGSPGPDGKTGPPGPAGQDGRPGPPGPPGARGQAGVMGFPGPKGAAGEPGKAGERGVPGPPGAVGPAGKDGEAGAQGPPGPAGPAGERGEQGPAGSPGFQGLPGPAGPPGEAGKPGEQGVPGDLGAPGPSGARGERGFPGERGVQGPPGPAGPRGANGAPGNDGAKGDAGAPGAPGSQGAPGLQGMPGERGAAGLPGPKGDRGDAGPKGADGAPGKDGVRGLTGPIGPPGPAGAPGDKGEAGPSGPAGPTGARGAPGDRGEPGPPGPAGFAGPPGADGQPGAKGEPGDAGAKGDAGPPGPAGPAGPPGPIGNVGAPGPKGARGSAGPPGATGFPGAAGRVGPPGPSGNAGPPGPPGPAGKEGSKGPRGETGPAGRPGEVGPPGPPGPAGEKGAPGADGPAGAPGTPGPQGIAGQRGVVGLPGQRGERGFPGLPGPSGEPGKQGPSGASGERGPPGPMGPPGLAGPPGESGREGAPGAEGSPGRDGSPGAKGDRGETGPAGPPGAPGAPGAPGPVGPAGKSGDRGETGPAGPAGPIGPVGARGPAGPQGPRGDKGETGEQGDRGIKGHRGFSGLQGPPGPPGSPGEQGPSGASGPAGPRGPPGSAGSPGKDGLNGLPGPIGPPGPRGRTGDAGPAGPPGPPGPPGPPGPPSGGYDLSFLPQPPQEKAHDGGRYYRA

SEQ ID NO: 3 - DNA, 3176 bp, synthetic construct
  source 1..3176: mol_type = other DNA
  misc_feature 6..21: function = RBS with ATG from pET151
agggccaactgtcatatggctatgacgagaaaagcaccggtatatctgtcccggggccaatgggcccatcaggaccacgcggtttgccaggcccaccgggtgccccgggtcctcaaggattccaaggaccacccggtgaaccaggtgaaccgggtgcttctggcccgatgggtcctagaggtccgccggggcccccaggcaagaatggagatgatggtgaagcgggtaaaccaggcagacccggtgagagaggtcccccgggaccacagggcgctcgcggacttccaggtacagcgggattgcctggaatgaaagggcatcgtggcttttctggcttggatggagcaaaaggcgatgctgggccagcaggtccaaagggtgaaccaggaagtccaggagaaaatggtgctcctggtcaaatgggaccccgtgggttaccaggtgagcggggacgtccaggagctcccggccccgcaggtgctcgcggtaacgacggtgccaccggtgcggctggaccaccgggtcctacagggccggcagggccccctggatttcctggtgcagtaggtgcgaagggagaaggtggacctcaaggtccccgaggatcggaaggcccccaaggagtccgcggtgagccaggtccgccgggtcctgctggtgcagcagggccggctggtaatccaggtgcggatggacagcctggtgccaaaggtgcaaatggtgctccggggattgccggcgccccaggatttcccggtgctagaggtccatctggcccgcaaggtccttctggaccgccgggccctaaaggcaacagcggtgaaccaggggctcccggaagcaaaggagataccggagccaagggagaaccgggcccgaccgggattcagggcccaccgggtccagcaggcgaagaaggtaaacgcggtgcacgtggggaaccaggtcctgcaggcttaccgggtccccctggtgagagaggcggtccgggttcacgaggctttccaggagcggatggagtggcaggccctaaagggccggcgggagagcggggcgcccctggccccgcaggtccaaaagggtctccaggtgaagctgggcgtccgggtgaagcaggattgcctggtgcaaaggggttaactggcagtcctggtagtccgggaccggatggtaaaactggtccgccgggcccggcaggtcaagatggacgtccaggacccccgggaccccctggagctcgaggtcaagctggagtaatgggctttccgggtccgaagggagcagcgggcgaacccggaaaggcaggcgaacggggagttccaggtccacccggtgcagtaggcccagcagggaaagatggcgaggctggtgctcaagggccacctggtccagcaggcccggctggcgaacgtggagaacaaggaccggcgggaagccctggatttcagggattgcctggcccagcgggaccccctggagaggcgggtaaaccaggagaacaaggtgtaccaggagatcttggtgcacctggtcctagcggagctcgtggtgaaagaggttttccaggtgagcgcggtgttcaaggtcccccggggccagcaggacctcgtggagcaaatggtgcgccaggtaacgatggcgcaaaaggtgatgccggtgcaccaggtgcaccagggtcacagggtgctcccgggttacaaggaatgccaggtgagagaggtgccgcagggttacctgggccgaagggcgatagaggcgacgctggaccaaaaggtgccgatggagctccgggtaaggatggagtcagaggtttaacaggaccaataggacccccaggtcctgctggtgcccctggcgataaaggtgaggcaggtcctagtggtccagccggtcccacaggtgcacgcggagctccaggtgatcgcggcgaaccgggaccaccggggcctgctgggtttgcgggtccacctggtgccgatggacaacctggtgcgaagggcgaacccggtgatgcaggcgcgaagggcgatgcaggaccaccaggaccagctggcccggcaggtccgccgggtcctatcggaaacgtcggtgcgcccgggcctaaaggtgctagagggtctgcaggcccgccaggtgctactggtttccctggtgcagctggtcgtgtagggccaccaggcccttcaggaaatgctggtccgcctggaccacctgggccagcaggaaaagaggggagtaaaggaccacgtggtgagacaggtccggctggccggcctggtgaagtcggtccacctggtccgcccggacccgctggagagaaaggtgcaccgggtgcagacggtccggctggagcgcctggaactccaggccctcaaggaatcgccggccaaagaggcgtagttggtttaccgggtcagcgcggtgaacgtggttttcctggacttcctggtccttccggtgaaccgggtaagcaaggaccgtctggagcaagcggggaacgtggaccaccgggcccgatgggtccacctgggttagctggtccaccgggcgagtctggtagagaaggcgcacccggggcagaaggttcaccaggacgagacggctcaccaggggccaaaggtgatagaggcgaaacaggaccagcgggcccgccgggagcacctggtgcgccgggcgctccaggtccagttggaccggctggaaagtcaggcgatagaggggaaacgggcccggcgggaccagccggccctattggaccagtaggagctcgtgggccggcggggccacaaggccctcgtggagataaaggtgagaccggtgaacagggagatcgtgggattaagggtcatcgaggattttcagggcttcaaggaccgcctggtccaccgggctcgccaggtgagcagggtccctctggtgcttctggaccagctggtccacgtggcccgccaggcagtgcaggctcgccaggtaaagatggtcttaacgggttacctggcccaattgggccaccaggtcctcgtggtcgtacaggcgatgcaggtccagcaggtccgcctggaccgccaggaccgcctggtccccctggtcccccatcaggcggatatgacctttcatttctccctcagccaccgcaagaaaaggctcatgatggtggacgttattatcgcgcttaa

SEQ ID NO: 4 - DNA, 3171 bp, synthetic construct
  source 1..3171: mol_type = other DNA
cagctgtcttacgggtatgatgaaaaaagcaccggcatttcagttccgggcccgatgggcccgagcggtccccgtggcctgccgggcccgccgggcgcgccgggtccgcagggcttccaaggcccgccgggcgaaccgggtgaaccgggcgccagcggcccgatgggcccacgtggcccgccgggcccgccgggcaaaaatggcgatgatggagaagccggcaaaccgggccgtccgggtgaacgtggcccgccgggtccgcagggcgcgcgcggcctgccgggtaccgccggcctgccgggcatgaaaggtcatcgcggcttcagcggcctggatggcgccaaaggtgatgcgggtccggcgggcccgaaaggcgaaccgggcagtccgggcgaaaatggcgccccgggccagatgggtccgcgcggtctgccgggtgaacgtggccgcccgggcgcgccgggtccggcaggcgcgcgcggcaacgatggcgcgaccggcgccgccggcccgccgggcccgaccggcccggcgggcccgccgggatttccgggtgctgtgggcgcgaaaggcgaaggtggcccgcagggcccgcgtggtagcgaaggtccgcagggcgttcgcggcgaaccgggcccgccgggcccggcaggcgcggccggcccggcgggcaatccgggtgccgatggccagccgggggccaaaggcgccaatggtgcgccgggcatcgcgggtgcaccgggttttccgggcgcgcgcggcccgagcggcccgcagggcccgagcggtccgccgggcccgaagggcaacagcggcgaaccgggcgccccgggcagcaaaggcgataccggcgcgaaaggcgaacctggcccgaccggcattcagggcccgccgggcccggcaggcgaagaaggcaaacgtggcgcccgcggcgaaccgggcccggcgggtctgccgggcccgccgggcgaacgtggcggcccgggcagtcgcggctttccgggcgccgatggcgtggcaggcccgaaaggtccggcgggcgaacgtggcgccccgggcccggcgggcccgaaaggcagcccgggggaagcgggccgtccgggtgaagccggcctgccgggcgcgaaaggcctgaccggctcgccgggcagcccgggcccggatggcaaaaccggcccgccgggcccggcaggccaggacggccgtccgggcccgccgggcccgccgggcgcccgcggtcaggccggcgtcatgggctttccgggtccgaaaggcgcggcgggcgaaccgggtaaagcgggcgaacgtggcgtgccgggcccgccgggcgccgttggcccggcaggcaaagatggcgaagcgggcgcccagggtccgccgggcccggcgggcccggccggcgaacgcggcgaacagggcccggcgggcagcccgggttttcagggcctgccgggcccggcaggcccgccgggcgaagccggtaaaccgggcgaacagggcgtgcctggcgatctgggcgcgccgggcccgtcgggagcccgtggtgaacgcggcttcccgggtgaacgtggtgtgcagggcccgccgggccctgccggcccgcgtggcgcgaacggcgcgccgggcaacgatggcgcgaaaggcgacgccggcgccccgggtgcgccgggcagccagggcgcgccgggcctgcagggtatgccgggcgaacgtggcgcggcgggtctgccgggcccgaaaggcgatcgcggtgatgctggcccgaaaggcgcggatggcgcgccgggcaaggatggtgtgcgtggcctgaccggcccgattggcccgccgggcccggcaggcgccccgggcgataaaggagaagcgggcccgagcggcccggccggcccgaccggtgcccgtggtgcgccgggcgatcgtggcgaaccgggtccgccgggtccggccggcttcgcgggcccgccgggcgcggatggccagccgggcgcgaaaggcgaacctggcgatgccggtgcaaagggagacgcgggccctccgggcccggcgggcccggccggaccaccgggcccgattggcaatgttggcgcgccgggcccgaaaggcgcacgtggtagcgcgggccctccgggcgccaccggctttccgggcgcggccggccgtgtgggcccgccgggcccgagcggcaacgcgggaccgccgggcccgccgggcccggccggcaaagaaggcagcaaaggcccgcgtggcgaaactggcccggccggccgtccgggcgaagttggcccgccgggcccgccgggcccggccggtgaaaaaggtgccccgggtgccgacggcccggcgggcgcaccgggtaccccgggtccgcagggtattgcgggccagcgcggcgttgttggtctgccgggtcaacgtggcgaacgcggtttcccgggcctgccgggtccgagcggcgaaccgggtaaacagggccccagcggcgcctcgggcgaacgcggtccgccgggcccgatgggcccgccgggcctggcgggcccgccgggcgaaagtggccgcgaaggcgcgccgggtgcagaaggcagtccgggccgtgatggttcaccgggtgcgaaaggtgatcgcggcgagacaggtccggccggcccgccgggcgcgccgggcgccccgggcgcaccgggtccggtcggtccggcgggcaaatcaggagatcgcggcgaaaccggtccggcgggtccggcgggcccgattggtccggtgggcgcgcgtggcccggcaggcccgcagggtccgcgcggtgataaaggcgaaaccggcgagcagggcgatcgcggtattaaaggccatcgtggtttcagcggtctgcaaggcccgccgggcccgccgggctcgccgggcgaacagggcccgtcgggtgcgtccggccctgccggtccgcgcggcccgccgggcagcgccggcagcccgggcaaagatggtttaaacggcctgccgggcccgattggcccgccgggcccgcgcggccgcaccggcgatgccggcccggcaggcccgccgggcccgccgggcccgccgggtccgccgggcccgccgagcggcggctatgatctgagctttctgccgcagccgccgcaggaaaaagcgcatgatggtggccgctactatcgagcgtaa

SEQ ID NO: 5 - DNA, 3477 bp, synthetic construct
  source 1..3477: mol_type = other DNA
atgagatttccttcaatttttactgctgttttattcgcagcatcctccgcattagctgctccagtcaacactacaacagaagatgaaacggcacaaattccggctgaagctgtcatcggttactcagatttagaaggggatttcgatgttgctgttttgccattttccaacagcacaaataacgggttattgtttataaatactactattgccagcattgctgctaaagaagaaggggtatctctcgagaaaagagaggctgaagctcatcaccatcaccatcacgaaaacctgtattttcagggccaattgtcttatggttacgatgaaaagtccactggtatttctgtccctggaccaatgggtccatcaggtcctagaggtttgccaggtcctccaggtgctccaggtccacaaggttttcaaggtccaccaggtgaaccaggagaacccggtgcttctggtccaatgggtccaagaggtccacctggacctcctggtaagaacggtgatgatggtgaggctggtaagccaggaagacctggagaaagaggaccacctggtccacaaggagctagaggtttacccggtacagctggtttgcctggtatgaagggtcatagaggtttctccggtttggatggagctaagggtgatgctggacctgctggtcctaagggagagccaggatctccaggtgagaacggagctcctggacaaatgggaccaagaggtctgcctggtgaaagaggtagaccaggtgctcctggtcctgccggagccagaggtaatgatggtgctactggtgctgctggtcctccaggtccaactggtcctgctggtcctccaggttttccaggtgctgttggagccaaaggtgaaggtggcccacaaggtcctagaggatctgaaggtccacagggtgttagaggtgaaccaggtccaccaggtccagctggagctgctggtcctgctggtaacccaggtgcagatggtcaaccaggtgctaagggtgccaacggtgctccaggcattgctggagctccaggttttccaggagctagaggtccttctggacctcaaggaccatctggtccacctggaccaaaaggtaactctggagaaccaggtgctcctggttccaaaggtgataccggtgctaaaggagagccaggtcctactggtattcaaggtcctcctggtcctgctggtgaagagggtaaaagaggagccagaggtgaacctggtccagccggtttgccaggtccaccaggtgaaagaggaggtccaggatctagaggttttccaggtgctgacggtgttgctggtccaaagggtcctgctggtgagagaggagccccaggtccagctggacctaaaggatctccaggagaagctggtcgtcctggtgaagctggtcttccaggtgctaagggtttgacaggctccccaggatcccctggtccagatggtaagactggaccacctggaccagctggtcaagatggaagaccaggtcctccaggaccacctggagccagaggccaagctggtgttatgggtttccctggtccaaaaggtgctgctggagaaccgggtaaagccggtgaaagaggtgttccaggtcctccaggtgctgttggtcctgctggtaaagatggagaagccggtgctcaaggaccaccaggtccagctggtccagctggagagagaggtgaacaaggtcctgctggatccccaggtttccaaggtttgcctggtcctgctggaccaccaggtgaagctggtaagccaggtgaacaaggagttccaggtgatttgggtgctcctggtccatccggtgctagaggtgaaagaggatttccaggagagagaggtgttcaaggaccacctggtcctgctggaccaagaggagcaaacggtgctccaggaaacgatggtgctaaaggtgatgctggtgctccaggagctccaggttcacaaggtgctccaggtttgcaaggaatgcctggagaaagaggtgctgctggattaccaggtccaaaaggagacagaggtgatgccggtccaaagggtgctgatggtgctccaggtaaggacggtgtgcgaggtttgactggaccaattggacctccaggtccagctggagccccaggagataagggtgaagctggtccatcgggtcctgctggtcctactggtgctagaggagctccaggagatagaggtgaacctggtccacctggacccgctggatttgctggtccaccaggtgctgatggtcaaccaggggctaaaggtgaaccaggtgacgctggagctaaaggagatgccggtccaccaggtccagccggtccagctggtcctcctggtccaattggtaatgttggcgctcctggtcctaagggtgccagaggttcagctggaccaccaggtgctactggtttcccaggtgctgccggtagagttggtccaccaggtccatctggtaacgctggtcctccaggtccaccaggtcctgctggaaaggagggatctaagggaccaagaggtgaaactggtccagctggaagacctggtgaagttggtcctccaggaccaccaggtcctgctggagaaaaaggtgctccaggtgctgatggaccagctggtgctcctggtaccccaggtccacaaggtattgctggtcaaagaggtgtggttggtcttcctggacaaagaggtgagagaggttttcctggtttgccaggtccttctggagaacctggaaaacagggtccctctggtgcttctggtgagagaggtcctccaggaccaatgggacctccaggtttggctggtccaccaggtgagtctggtagagagggtgctccaggtgctgagggttctccaggtagagatggtagtccaggtgctaaaggagacagaggagagactggtccagctggtcctccaggtgctcctggtgctcccggtgctcctggtcctgtcggtcctgctggaaagtctggtgatagaggtgagactggtccagctggaccagctggtccaatcggaccagttggagctagaggtcctgctggtcctcaaggtccaagaggtgacaagggtgaaacaggtgagcaaggtgacagaggtattaaaggacatagaggtttctctggtctacagggacctcctggtcctccaggttccccaggtgagcaaggtccttctggtgcttcaggtcctgctggtccaagaggtccaccaggttctgctggttctccaggaaaggatggtttgaatggtttgcctggacctattggtcctcctggacctagaggtagaacaggtgatgctggtcctgctggtccacctggtcctcctggtcctcctggtccccctggacctccatctggaggttacgatttgtcttttttgccacaacctccacaggaaaaagcccatgacggtggaagatattatagagcttaa

SEQ ID NO: 6 - protein, 1158 aa, synthetic construct
  MOTIF 90..95: note = 6x His-Tag
  BINDING 96..101: note = TEV Protease Recognition site
MRFPSIFTAVLFAASSALAAPVNTTTEDETAQIPAEAVIGYSDLEGDFDVAVLPFSNSTNNGLLFINTTIASIAAKEEGVSLEKREAEAHHHHHHENLYFQGQLSYGYDEKSTGISVPGPMGPSGPRGLPGPPGAPGPQGFQGPPGEPGEPGASGPMGPRGPPGPPGKNGDDGEAGKPGRPGERGPPGPQGARGLPGTAGLPGMKGHRGFSGLDGAKGDAGPAGPKGEPGSPGENGAPGQMGPRGLPGERGRPGAPGPAGARGNDGATGAAGPPGPTGPAGPPGFPGAVGAKGEGGPQGPRGSEGPQGVRGEPGPPGPAGAAGPAGNPGADGQPGAKGANGAPGIAGAPGFPGARGPSGPQGPSGPPGPKGNSGEPGAPGSKGDTGAKGEPGPTGIQGPPGPAGEEGKRGARGEPGPAGLPGPPGERGGPGSRGFPGADGVAGPKGPAGERGAPGPAGPKGSPGEAGRPGEAGLPGAKGLTGSPGSPGPDGKTGPPGPAGQDGRPGPPGPPGARGQAGVMGFPGPKGAAGEPGKAGERGVPGPPGAVGPAGKDGEAGAQGPPGPAGPAGERGEQGPAGSPGFQGLPGPAGPPGEAGKPGEQGVPGDLGAPGPSGARGERGFPGERGVQGPPGPAGPRGANGAPGNDGAKGDAGAPGAPGSQGAPGLQGMPGERGAAGLPGPKGDRGDAGPKGADGAPGKDGVRGLTGPIGPPGPAGAPGDKGEAGPSGPAGPTGARGAPGDRGEPGPPGPAGFAGPPGADGQPGAKGEPGDAGAKGDAGPPGPAGPAGPPGPIGNVGAPGPKGARGSAGPPGATGFPGAAGRVGPPGPSGNAGPPGPPGPAGKEGSKGPRGETGPAGRPGEVGPPGPPGPAGEKGAPGADGPAGAPGTPGPQGIAGQRGVVGLPGQRGERGFPGLPGPSGEPGKQGPSGASGERGPPGPMGPPGLAGPPGESGREGAPGAEGSPGRDGSPGAKGDRGETGPAGPPGAPGAPGAPGPVGPAGKSGDRGETGPAGPAGPIGPVGARGPAGPQGPRGDKGETGEQGDRGIKGHRGFSGLQGPPGPPGSPGEQGPSGASGPAGPRGPPGSAGSPGKDGLNGLPGPIGPPGPRGRTGDAGPAGPPGPPGPPGPPGPPSGGYDLSFLPQPPQEKAHDGGRYYRA

SEQ ID NO: 7 - protein, 517 aa, Bos taurus
HPGFFTSIGQMTDLIHTEKDLVTSLKDYIKAEEDKLEQIKKWAEKLDRLTSTATKDPEGFVGHPVNAFKLMKRLNTEWSELENLVLKDMSDGFISNLTIQRQYFPNDEDQVGAAKALLRLQDTYNLDTDTISKGDLPGVKHKSFLTVEDCFELGKVAYTEADYYHTELWMEQALRQLDEGEVSTVDKVSVLDYLSYAVYQQGDLDKALLLTKKLLELDPEHQRANGNLKYFEYIMAKEKDANKSSSDDQSDQKTTLKKKGAAVDYLPERQKYEMLCRGEGIKMTPRRQKKLFCRYHDGNRNPKFILAPAKQEDEWDKPRIIRFHDIISDAEIEVVKDLAKPRLRRATISNPITGDLETVHYRISKSAWLSGYENPVVSRINMRIQDLTGLDVSTAEELQVANYGVGGQYEPHFDFARKDEPDAFKELGTGNRIATWLFYMSDVLAGGATVFPEVGASVWPKKGTAVFWYNLFASGEGDYSTRHAACPVLVGNKWVSNKWLHERGQEFRRPCTLSELE

SEQ ID NO: 8 - DNA, 1554 bp, Bos taurus
  source 1..1554: mol_type = other DNA
catcctggtttctttacttctattggacaaatgactgacttgatccataccgaaaaggatttggttacttccttgaaagattacattaaggctgaagaggataaattggaacagattaaaaaatgggctgaaaagttggatagattgacttccacagctactaaagatccagaaggtttcgttggtcatccagttaacgcttttaagttgatgaagagattgaacactgaatggtctgagttggaaaatttggtcctaaaggatatgtctgacggttttatctctaacttgactatccaaagacaatacttcccaaatgatgaagaccaagttggtgctgctaaagctcttttgagactgcaagacacctacaacttggataccgatacaatttctaagggtgatttgccaggtgttaagcacaagtcttttttaaccgttgaagattgtttcgagttgggaaaggttgcatatactgaggctgactactaccatactgaattgtggatggaacaggctttgagacaattagatgaaggtgaggtttctacagttgataaggtttctgttttggattacttgtcttatgcagtttaccagcaaggtgacttggataaagcattgttgttgactaagaagttgttggaattggaccctgagcatcaaagagcaaatggaaacttgaaatattttgagtacattatggctaaagaaaaagatgcaaacaagtcttcttctgatgatcaatccgaccaaaagacaactttgaagaagaagggtgctgctgttgattaccttccagaaagacagaagtacgagatgttatgtagaggtgaaggaattaagatgactccaagaagacagaaaaagttgttttgtagataccatgacggtaacagaaacccaaagtttattttggctcctgctaagcaggaggatgagtgggataagcctagaattatcagattccatgacattatctctgacgctgagatcgaggttgttaaggatttggctaagccaagattgagaagagctactatttctaatcctatcactggtgatttggagactgttcattatagaatttctaaatccgcttggttgtctggttatgaaaaccctgttgtgtctagaattaacatgagaattcaagacctcactggtttggatgtttctacagccgaagaattacaagtcgctaactacggtgttggtggacaatacgagccacatttcgactttgctcgtaaggatgaaccagacgcttttaaggaattaggtaccggtaacagaatcgctacatggcttttctacatgtctgatgttctggctggaggagctactgtttttccagaagttggtgcttctgtctggccaaagaaaggtaccgctgtgttttggtataatttgttcgcatctggtgaaggcgattactctaccagacatgctgcttgtccagtcttggtgggtaataagtgggtttccaacaaatggttgcatgaaagaggtcaggagttcagaaggccatgtaccttgtctgaattggaataa

SEQ ID NO: 9 - protein, 490 aa, Bos taurus
APDEEDHVLVLHKGNFDEALAAHKYLLVEFYAPWCGHCKALAPEYAKAAGKLKAEGSEIRLAKVDATEESDLAQQYGVRGYPTIKFFKNGDTASPKEYTAGREADDIVNWLKKRTGPAASTLSDGAAAEALVESSEVAVIGFFKDMESDSAKQFFLAAEVIDDIPFGITSNSDVFSKYQLDKDGVVLFKKFDEGRNNFEGEVTKEKLLDFIKHNQLPLVIEFTEQTAPKIFGGEIKTHILLFLPKSVSDYEGKLSNFKKAAESFKGKILFIFIDSDHTDNQRILEFFGLKKEECPAVRLITLEEEMTKYKPESDELTAEKITEFCHRFLEGKIKPHLMSQELPDDWDKQPVKVLVGKNFEEVAFDEKKNVFVEFYAPWCGHCKQLAPIWDKLGETYKDHENIVIAKMDSTANEVEAVKVHSFPTLKFFPASADRTVIDYNGERTLDGFKKFLESGGQDGAGDDDDLEDLEEAEEPDLEEDDDQKAVKDEL

SEQ ID NO: 10 - DNA, 13574 bp, synthetic construct
  source 1..13574: mol_type = other DNA
  regulatory 22..775: note = CaMV35S (enhanced); regulatory_class = promoter
  misc_feature 809..826: function = 6x His Tag
  misc_feature 833..850: function = TEV protease cleavage site
  CDS 857..5245: gene = Collagen alpha-1(I) chain; protein_id = 19; translation = MFSFVDLRLLLLLAATALLTHGQEEGQEEGQEEDIPPVTCVQNGLRYHDRDVWKPVPCQICVCDNGNVLCDDVICDELKDCPNAKVPTDECCPVCPEGQESPTDQETTGVEGPKGDTGPRGPRGPAGPPGRDGIPGQPGLPGPPGPPGPPGPPGLGGNFAPQLSYGYDEKSTGISVPGPMGPSGPRGLPGPPGAPGPQGFQGPPGEPGEPGASGPMGPRGPPGPPGKNGDDGEAGKPGRPGERGPPGPQGARGLPGTAGLPGMKGHRGFSGLDGAKGDAGPAGPKGEPGSPGENGAPGQMGPRGLPGERGRPGAPGPAGARGNDGATGAAGPPGPTGPAGPPGFPGAVGAKGEGGPQGPRGSEGPQGVRGEPGPPGPAGAAGPAGNPGADGQPGAKGANGAPGIAGAPGFPGARGPSGPQGPSGPPGPKGNSGEPGAPGSKGDTGAKGEPGPTGIQGPPGPAGEEGKRGARGEPGPAGLPGPPGERGGPGSRGFPGADGVAGPKGPAGERGAPGPAGPKGSPGEAGRPGEAGLPGAKGLTGSPGSPGPDGKTGPPGPAGQDGRPGPPGPPGARGQAGVMGFPGPKGAAGEPGKAGERGVPGPPGAVGPAGKDGEAGAQGPPGPAGPAGERGEQGPAGSPGFQGLPGPAGPPGEAGKPGEQGVPGDLGAPGPSGARGERGFPGERGVQGPPGPAGPRGANGAPGNDGAKGDAGAPGAPGSQGAPGLQGMPGERGAAGLPGPKGDRGDAGPKGADGAPGKDGVRGLTGPIGPPGPAGAPGDKGEAGPSGPAGPTGARGAPGDRGEPGPPGPAGFAGPPGADGQPGAKGEPGDAGAKGDAGPPGPAGPAGPPGPIGNVGAPGPKGARGSAGPPGATGFPGAAGRVGPPGPSGNAGPPGPPGPAGKEGSKGPRGETGPAGRPGEVGPPGPPGPAGEKGAPGADGPAGAPGTPGPQGIAGQRGVVGLPGQRGERGFPGLPGPSGEPGKQGPSGASGERGPPGPMGPPGLAGPPGESGREGAPGAEGSPGRDGSPGAKGDRGETGPAGPPGAPGAPGAPGPVGPAGKSGDRGETGPAGPAGPIGPVGARGPAGPQGPRGDKGETGEQGDRGIKGHRGFSGLQGPPGPPGSPGEQGPSGASGPAGPRGPPGSAGSPGKDGLNGLPGPIGPPGPRGRTGDAGPAGPPGPPGPPGPPGPPSGGYDLSFLPQPPQEKAHDGGRYYRADDANVVRDRDLEVDTTLKSLSQQIENIRSPEGSRKNPARTCRDLKMCHSDWKSGEYWIDPNQGCNLDAIKVFCNMETGETCVYPTQPSVAQKNWYISKNPKEKRHVWYGESMTGGFQFEYGGQGSDPADVAIQLTFLRLMSTEASQNITYHCKNSVAYMDQQTGNLKKALLLQGSNEIEIRAEGNSRFTYSVTYDGCTSHTGAWGKTVIEYKTTKTSRLPIIDVAPLDVGAPDQEFGFDVGPACFL
  misc_feature 857..922: function = Signal
  propeptide 923..1339
  misc_feature 1148..4507: note = Region of interest
  misc_feature 11860..11884: function = plasmid transfer to host cells; note = LB T_DNA repeat
  polyA_site 11975..12149: note = CaMV 35S pA
  misc_feature 12169..12720: function = Bar_plant resistance to tophophinothricin
  regulatory 12778..13531: note = CaMV35S (enhanced); regulatory_class = promoter
  misc_feature 5580..5604: function = plasmid transfer to host cells; note = RB T-DNA repeat
caactttgtatagaaaagttggccaacatggtggagcacgacactctcgtctactccaagaatatcaaagatacagtctcagaagaccaaagggctattgagacttttcaacaaagggtaatatcgggaaacctcctcggattccattgcccagctatctgtcacttcatcaaaaggacagtagaaaaggaaggtggcacctacaaatgccatcattgcgataaaggaaaggctatcgttcaagatgcctctgccgacagtggtcccaaagatggacccccacccacgaggagcatcgtggaaaaagaagacgttccaaccacgtcttcaaagcaagtggattgatgtgaacatggtggagcacgacactctcgtctactccaagaatatcaaagatacagtctcagaagaccaaagggctattgagacttttcaacaaagggtaatatcgggaaacctcctcggattccattgcccagctatctgtcacttcatcaaaaggacagtagaaaaggaaggtggcacctacaaatgccatcattgcgataaaggaaaggctatcgttcaagatgcctctgccgacagtggtcccaaagatggacccccacccacgaggagcatcgtggaaaaagaagacgttccaaccacgtcttcaaagcaagtggattgatgtgatatctccactgacgtaagggatgacgcacaatcccactatccttcgcaagacccttcctctatataaggaagttcatttcatttggagaggacacgctgacaagtttgtacaaaaaagcaggctgccaccatgcatcaccatcatcatcatggatctgagaatttatattttcaaggtagcatgttttctttcgttgatttgaggttgctccttcttttagcagctactgcattgcttactcatggtcaagaagagggtcaagaggaaggccaagaggaggatattccaccagtcacttgcgtgcaaaatggtcttaggtatcatgatagagatgtctggaaacctgttccatgtcaaatttgtgtgtgcgataatggaaacgtgctatgcgatgatgttatttgcgatgaattgaaagattgcccaaatgctaaggtgccaactgatgaatgttgtccagtttgcccagagggacaagaaagtccaacagatcaagaaactacaggtgttgaaggtccaaagggggatactggccctagaggtccacggggtccagctggaccaccaggaagagatggaattccaggtcaacctggacttccaggtccaccaggaccaccaggcccaccaggtcctcctggtttgggaggtaattttgcaccacaattgagttatggatacgacgaaaaatcaactggaatatcagtgccaggaccaatgggtccatcaggacctaggggtcttccagggccacctggcgctcctggtcctcagggatttcaaggtcctccaggtgaacctggagagcctggtgcttctggtccaatgggaccaagaggccctcctggtccacctggtaaaaatggtgatgatggtgaggctggaaagcctggtcgtcctggagaaagaggaccaccaggaccacagggagctagaggtttgccaggtacagccggtcttccaggaatgaaaggacacaggggtttttctggtcttgatggtgctaagggagacgcaggacctgctggaccaaagggtgaacctggatctcctggtgaaaatggtgctcctggacaaatgggacctagaggattgcctggcgaaagaggaagacctggtgctcctggaccagctggagctagaggaaatgatggagctactggtgctgccggaccaccaggaccaactggaccagctggaccacctggttttccaggagcagttggggctaagggagaaggtggaccacaaggacctagaggatcagaaggacctcaaggagttaggggagaaccaggtcctcctggtcctgctggagctgctggacccgctggtaacccaggagcagatggacaacctggagcaaaaggggctaatggtgctcctggtattgcaggtgctcctggattccctggtgctagaggaccttcaggacctcagggaccatccggtcctccaggaccaaagggaaactctggtgaaccaggggctcctggatctaagggagatactggagctaagggtgagccaggacctacaggaattcaaggaccaccaggacctgcaggagaggaaggtaagaggggtgctagaggtgaacctggaccagctggattgccaggcccacctggagagaggggtggtccaggttctagaggttttccaggagctgatggagttgctggtccaaagggtcctgctggtgagagaggtgcacctggaccagcaggacctaaaggatcacctggagaagctggtcgtcctggtgaggctggtcttccaggtgctaagggccttacaggatctccaggatcaccaggtccagatggaaagactggaccaccaggtcctgcaggacaagatggaaggcctggtccacctggaccacctggtgctaggggacaagctggtgttatgggattcccaggtccaaagggtgcagctggtgagcctggtaaagctggtgaaagaggagttccaggacctcctggtgctgttggacctgctggtaaagatggtgaagcaggtgctcagggtccaccaggtccagccggtccagctggtgagaggggagagcaaggtcctgctggatctcctggatttcaaggtttgcctggacctgctggacctccaggagaggctggtaaacctggtgagcagggtgtgcctggtgatcttggtgctcctggacctagtggcgcaagaggcgaaaggggatttccaggtgaaagaggagttcagggaccaccaggtccagctggtccaagaggcgctaatggagctccaggaaatgatggagcaaagggtgatgctggcgctccaggagctcctggttctcaaggtgcacctggattgcaaggaatgccaggagagagaggtgcagctggtttgccgggaccaaagggtgatagaggtgatgctggtcctaagggagctgatggagctccaggaaaggatggtgtgagaggattgactggtccaattggaccaccaggtcctgctggagcaccaggagataaaggagaagctggtccttcaggaccagccggtccaactggagctagaggagctccaggagatagaggtgaaccaggaccaccaggacctgctgggtttgcaggtccacctggtgctgatggacaacctggtgctaaaggagaaccaggcgatgctggtgctaagggagatgctggcccacctggtccagctggtcctgctgggccaccaggtcctatcggaaatgttggtgctccagggcctaaaggagctagaggatcagcaggtcccccaggtgctacaggttttccaggggctgctggaagagtgggtcccccaggtccttctgggaatgcaggaccaccaggtcctccaggaccagctggaaaagaaggaagtaagggaccaaggggagaaactggacctgcaggacgtccaggtgaagttggtccacctggacctccaggtccagctggagagaaaggagctccaggagctgatggtccagcaggtgctcctggtactccaggtccacaaggtattgctggtcaaaggggagtggttggtctcccaggtcagagaggtgaaagaggtttcccaggtttgcctggaccatctggagaaccaggtaagcagggcccatctggagcttctggtgagagagggccacctggacctatgggacctcctgggcttgctggacctccaggggaatctggtagggagggtgctccaggtgctgaaggatcacctggtagagatggatcacctggagctaaaggtgatagaggggaaacaggtccagcaggtccacctggcgctcctggtgctccaggagcaccagggccagttggacctgctggaaagtctggagataggggagagactggaccagctggacctgctggaccaatcggtcctgttggcgctagaggtcctgctggaccacaaggtcctaggggagataaaggtgaaacaggtgaacaaggagatagaggaattaaaggtcatagagggttttctggtttgcaaggacctccaggacctcctggatctccaggagagcaaggaccatctggtgcaagcggacctgctggtcctagaggacctccaggttcagctggctcacctggtaaggatggattaaatggtttgcctggaccaataggtccaccaggacctagaggaaggacaggtgatgcaggaccagctggtccacctggtccaccaggaccaccaggaccaccaggtccaccttctggtggatatgatcttagttttcttcctcaacctccccaggagaaagctcatgatggtggtagatattatagggctgatgatgcaaatgttgttagagatagagatcttgaggttgatactactcttaaatctcttagccaacaaattgaaaacattcgttctcctgagggaagcagaaaaaatcctgcaaggacttgtagagatcttaagatgtgccattcagattggaagtctggtgagtactggattgatccaaatcaaggttgtaatttggatgctatcaaagttttttgtaatatggaaactggagagacatgtgtgtaccctacacaaccttctgttgctcaaaaaaattggtatatttcaaaaaatcctaaagaaaagagacatgtttggtatggagaatctatgactggaggatttcaatttgagtatggtggacaaggatcagatccagctgatgtggctattcaacttacttttcttagattgatgtccactgaagcttctcaaaatattacatatcattgtaagaattctgttgcttatatggatcaacagactggaaatcttaagaaggcattgttgttgcaaggctcaaacgaaattgagattagggctgaaggtaatagtcgatttacttattctgttacatatgatggatgtacatctcacacaggtgcttggggaaaaacagttattgagtataaaactacaaaaactagtagacttccaattattgatgttgcaccattggatgttggtgctcctgatcaagaatttgggtttgatgttggacctgcttgtttccttgcatttgtttattaaacccagctttcttgtacaaagtggtagctcgaatttccccgatcgttcaaacatttggcaataaagtttcttaagattgaatcctgttgccggtcttgcgatgattatcatataatttctgttgaattacgttaagcatgtaataattaacatgtaatgcatgacgttatttatgagatgggtttttatgattagagtcccgcaattatacatttaatacgcgatagaaaacaaaatatagcgcgcaaactaggataaattatcgcgcgcggtgtcatctatgttactagatcgggaaagcttttaaactatcagtgtttgacaggatatattggcgggtaaacctaagagaaaagagcgtttattagaataatcggatatttaaaagggcgtgaaaaggtttatccgttcgtccatttgtatgtgcatgccaaccacagggttcccctcgggatcaaagtactttgatccaacccctccgctgctatagtgcagtcggcttctgacgttcagtgcagccgtcttctgaaaacgacatgtcgcacaagtcctaagttacgcgacaggctgccgccctgcccttttcctggcgttttcttgtcgcgtgttttagtcgcataaagtagaatacttgcgactagaaccggagacattacgccatgaacaagagcgccgccgctggcctgctgggctatgcccgcgtcagcaccgacgaccaggacttgaccaaccaacgggccgaactgcacgcggccggctgcaccaagctgttttccgagaagatcaccggcaccaggcgcgaccgcccggagctggccaggatgcttgaccacctacgccctggcgacgttgtgacagtgaccaggctagaccgcctggcccgcagcacccgcgacctactggacattgccgagcgcatccaggaggccggcgcgggcctgcgtagcctggcagagccgtgggccgacaccaccacgccggccggccgcatggtgttgaccgtgttcgccggcattgccgagttcgagcgttccctaatcatcgaccgcacccggagcgggcgcgaggccgccaaggcccgaggcgtgaagtttggcccccgccctaccctcaccccggcacagatcgcgcacgcccgcgagctgatcgaccaggaaggccgcaccgtgaaagaggcggctgcactgcttggcgtgcatcgctcgaccctgtaccgcgcacttgagcgcagcgaggaagtgacgcccaccgaggccaggcggcgcggtgccttccgtgaggacgcattgaccgaggccgacgccctggcggccgccgagaatgaacgccaagaggaacaagcatgaaaccgcaccaggacggccaggacgaaccgtttttcattaccgaagagatcgaggcggagatgatcgcggccgggtacgtgttcgagccgcccgcgcacgtctcaaccgtgcggctgcatgaaatcctggccggtttgtctgatgccaagctggcggcctggccggccagcttggccgctgaagaaaccgagcgccgccgtctaaaaaggtgatgtgtatttgagtaaaacagcttgcgtcatgcggtcgctgcgtatatgatgcgatgagtaaataaacaaatacgcaaggggaacgcatgaaggttatcgctgtacttaaccagaaaggcgggtcaggcaagacgaccatcgcaacccatctagcccgcgccctgcaactcgccggggccgatgttctgttagtcgattccgatccccagggcagtgcccgcgattgggcggccgtgcgggaagatcaaccgctaaccgttgtcggcatcgaccgcccgacgattgaccgcgacgtgaaggccatcggccggcgcgacttcgtagtgatcgacggagcgccccaggcggcggacttggctgtgtccgcgatcaaggcagccgacttcgtgctgattccggtgcagccaagcccttacgacatatgggccaccgccgacctggtggagctggttaagcagcgcattgaggtcacggatggaaggctacaagcggcctttgtcgtgtcgcgggcgatcaaaggcacgcgcatcggcggtgaggttgccgaggcgctggccgggtacgagctgcccattcttgagtcccgtatcacgcagcgcgtgagctacccaggcactgccgccgccggcacaaccgttcttgaatcagaacccgagggcgacgctgcccgcgaggtccaggcgctggccgctgaaattaaatcaaaactcatttgagttaatgaggtaaagagaaaatgagcaaaagcacaaacacgctaagtgccggccgtccgagcgcacgcagcagcaaggctgcaacgttggccagcctggcagacacgccagccatgaagcgggtcaactttcagttgccggcggaggatcacaccaagctgaagatgtacgcggtacgccaaggcaagaccattaccgagctgctatctgaatacatcgcgcagctaccagagtaaatgagcaaatgaataaatgagtagatgaattttagcggctaaaggaggcggcatggaaaatcaagaacaaccaggcaccgacgccgtggaatgccccatgtgtggaggaacgggcggttggccaggcgtaagcggctgggttgcctgccggccctgcaatggcactggaacccccaagcccgaggaatcggcgtgagcggtcgcaaaccatccggcccggtacaaatcggcgcggcgctgggtgatgacctggtggagaagttgaaggccgcgcaggccgcccagcggcaacgcatcgaggcagaagcacgccccggtgaatcgtggcaagcggccgctgatcgaatccgcaaagaatcccggcaaccgccggcagccggtgcgccgtcgattaggaagccgcccaagggcgacgagcaaccagattttttcgttccgatgctctatgacgtgggcacccgcgatagtcgcagcatcatggacgtggccgttttccgtctgtcgaagcgtgaccgacgagctggcgaggtgatccgctacgagcttccagacgggcacgtagaggtttccgcagggccggccggcatggccagtgtgtgggattacgacctggtactgatggcggtttcccatctaaccgaatccatgaaccgataccgggaagggaagggagacaagcccggccgcgtgttccgtccacacgttgcggacgtactcaagttctgccggcgagccgatggcggaaagcagaaagacgacctggtagaaacctgcattcggttaaacaccacgcacgttgccatgcagcgtacgaagaaggccaagaacggccgcctggtgacggtatccgagggtgaagccttgattagccgctacaagatcgtaaagagcgaaaccgggcggccggagtacatcgagatcgagctagctgattggatgtaccgcgagatcacagaaggcaagaacccggacgtgctgacggttcaccccgattactttttgatcgatcccggcatcggccgttttctctaccgcctggcacgccgcgccgcaggcaaggcagaagccagatggttgttcaagacgatctacgaacgcagtggcagcgccggagagttcaagaagttctgtttcaccgtgcgcaagctgatcgggtcaaatgacctgccggagtacgatttgaaggaggaggcggggcaggctggcccgatcctagtcatgcgctaccgcaacctgatcgagggcgaagcatccgccggttcctaatgtacggagcagatgctagggcaaattgccctagcaggggaaaaaggtcgaaaaggtctctttcctgtggatagcacgtacattgggaacccaaagccgtacattgggaaccggaacccgtacattgggaacccaaagccgtacattgggaaccggtcacacatgtaagtgactgatataaaagagaaaaaaggcgatttttccgcctaaaactctttaaaacttattaaaactcttaaaacccgcctggcctgtgcataactgtctggccagcgcacagccgaagagctgcaaaaagcgcctacccttcggtcgctgcgctccctacgccccgccgcttcgcgtcggcctatcgcggccgctggccgctcaaaaatggctggcctacggccaggcaatctaccagggcgcggacaagccgcgccgtcgccactcgaccgccggcgcccacatcaaggcaccctgcctcgcgcgtttcggtgatgacggtgaaaacctctgacacatgcagctcccggagacggtcacagcttgtctgtaagcggatgccgggagcagacaagcccgtcagggcgcgtcagcgggtgttggcgggtgtcggggcgcagccatgacccagtcacgtagcgatagcggagtgtatactggcttaactatgcggcatcagagcagattgtactgagagtgcaccatatgcggtgtgaaataccgcacagatgcgtaaggagaaaataccgcatcaggcgctcttccgcttcctcgctcactgactcgctgcgctcggtcgttcggctgcggcgagcggtatcagctcactcaaaggcggtaatacggttatccacagaatcaggggataacgcaggaaagaacatgtgagcaaaaggccagcaaaaggccaggaaccgtaaaaaggccgcgttgctggcgtttttccataggctccgcccccctgacgagcatcacaaaaatcgacgctcaagtcagaggtggcgaaacccgacaggactataaagataccaggcgtttccccctggaagctccctcgtgcgctctcctgttccgaccctgccgcttaccggatacctgtccgcctttctcccttcgggaagcgtggcgctttctcatagctcacgctgtaggtatctcagttcggtgtaggtcgttcgctccaagctgggctgtgtgcacgaaccccccgttcagcccgaccgctgcgccttatccggtaactatcgtcttgagtccaacccggtaagacacgacttatcgccactggcagcagccactggtaacaggattagcagagcgaggtatgtaggcggtgctacagagttcttgaagtggtggcctaactacggctacactagaaggacagtatttggtatctgcgctctgctgaagccagttaccttcggaaaaagagttggtagctcttgatccggcaaacaaaccaccgctggtagcggtggtttttttgtttgcaagcagcagattacgcgcagaaaaaaaggatctcaagaagatcctttgatcttttctacggggtctgacgctcagtggaacgaaaactcacgttaagggattttggtcatgcattctaggtactaaaacaattcatccagtaaaatataatattttattttctcccaatcaggcttgatccccagtaagtcaaaaaatagctcgacatactgttcttccccgatatcctccctgatcgaccggacgcagaaggcaatgtcataccacttgtccgccctgccgcttctcccaagatcaataaagccacttactttgccatctttcacaaagatgttgctgtctcccaggtcgccgtgggaaaagacaagttcctcttcgggcttttccgtctttaaaaaatcatacagctcgcgcggatctttaaatggagtgtcttcttcccagttttcgcaatccacatcggccagatcgttattcagtaagtaatccaattcggctaagcggctgtctaagctattcgtatagggacaatccgatatgtcgatggagtgaaagagcctgatgcactccgcatacagctcgataatcttttcagggctttgttcatcttcatactcttccgagcaaaggacgccatcggcctcactcatgagcagattgctccagccatcatgccgttcaaagtgcaggacctttggaacaggcagctttccttccagccatagcatcatgtccttttcccgttccacatcataggtggtccctttataccggctgtccgtcatttttaaatataggttttcattttctcccaccagcttatataccttagcaggagacattccttccgtatcttttacgcagcggtatttttcgatcagttttttcaattccggtgatattctcattttagccatttattatttccttcctcttttctacagtatttaaagataccccaagaagctaattataacaagacgaactccaattcactgttccttgcattctaaaaccttaaataccagaaaacagctttttcaaagttgttttcaaagttggcgtataacatagtatcgacggagccgattttgaaaccgcggtgatcacaggcagcaacgctctgtcatcgttacaatcaacatgctaccctccgcgagatcatccgtgtttcaaacccggcagcttagttgccgttcttccgaatagcatcggtaacatgagcaaagtctgccgccttacaacggctctcccgctgacgccgtcccggactgatgggctgcctgtatcgagtggtgattttgtgccgagctgccggtcggggagctgttggctggctggtggcaggatatattgtggtgtaaacaaattgacgcttagacaacttaataacacattgcggacgtttttaatgtactgaattaacgccgaattgaattcgagctcggtaccgggggatctggattttagtactggattttggttttaggaattagaaattttattgatagaagtattttacaaatacaaatacatactaagggtttcttatatgctcaacacatgagcgaaaccctataggaaccctaattcccttatctgggaactactcacacattattatggagaaactcgagcttgtcgatcgactcaaatctcggtgacgggcaggaccggacggggcggtaccggcaggctgaagtccagctgccagaaacccacgtcatgccagttcccgtgcttgaagccggccgcccgcagcatgccgcggggggcatatccgagcgcctcgtgcatgcgcacgctcgggtcgttgggcagcccgatgacagcgaccacgctcttgaagccctgtgcctccagggacttcagcaggtgggtgtagagcgtggagcccagtcccgtccgctggtggcggggggagacgtacacggtcgactcggccgtccagtcgtaggcgttgcgtgccttccaggggcccgcgtaggcgatgccggcgacctcgccgtccacctcggcgacgagccagggatagcgctcccgcagacggacgaggtcgtccgtccactcctgcggttcctgcggctcggtacggaagttgaccgtgcttgtctcgatgtagtggttgacgatggtgcagaccgccggcatgtccgcctcggtggcacggcggatgtcggccgggcgtcgttctgggctcatggtagacgatctgcgaaagctcgagagagatagatttgtagagagagactggtgatttcagcgtgtcctctccaaatgaaatgaacttccttatatagaggaagggtcttgcgaaggatagtgggattgtgcgtcatcccttacgtcagtggagatatcacatcaatccacttgctttgaagacgtggttggaacgtcttctttttccacgatgctcctcgtgggtgggggtccatctttgggaccactgtcggcagaggcatcttgaacgatagcctttcctttatcgcaatgatggcatttgtaggtgccaccttccttttctactgtccttttgatgaagtgacagatagctgggcaatggaatccgaggaggtttcccgatattaccctttgttgaaaagtctcaatagccctttggtcttctgagactgtatctttgatattcttggagtagacgagagtgtcgtgctccaccatgttcacatcaatccacttgctttgaagacgtggttggaacgtcttctttttccacgatgctcctcgtgggtgggggtccatctttgggaccactgtcggcagaggcatcttgaacgatagcctttcctttatcgcaatgatggcatttgtaggtgccaccttccttttctactgtccttttgatgaagtgacagatagctgggcaatggaatccgaggaggtttcccgatattaccctttgttgaaaagtctcaatagccctttggtcttctgagactgtatctttgatattcttggagtagacgagagtgtcgtgctccaccatgttggcgtacccggggatcctctagagtcgacctgcaggcatgcaagct

SEQ ID NO: 11 - DNA, 13523 bp, synthetic construct
  source 1..13523: mol_type = other DNA
  CDS 806..5209: note = bovine_Col1alpha1_AFVY; protein_id = 20; translation = MFSFVDLRLLLLLAATALLTHGQEEGQEEGQEEDIPPVTCVQNGLRYHDRDVWKPVPCQICVCDNGNVLCDDVICDELKDCPNAKVPTDECCPVCPEGQESPTDQETTGVEGPKGDTGPRGPRGPAGPPGRDGIPGQPGLPGPPGPPGPPGPPGLGGNFAPQLSYGYDEKSTGISVPGPMGPSGPRGLPGPPGAPGPQGFQGPPGEPGEPGASGPMGPRGPPGPPGKNGDDGEAGKPGRPGERGPPGPQGARGLPGTAGLPGMKGHRGFSGLDGAKGDAGPAGPKGEPGSPGENGAPGQMGPRGLPGERGRPGAPGPAGARGNDGATGAAGPPGPTGPAGPPGFPGAVGAKGEGGPQGPRGSEGPQGVRGEPGPPGPAGAAGPAGNPGADGQPGAKGANGAPGIAGAPGFPGARGPSGPQGPSGPPGPKGNSGEPGAPGSKGDTGAKGEPGPTGIQGPPGPAGEEGKRGARGEPGPAGLPGPPGERGGPGSRGFPGADGVAGPKGPAGERGAPGPAGPKGSPGEAGRPGEAGLPGAKGLTGSPGSPGPDGKTGPPGPAGQDGRPGPPGPPGARGQAGVMGFPGPKGAAGEPGKAGERGVPGPPGAVGPAGKDGEAGAQGPPGPAGPAGERGEQGPAGSPGFQGLPGPAGPPGEAGKPGEQGVPGDLGAPGPSGARGERGFPGERGVQGPPGPAGPRGANGAPGNDGAKGDAGAPGAPGSQGAPGLQGMPGERGAAGLPGPKGDRGDAGPKGADGAPGKDGVRGLTGPIGPPGPAGAPGDKGEAGPSGPAGPTGARGAPGDRGEPGPPGPAGFAGPPGADGQPGAKGEPGDAGAKGDAGPPGPAGPAGPPGPIGNVGAPGPKGARGSAGPPGATGFPGAAGRVGPPGPSGNAGPPGPPGPAGKEGSKGPRGETGPAGRPGEVGPPGPPGPAGEKGAPGADGPAGAPGTPGPQGIAGQRGVVGLPGQRGERGFPGLPGPSGEPGKQGPSGASGERGPPGPMGPPGLAGPPGESGREGAPGAEGSPGRDGSPGAKGDRGETGPAGPPGAPGAPGAPGPVGPAGKSGDRGETGPAGPAGPIGPVGARGPAGPQGPRGDKGETGEQGDRGIKGHRGFSGLQGPPGPPGSPGEQGPSGASGPAGPRGPPGSAGSPGKDGLNGLPGPIGPPGPRGRTGDAGPAGPPGPPGPPGPPGPPSGGYDLSFLPQPPQEKAHDGGRYYRADDANVVRDRDLEVDTTLKSLSQQIENIRSPEGSRKNPARTCRDLKMCHSDWKSGEYWIDPNQGCNLDAIKVFCNMETGETCVYPTQPSVAQKNWYISKNPKEKRHVWYGESMTGGFQFEYGGQGSDPADVAIQLTFLRLMSTEASQNITYHCKNSVAYMDQQTGNLKKALLLQGSNEIEIRAEGNSRFTYSVTYDGCTSHTGAWGKTVIEYKTTKTSRLPIIDVAPLDVGAPDQEFGFDVGPACFLAFVY
  sig_peptide 5195..5209: function = Vacuolar localisation signal; note = AFVY
  regulatory 5250..5503: note = Nos pA; regulatory_class = terminator
  misc_feature 5529..5553: function = plasmid transfer to host cells; note = RB T-DNA repeat
  misc_feature 11809..11833: function = plasmid transfer to host cells; note = LB T-DNA repeat
  polyA_site 11924..12098: note = CaMV 35S pA
  misc_feature 12118..12669: function = tophosphinothricin resistance; note = Bar
  regulatory 12727..13480: note = CaMV35S (enhanced) (1); regulatory_class = promoter
  regulatory 22..775: note = CaMV35S(enhanced); regulatory_class = promoter
caactttgtatagaaaagttggccaacatggtggagcacgacactctcgtctactccaagaatatcaaagatacagtctcagaagaccaaagggctattgagacttttcaacaaagggtaatatcgggaaacctcctcggattccattgcccagctatctgtcacttcatcaaaaggacagtagaaaaggaaggtggcacctacaaatgccatcattgcgataaaggaaaggctatcgttcaagatgcctctgccgacagtggtcccaaagatggacccccacccacgaggagcatcgtggaaaaagaagacgttccaaccacgtcttcaaagcaagtggattgatgtgaacatggtggagcacgacactctcgtctactccaagaatatcaaagatacagtctcagaagaccaaagggctattgagacttttcaacaaagggtaatatcgggaaacctcctcggattccattgcccagctatctgtcacttcatcaaaaggacagtagaaaaggaaggtggcacctacaaatgccatcattgcgataaaggaaaggctatcgttcaagatgcctctgccgacagtggtcccaaagatggacccccacccacgaggagcatcgtggaaaaagaagacgttccaaccacgtcttcaaagcaagtggattgatgtgatatctccactgacgtaagggatgacgcacaatcccactatccttcgcaagacccttcctctatataaggaagttcatttcatttggagaggacacgctgacaagtttgtacaaaaaagcaggctgccaccatgttttcttttgttgatcttagattgctccttcttcttgctgctacagcacttcttactcacgggcaagaagaaggtcaggaagaaggtcaagaagaagatattccaccagttacttgtgttcaaaacggtcttagataccatgatagggatgtttggaagcctgtgccatgtcaaatttgtgtttgtgataatggaaatgttttatgtgatgatgtaatttgtgatgaacttaaggattgccctaatgctaaggtaccaactgatgaatgttgtcctgtgtgtccagagggtcaagaatctcctacagatcaagaaactactggagttgaaggaccaaaaggtgatactggacccaggggccctaggggtccagcaggtcctccaggaagggatggaattcctggccagcctggtctaccaggaccaccgggaccacctggccctcctggtccacctggacttggaggtaattttgcacctcaactttcttacggatacgatgagaagtctacaggtatttctgttcctggacctatgggtccttcaggtccaagaggtcttccaggccctccaggagctccaggccctcaaggatttcaaggtcctcctggtgaaccaggagaaccaggagcatcaggaccaatgggacccagaggacctccaggtcctcctggaaaaaatggtgatgatggcgaggctggtaagccaggtagacctggtgaaagagggcctccaggtccacaaggtgctagaggactaccaggaacagctggtcttccaggaatgaagggtcataggggattttctggtttggatggagcaaaaggtgatgctggaccagctggtccaaaaggagaaccaggatctcctggagagaatggagctccaggacaaatgggacctagaggacttccaggtgaaagaggaagaccaggagcaccaggacctgctggtgctagaggaaatgatggggctactggtgctgctggaccacctggaccaacaggacctgcaggaccacctggttttccaggtgctgttggagctaagggagagggaggaccacaaggacctcgtggctcagaaggtccacaaggtgtcagaggtgagccaggtccacctggacctgctggagcagctggtcctgctggaaatcccggtgctgatggacagcctggagccaaaggagcaaacggagctcctggaattgctggtgcacctggtttccctggtgccagaggaccttcaggtcctcaggggccttctggtccaccaggtcctaaaggaaactctggagagcctggagctcctggttctaaaggagatacaggcgctaagggcgaacctggacctacaggaatccaaggacctcctggtccagcaggtgaggaagggaagagaggagctagaggagagcctggacctgctggtcttcctggcccaccaggagaaagaggaggtcctggatctagaggattcccaggagctgatggagttgccggacctaaaggacctgctggtgaaagaggagctccaggtccagcaggtcctaaaggatcaccaggagaagctggtaggccaggtgaagctggtttgccaggagctaaaggtcttacaggatctcctggctctccaggtcctgatgggaagactggaccaccaggtcctgctggacaagatggaaggccaggtcctccaggaccacctggagcaagaggtcaagctggtgtgatgggttttccaggaccaaagggagctgcaggagaaccaggtaaggctggagaaaggggagtacctggtcctcctggtgctgttggtccagctggtaaagatggagaagcaggagcacaaggtcctccaggtcctgcaggacctgctggagaaagaggtgaacaaggacctgcaggatcaccaggatttcaaggattgcctggccctgcaggacctccaggtgaagctggtaagccaggagagcaaggtgtcccaggtgatctcggggctcctggtccatcaggagcaagaggagagagaggatttccaggagaaagaggagttcagggaccaccaggaccagcaggaccaagaggtgctaacggcgcaccaggaaatgacggtgcaaagggggatgctggtgctccaggagctcctggatcacaaggagctccaggtttgcaaggcatgccaggagaaagaggagcagcaggattgcctggacctaagggtgatagaggcgatgcaggaccaaaaggagctgatggtgctccaggtaaggatggagttcgtggattgacaggtccaattggtccaccaggaccagctggagctcctggagataaaggcgaagctggaccatcaggaccagctggaccaactggtgctagaggagctcctggagacaggggagagcctggacctcctggtcctgctggtttcgctggacctcctggagcagatggacagccaggtgcaaagggagagccaggtgatgccggagctaaaggggatgctggtccacctggtccagcaggtccagctggtcctcctggccctataggtaatgttggtgctcctggtccaaaaggagctagagggtctgctggtcctccaggagctacaggttttcctggagcagctggaagagttggtcctccaggtccttcaggaaatgctggacctcctggtccaccaggacctgctggaaaggaaggatcaaaaggtccaagaggtgaaactggacctgctggtaggccaggagaagtgggtccaccaggaccaccaggacctgcaggagaaaagggtgctccaggagctgatggtcctgctggtgctccaggaacacctggaccacaaggaattgctggtcaaagaggtgttgtgggtcttccaggtcaaagaggtgaaagaggtttccctggacttcctggtccatcaggtgaacctggaaagcaaggtccaagtggagcttctggagaaagaggtcctccaggacctatgggtcctcctggtttggcaggtcctcctggagaatctggtagagaaggtgcacctggagcagaaggttctccaggtagggatggatctcctggagctaaaggagataggggtgaaacaggacctgcaggaccacctggagcacctggagctcctggtgctccaggaccagttggaccagcaggtaagtctggagatcgtggtgaaactggaccagctggaccagctggacctattggtcctgttggtgctaggggaccagcaggcccacaaggacctagaggtgataaaggagaaactggtgaacagggtgatagaggaataaaaggccatagagggttcagtggactccaaggacctcctggtccaccaggatctcctggagagcaaggaccttctggtgcttctggcccagctggtcctagaggacctccaggttctgcaggatctcctggtaaagatggattgaacggtcttccaggacctattggtcctcctggacctaggggaaggactggtgatgctggtccagctggaccaccaggtccacctggtcctccaggaccaccaggtccaccaagtggtggttatgatcttagctttcttcctcaacctcctcaagagaaggcccacgatggaggacgttattatagagctgatgatgctaacgttgttagagatagagatttggaagttgatactactttgaaatctctttcacaacaaattgaaaatattagatcacctgaaggatcaaggaagaaccctgctaggacttgtagagatcttaaaatgtgccatagcgattggaagtctggagagtattggattgatccaaatcaaggatgcaacttggatgctattaaagttttctgtaacatggagactggagaaacatgtgtttacccaactcaaccaagcgttgctcaaaaaaactggtacatctcaaaaaatccaaaagaaaagaggcatgtgtggtatggagaatctatgactggaggattccagtttgaatatggaggtcaaggttctgatcctgctgatgttgctattcaattgactttcttgagacttatgtctacagaggcatcacaaaacattacttatcattgcaagaactcagttgcttatatggatcaacaaactggaaatcttaaaaaggctcttctcttgcaaggatctaatgaaattgagataagagctgaaggaaactctagatttacttattctgttacatacgatggatgcacttcacatactggtgcatggggtaaaactgtaattgagtacaagactactaagacatctcgtcttcctattattgatgttgctccacttgatgttggtgctccagaccaagaatttggttttgatgtgggtcctgcatgttttcttgcttttgtttattaaacccagctttcttgtacaaagtggtagctcgaatttccccgatcgttcaaacatttggcaataaagtttcttaagattgaatcctgttgccggtcttgcgatgattatcatataatttctgttgaattacgttaagcatgtaataattaacatgtaatgcatgacgttatttatgagatgggtttttatgattagagtcccgcaattatacatttaatacgcgatagaaaacaaaatatagcgcgcaaactaggataaattatcgcgcgcggtgtcatctatgttactagatcgggaaagcttttaaactatcagtgtttgacaggatatattggcgggtaaacctaagagaaaagagcgtttattagaataatcggatatttaaaagggcgtgaaaaggtttatccgttcgtccatttgtatgtgcatgccaaccacagggttcccctcgggatcaaagtactttgatccaacccctccgctgctatagtgcagtcggcttctgacgttcagtgcagccgtcttctgaaaacgacatgtcgcacaagtcctaagttacgcgacaggctgccgccctgcccttttcctggcgttttcttgtcgcgtgttttagtcgcataaagtagaatacttgcgactagaaccggagacattacgccatgaacaagagcgccgccgctggcctgctgggctatgcccgcgtcagcaccgacgaccaggacttgaccaaccaacgggccgaactgcacgcggccggctgcaccaagctgttttccgagaagatcaccggcaccaggcgcgaccgcccggagctggccaggatgcttgaccacctacgccctggcgacgttgtgacagtgaccaggctagaccgcctggcccgcagcacccgcgacctactggacattgccgagcgcatccaggaggccggcgcgggcctgcgtagcctggcagagccgtgggccgacaccaccacgccggccggccgcatggtgttgaccgtgttcgccggcattgccgagttcgagcgttccctaatcatcgaccgcacccggagcgggcgcgaggccgccaaggcccgaggcgtgaagtttggcccccgccctaccctcaccccggcacagatcgcgcacgcccgcgagctgatcgaccaggaaggccgcaccgtgaaagaggcggctgcactgcttggcgtgcatcgctcgaccctgtaccgcgcacttgagcgcagcgaggaagtgacgcccaccgaggccaggcggcgcggtgccttccgtgaggacgcattgaccgaggccgacgccctggcggccgccgagaatgaacgccaagaggaacaagcatgaaaccgcaccaggacggccaggacgaaccgtttttcattaccgaagagatcgaggcggagatgatcgcggccgggtacgtgttcgagccgcccgcgcacgtctcaaccgtgcggctgcatgaaatcctggccggtttgtctgatgccaagctggcggcctggccggccagcttggccgctgaagaaaccgagcgccgccgtctaaaaaggtgatgtgtatttgagtaaaacagcttgcgtcatgcggtcgctgcgtatatgatgcgatgagtaaataaacaaatacgcaaggggaacgcatgaaggttatcgctgtacttaaccagaaaggcgggtcaggcaagacgaccatcgcaacccatctagcccgcgccctgcaactcgccggggccgatgttctgttagtcgattccgatccccagggcagtgcccgcgattgggcggccgtgcgggaagatcaaccgctaaccgttgtcggcatcgaccgcccgacgattgaccgcgacgtgaaggccatcggccggcgcgacttcgtagtgatcgacggagcgccccaggcggcggacttggctgtgtccgcgatcaaggcagccgacttcgtgctgattccggtgcagccaagcccttacgacatatgggccaccgccgacctggtggagctggttaagcagcgcattgaggtcacggatggaaggctacaagcggcctttgtcgtgtcgcgggcgatcaaaggcacgcgcatcggcggtgaggttgccgaggcgctggccgggtacgagctgcccattcttgagtcccgtatcacgcagcgcgtgagctacccaggcactgccgccgccggcacaaccgttcttgaatcagaacccgagggcgacgctgcccgcgaggtccaggcgctggccgctgaaattaaatcaaaactcatttgagttaatgaggtaaagagaaaatgagcaaaagcacaaacacgctaagtgccggccgtccgagcgcacgcagcagcaaggctgcaacgttggccagcctggcagacacgccagccatgaagcgggtcaactttcagttgccggcggaggatcacaccaagctgaagatgtacgcggtacgccaaggcaagaccattaccgagctgctatctgaatacatcgcgcagctaccagagtaaatgagcaaatgaataaatgagtagatgaattttagcggctaaaggaggcggcatggaaaatcaagaacaaccaggcaccgacgccgtggaatgccccatgtgtggaggaacgggcggttggccaggcgtaagcggctgggttgcctgccggccctgcaatggcactggaacccccaagcccgaggaatcggcgtgagcggtcgcaaaccatccggcccggtacaaatcggcgcggcgctgggtgatgacctggtggagaagttgaaggccgcgcaggccgcccagcggcaacgcatcgaggcagaagcacgccccggtgaatcgtggcaagcggccgctgatcgaatccgcaaagaatcccggcaaccgccggcagccggtgcgccgtcgattaggaagccgcccaagggcgacgagcaaccagattttttcgttccgatgctctatgacgtgggcacccgcgatagtcgcagcatcatggacgtggccgttttccgtctgtcgaagcgtgaccgacgagctggcgaggtgatccgctacgagcttccagacgggcacgtagaggtttccgcagggccggccggcatggccagtgtgtgggattacgacctggtactgatggcggtttcccatctaaccgaatccatgaaccgataccgggaagggaagggagacaagcccggccgcgtgttccgtccacacgttgcggacgtactcaagttctgccggcgagccgatggcggaaagcagaaagacgacctggtagaaacctgcattcggttaaacaccacgcacgttgccatgcagcgtacgaagaaggccaagaacggccgcctggtgacggtatccgagggtgaagccttgattagccgctacaagatcgtaaagagcgaaaccgggcggccggagtacatcgagatcgagctagctgattggatgtaccgcgagatcacagaaggcaagaacccggacgtgctgacggttcaccccgattactttttgatcgatcccggcatcggccgttttctctaccgcctggcacgccgcgccgcaggcaaggcagaagccagatggttgttcaagacgatctacgaacgcagtggcagcgccggagagttcaagaagttctgtttcaccgtgcgcaagctgatcgggtcaaatgacctgccggagtacgatttgaaggaggaggcggggcaggctggcccgatcctagtcatgcgctaccgcaacctgatcgagggcgaagcatccgccggttcctaatgtacggagcagatgctagggcaaattgccctagcaggggaaaaaggtcgaaaaggtctctttcctgtggatagcacgtacattgggaacccaaagccgtacattgggaaccggaacccgtacattgggaacccaaagccgtacattgggaaccggtcacacatgtaagtgactgatataaaagagaaaaaaggcgatttttccgcctaaaactctttaaaacttattaaaactcttaaaacccgcctggcctgtgcataactgtctggccagcgcacagccgaagagctgcaaaaagcgcctacccttcggtcgctgcgctccctacgccccgccgcttcgcgtcggcctatcgcggccgctggccgctcaaaaatggctggcctacggccaggcaatctaccagggcgcggacaagccgcgccgtcgccactcgaccgccggcgcccacatcaaggcaccctgcctcgcgcgtttcggtgatgacggtgaaaacctctgacacatgcagctcccggagacggtcacagcttgtctgtaagcggatgccgggagcagacaagcccgtcagggcgcgtcagcgggtgttggcgggtgtcggggcgcagccatgacccagtcacgtagcgatagcggagtgtatactggcttaactatgcggcatcagagcagattgtactgagagtgcaccatatgcggtgtgaaataccgcacagatgcgtaaggagaaaataccgcatcaggcgctcttccgcttcctcgctcactgactcgctgcgctcggtcgttcggctgcggcgagcggtatcagctcactcaaaggcggtaatacggttatccacagaatcaggggataacgcaggaaagaacatgtgagcaaaaggccagcaaaaggccaggaaccgtaaaaaggccgcgttgctggcgtttttccataggctccgcccccctgacgagcatcacaaaaatcgacgctcaagtcagaggtggcgaaacccgacaggactataaagataccaggcgtttccccctggaagctccctcgtgcgctctcctgttccgaccctgccgcttaccggatacctgtccgcctttctcccttcgggaagcgtggcgctttctcatagctcacgctgtaggtatctcagttcggtgtaggtcgttcgctccaagctgggctgtgtgcacgaaccccccgttcagcccgaccgctgcgccttatccggtaactatcgtcttgagtccaacccggtaagacacgacttatcgccactggcagcagccactggtaacaggattagcagagcgaggtatgtaggcggtgctacagagttcttgaagtggtggcctaactacggctacactagaaggacagtatttggtatctgcgctctgctgaagccagttaccttcggaaaaagagttggtagctcttgatccggcaaacaaaccaccgctggtagcggtggtttttttgtttgcaagcagcagattacgcgcagaaaaaaaggatctcaagaagatcctttgatcttttctacggggtctgacgctcagtggaacgaaaactcacgttaagggattttggtcatgcattctaggtactaaaacaattcatccagtaaaatataatattttattttctcccaatcaggcttgatccccagtaagtcaaaaaatagctcgacatactgttcttccccgatatcctccctgatcgaccggacgcagaaggcaatgtcataccacttgtccgccctgccgcttctcccaagatcaataaagccacttactttgccatctttcacaaagatgttgctgtctcccaggtcgccgtgggaaaagacaagttcctcttcgggcttttccgtctttaaaaaatcatacagctcgcgcggatctttaaatggagtgtcttcttcccagttttcgcaatccacatcggccagatcgttattcagtaagtaatccaattcggctaagcggctgtctaagctattcgtatagggacaatccgatatgtcgatggagtgaaagagcctgatgcactccgcatacagctcgataatcttttcagggctttgttcatcttcatactcttccgagcaaaggacgccatcggcctcactcatgagcagattgctccagccatcatgccgttcaaagtgcaggacctttggaacaggcagctttccttccagccatagcatcatgtccttttcccgttccacatcataggtggtccctttataccggctgtccgtcatttttaaatataggttttcattttctcccaccagcttatataccttagcaggagacattccttccgtatcttttacgcagcggtatttttcgatcagttttttcaattccggtgatattctcattttagccatttattatttccttcctcttttctacagtatttaaagataccccaagaagctaattataacaagacgaactccaattcactgttccttgcattctaaaaccttaaataccagaaaacagctttttcaaagttgttttcaaagttggcgtataacatagtatcgacggagccgattttgaaaccgcggtgatcacaggcagcaacgctctgtcatcgttacaatcaacatgctaccctccgcgagatcatccgtgtttcaaacccggcagcttagttgccgttcttccgaatagcatcggtaacatgagcaaagtctgccgccttacaacggctctcccgctgacgccgtcccggactgatgggctgcctgtatcgagtggtgattttgtgccgagctgccggtcggggagctgttggctggctggtggcaggatatattgtggtgtaaacaaattgacgcttagacaacttaataacacattgcggacgtttttaatgtactgaattaacgccgaattgaattcgagctcggtaccgggggatctggattttagtactggattttggttttaggaattagaaattttattgatagaagtattttacaaatacaaatacatactaagggtttcttatatgctcaacacatgagcgaaaccctataggaaccctaattcccttatctgggaactactcacacattattatggagaaactcgagcttgtcgatcgactcaaatctcggtgacgggcaggaccggacggggcggtaccggcaggctgaagtccagctgccagaaacccacgtcatgccagttcccgtgcttgaagccggccgcccgcagcatgccgcggggggcatatccgagcgcctcgtgcatgcgcacgctcgggtcgttgggcagcccgatgacagcgaccacgctcttgaagccctgtgcctccagggacttcagcaggtgggtgtagagcgtggagcccagtcccgtccgctggtggcggggggagacgtacacggtcgactcggccgtccagtcgtaggcgttgcgtgccttccaggggcccgcgtaggcgatgccggcgacctcgccgtccacctcggcgacgagccagggatagcgctcccgcagacggacgaggtcgtccgtccactcctgcggttcctgcggctcggtacggaagttgaccgtgcttgtctcgatgtagtggttgacgatggtgcagaccgccggcatgtccgcctcggtggcacggcggatgtcggccgggcgtcgttctgggctcatggtagacgatctgcgaaagctcgagagagatagatttgtagagagagactggtgatttcagcgtgtcctctccaaatgaaatgaacttccttatatagaggaagggtcttgcgaaggatagtgggattgtgcgtcatcccttacgtcagtggagatatcacatcaatccacttgctttgaagacgtggttggaacgtcttctttttccacgatgctcctcgtgggtgggggtccatctttgggaccactgtcggcagaggcatcttgaacgatagcctttcctttatcgcaatgatggcatttgtaggtgccaccttccttttctactgtccttttgatgaagtgacagatagctgggcaatggaatccgaggaggtttcccgatattaccctttgttgaaaagtctcaatagccctttggtcttctgagactgtatctttgatattcttggagtagacgagagtgtcgtgctccaccatgttcacatcaatccacttgctttgaagacgtggttggaacgtcttctttttccacgatgctcctcgtgggtgggggtccatctttgggaccactgtcggcagaggcatcttgaacgatagcctttcctttatcgcaatgatggcatttgtaggtgccaccttccttttctactgtccttttgatgaagtgacagatagctgggcaatggaatccgaggaggtttcccgatattaccctttgttgaaaagtctcaatagccctttggtcttctgagactgtatctttgatattcttggagtagacgagagtgtcgtgctccaccatgttggcgtacccggggatcctctagagtcgacctgcaggcatgcaagct

SEQ ID NO: 12 - DNA, 11446 bp, synthetic construct
  source 1..11446: mol_type = other DNA
  misc_feature 1..6795: note = pPD7-His-TEV-Col1a(triplehelicaldomain only)-tNos
  misc_feature 1..2057: note = 35S-His-TEV-Col1a(triplehelicaldomain only-tNos
  misc_feature 713..1507: function = Kanamycin Resitance
  gene 716..1507: note = alphA gene; note = Aminoglycoside 3'-phosphotransferase Protein
  misc_feature 1932..1956: function = plasmid transfer to host cells; note = LB T-DNA repeat
  misc_RNA 2040..2737: note = p19-Suppressor
  regulatory 2738..3083: note = p35S_short; regulatory_class = promoter
  regulatory 3088..3543: note = pPD7; regulatory_class = promoter
  misc_feature 3525..6775: note = 35S-His-TEV-Col1a(triplehelicaldomain only)-tNos
  CDS 3560..6775: gene = Col1a; protein_id = 13; translation = MHHHHHHGSENLYFQGQLSYGYDEKSTGISVPGPMGPSGPRGLPGPPGAPGPQGFQGPPGEPGEPGASGPMGPRGPPGPPGKNGDDGEAGKPGRPGERGPPGPQGARGLPGTAGLPGMKGHRGFSGLDGAKGDAGPAGPKGEPGSPGENGAPGQMGPRGLPGERGRPGAPGPAGARGNDGATGAAGPPGPTGPAGPPGFPGAVGAKGEGGPQGPRGSEGPQGVRGEPGPPGPAGAAGPAGNPGADGQPGAKGANGAPGIAGAPGFPGARGPSGPQGPSGPPGPKGNSGEPGAPGSKGDTGAKGEPGPTGIQGPPGPAGEEGKRGARGEPGPAGLPGPPGERGGPGSRGFPGADGVAGPKGPAGERGAPGPAGPKGSPGEAGRPGEAGLPGAKGLTGSPGSPGPDGKTGPPGPAGQDGRPGPPGPPGARGQAGVMGFPGPKGAAGEPGKAGERGVPGPPGAVGPAGKDGEAGAQGPPGPAGPAGERGEQGPAGSPGFQGLPGPAGPPGEAGKPGEQGVPGDLGAPGPSGARGERGFPGERGVQGPPGPAGPRGANGAPGNDGAKGDAGAPGAPGSQGAPGLQGMPGERGAAGLPGPKGDRGDAGPKGADGAPGKDGVRGLTGPIGPPGPAGAPGDKGEAGPSGPAGPTGARGAPGDRGEPGPPGPAGFAGPPGADGQPGAKGEPGDAGAKGDAGPPGPAGPAGPPGPIGNVGAPGPKGARGSAGPPGATGFPGAAGRVGPPGPSGNAGPPGPPGPAGKEGSKGPRGETGPAGRPGEVGPPGPPGPAGEKGAPGADGPAGAPGTPGPQGIAGQRGVVGLPGQRGERGFPGLPGPSGEPGKQGPSGASGERGPPGPMGPPGLAGPPGESGREGAPGAEGSPGRDGSPGAKGDRGETGPAGPPGAPGAPGAPGPVGPAGKSGDRGETGPAGPAGPIGPVGARGPAGPQGPRGDKGETGEQGDRGIKGHRGFSGLQGPPGPPGSPGEQGPSGASGPAGPRGPPGSAGSPGKDGLNGLPGPIGPPGPRGRTGDAGPAGPPGPPGPPGPPGPPSGGYDLSFLPQPPQEKAHDGGRYYRA
  CDS 3608..6775: gene = Collagen alpha-1(I) chain; protein_id = 14; translation = QLSYGYDEKSTGISVPGPMGPSGPRGLPGPPGAPGPQGFQGPPGEPGEPGASGPMGPRGPPGPPGKNGDDGEAGKPGRPGERGPPGPQGARGLPGTAGLPGMKGHRGFSGLDGAKGDAGPAGPKGEPGSPGENGAPGQMGPRGLPGERGRPGAPGPAGARGNDGATGAAGPPGPTGPAGPPGFPGAVGAKGEGGPQGPRGSEGPQGVRGEPGPPGPAGAAGPAGNPGADGQPGAKGANGAPGIAGAPGFPGARGPSGPQGPSGPPGPKGNSGEPGAPGSKGDTGAKGEPGPTGIQGPPGPAGEEGKRGARGEPGPAGLPGPPGERGGPGSRGFPGADGVAGPKGPAGERGAPGPAGPKGSPGEAGRPGEAGLPGAKGLTGSPGSPGPDGKTGPPGPAGQDGRPGPPGPPGARGQAGVMGFPGPKGAAGEPGKAGERGVPGPPGAVGPAGKDGEAGAQGPPGPAGPAGERGEQGPAGSPGFQGLPGPAGPPGEAGKPGEQGVPGDLGAPGPSGARGERGFPGERGVQGPPGPAGPRGANGAPGNDGAKGDAGAPGAPGSQGAPGLQGMPGERGAAGLPGPKGDRGDAGPKGADGAPGKDGVRGLTGPIGPPGPAGAPGDKGEAGPSGPAGPTGARGAPGDRGEPGPPGPAGFAGPPGADGQPGAKGEPGDAGAKGDAGPPGPAGPAGPPGPIGNVGAPGPKGARGSAGPPGATGFPGAAGRVGPPGPSGNAGPPGPPGPAGKEGSKGPRGETGPAGRPGEVGPPGPPGPAGEKGAPGADGPAGAPGTPGPQGIAGQRGVVGLPGQRGERGFPGLPGPSGEPGKQGPSGASGERGPPGPMGPPGLAGPPGESGREGAPGAEGSPGRDGSPGAKGDRGETGPAGPPGAPGAPGAPGPVGPAGKSGDRGETGPAGPAGPIGPVGARGPAGPQGPRGDKGETGEQGDRGIKGHRGFSGLQGPPGPPGSPGEQGPSGASGPAGPRGPPGSAGSPGKDGLNGLPGPIGPPGPRGRTGDAGPAGPPGPPGPPGPPGPPSGGYDLSFLPQPPQEKAHDGGRYYRA
  regulatory 6819..7074: note = NOS; regulatory_class = terminator
  polyA_site 6819..7072: note = Nos pA
  repeat_region 7098..7122: function = plasmid transfer to host cells; note = RB T-DNA repeat
aggccaggaaccgtaaaaaggccgcgttgctggcgtttttccataggctccgcccccctgacgagcatcacaaaaatcgacgctcaagtcagaggtggcgaaacccgacaggactataaagataccaggcgtttccccctggaagctccctcgtgcgctctcctgttccgaccctgccgcttaccggatacctgtccgcctttctcccttcgggaagcgtggcgctttctcatagctcacgctgtaggtatctcagttcggtgtaggtcgttcgctccaagctgggctgtgtgcacgaaccccccgttcagcccgaccgctgcgccttatccggtaactatcgtcttgagtccaacccggtaagacacgacttatcgccactggcagcagccactggtaacaggattagcagagcgaggtatgtaggcggtgctacagagttcttgaagtggtggcctaactacggctacactagaaggacagtatttggtatctgcgctctgctgaagccagttaccttcggaaaaagagttggtagctcttgatccggcaaacaaaccaccgctggtagcggtggtttttttgtttgcaagcagcagattacgcgcagaaaaaaaggatctcaagaagatcctttgatcttttctacggggtctgacgctcagtggaacgaaaactcacgttaagggattttggtcatgcattctaggtactaaaacaattcatccagtaaaatataatattttattttctcccaatcaggcttgatccccagtaagtcaaaaaatagctcgacatactgttcttccccgatatcctccctgatcgaccggacgcagaaggcaatgtcataccacttgtccgccctgccgcttctcccaagatcaataaagccacttactttgccatctttcacaaagatgttgctgtctcccaggtcgccgtgggaaaagacaagttcctcttcgggcttttccgtctttaaaaaatcatacagctcgcgcggatctttaaatggagtgtcttcttcccagttttcgcaatccacatcggccagatcgttattcagtaagtaatccaattcggctaagcggctgtctaagctattcgtatagggacaatccgatatgtcgatggagtgaaagagcctgatgcactccgcatacagctcgataatcttttcagggctttgttcatcttcatactcttccgagcaaaggacgccatcggcctcactcatgagcagattgctccagccatcatgccgttcaaagtgcaggacctttggaacaggcagctttccttccagccatagcatcatgtccttttcccgttccacatcataggtggtccctttataccggctgtccgtcatttttaaatataggttttcattttctcccaccagcttatataccttagcaggagacattccttccgtatcttttacgcagcggtatttttcgatcagttttttcaattccggtgatattctcattttagccatttattatttccttcctcttttctacagtatttaaagataccccaagaagctaattataacaagacgaactccaattcactgttccttgcattctaaaaccttaaataccagaaaacagctttttcaaagttgttttcaaagttggcgtataacatagtatcgacggagccgattttgaaaccgcggtgatcacaggcagcaacgctctgtcatcgttacaatcaacatgctaccctccgcgagatcatccgtgtttcaaacccggcagcttagttgccgttcttccgaatagcatcggtaacatgagcaaagtctgccgccttacaacggctctcccgctgacgccgtcccggactgatgggctgcctgtatcgagtggtgattttgtgccgagctgccggtcggggagctgttggctggctggtggcaggatatattgtggtgtaaacaaattgacgcttagacaacttaataacacattgcggacgtttttaatgtactgaattaacgccgaattgaattcgagctcggtggaggatctggattttagtactggattttggttttaggaattagaaattttattgatagaagtattttacaaatacaaatacatactaagggtttcttatatgctcaacacatgagcgaaaccctataggaaccctaattcccttatctgggaactactcacacattattatggagaaactattcactctccttctcaaacgtttctgttccctctggacagccccgactgacgttggactcaacctcaatgggcgctaattgtaatagctcctgtttgcttcttatggccatttcgcaaaggtgttgcagtgttctgctaccaccactcactgtaattgacacacctctgaaacggatggagtaagtgcaaccaatttgatcaaatccaaagaaacgactagcagcgtaatttactgagtcaccagtccaggaacctagaactcgatggagagaggcctctgtccgatcatagcgtaggtagcgtttgaaaactaccttgccaaatccccaggactctttaaatcccagtgggttgtcctggttggagtttgtttcgtcattgtgtaaacgccattctgtccaagatgggctctcatcgggtaacttaaatgggctggtagtgccgccagaaccaccgtcccatctctctgaattggcctgctctcttgcatcattaccctggattgctctctccattgtcctctccaaatgaaatgaacttccttatatagaggaagggtcttgcgaaggatagtgggattgtgcgtcatcccttacgtcagtggagatgtcacatcaatccacttgctttgtagacgtggttggaacctcttctttttccacgatgctcctcgtgggtgggggtccatctttgggaccactgtcggcagagagatcttgaatgatagcctttcctttatcgcaatgatggcatttgtaggagccaccttccttttctactgtcctttcgatgaagtgacagatagctgggcaatggaatccgaggaggtttcccgaaattatcctttgttgaaaagtctcaaacaataggcaaccgtggacttcttcactagctcatcgagatagcaatgccactagctaatttcttacgttgtatcttatttgttttactttggggcatgacatggttaaaccccatcaaagagaaagtgtttcatccactagtcaatatacgaattcattcgaatttatccctgtaaatcctagttcttaggatgaactggtgtaataaacagcaaaaaaaaataaaaaaaaataaatctggaatcattcgaccacctcaataaactaaagctaccaattaccacaatatagtcatccatatccacttagatataaaagataaaagtaaacaaatattaaatttcatatgcacgcataggaaactcatgatcttatcttttaaatagacatctagttttcttaggttataaatagacattttgtcctagaacttcttcactactaaaacctagcctcaaaaagcaggctgccaccatgcatcaccatcatcatcatggatctgagaatttatattttcaaggtcaattgagttatggatacgacgaaaaatcaactggaatatcagtgccaggaccaatgggtccatcaggacctaggggtcttccagggccacctggcgctcctggtcctcagggatttcaaggtcctccaggtgaacctggagagcctggtgcttctggtccaatgggaccaagaggccctcctggtccacctggtaaaaatggtgatgatggtgaggctggaaagcctggtcgtcctggagaaagaggaccaccaggaccacagggagctagaggtttgccaggtacagccggtcttccaggaatgaaaggacacaggggtttttctggtcttgatggtgctaagggagacgcaggacctgctggaccaaagggtgaacctggatctcctggtgaaaatggtgctcctggacaaatgggacctagaggattgcctggcgaaagaggaagacctggtgctcctggaccagctggagctagaggaaatgatggagctactggtgctgccggaccaccaggaccaactggaccagctggaccacctggttttccaggagcagttggggctaagggagaaggtggaccacaaggacctagaggatcagaaggacctcaaggagttaggggagaaccaggtcctcctggtcctgctggagctgctggacccgctggtaacccaggagcagatggacaacctggagcaaaaggggctaatggtgctcctggtattgcaggtgctcctggattccctggtgctagaggaccttcaggacctcagggaccatccggtcctccaggaccaaagggaaactctggtgaaccaggggctcctggatctaagggagatactggagctaagggtgagccaggacctacaggaattcaaggaccaccaggacctgcaggagaggaaggtaagaggggtgctagaggtgaacctggaccagctggattgccaggcccacctggagagaggggtggtccaggttctagaggttttccaggagctgatggagttgctggtccaaagggtcctgctggtgagagaggtgcacctggaccagcaggacctaaaggatcacctggagaagctggtcgtcctggtgaggctggtcttccaggtgctaagggccttacaggatctccaggatcaccaggtccagatggaaagactggaccaccaggtcctgcaggacaagatggaaggcctggtccacctggaccacctggtgctaggggacaagctggtgttatgggattcccaggtccaaagggtgcagctggtgagcctggtaaagctggtgaaagaggagttccaggacctcctggtgctgttggacctgctggtaaagatggtgaagcaggtgctcagggtccaccaggtccagccggtccagctggtgagaggggagagcaaggtcctgctggatctcctggatttcaaggtttgcctggacctgctggacctccaggagaggctggtaaacctggtgagcagggtgtgcctggtgatcttggtgctcctggacctagtggcgcaagaggcgaaaggggatttccaggtgaaagaggagttcagggaccaccaggtccagctggtccaagaggcgctaatggagctccaggaaatgatggagcaaagggtgatgctggcgctccaggagctcctggttctcaaggtgcacctggattgcaaggaatgccaggagagagaggtgcagctggtttgccgggaccaaagggtgatagaggtgatgctggtcctaagggagctgatggagctccaggaaaggatggtgtgagaggattgactggtccaattggaccaccaggtcctgctggagcaccaggagataaaggagaagctggtccttcaggaccagccggtccaactggagctagaggagctccaggagatagaggtgaaccaggaccaccaggacctgctgggtttgcaggtccacctggtgctgatggacaacctggtgctaaaggagaaccaggcgatgctggtgctaagggagatgctggcccacctggtccagctggtcctgctgggccaccaggtcctatcggaaatgttggtgctccagggcctaaaggagctagaggatcagcaggtcccccaggtgctacaggttttccaggggctgctggaagagtgggtcccccaggtccttctgggaatgcaggaccaccaggtcctccaggaccagctggaaaagaaggaagtaagggaccaaggggagaaactggacctgcaggacgtccaggtgaagttggtccacctggacctccaggtccagctggagagaaaggagctccaggagctgatggtccagcaggtgctcctggtactccaggtccacaaggtattgctggtcaaaggggagtggttggtctcccaggtcagagaggtgaaagaggtttcccaggtttgcctggaccatctggagaaccaggtaagcagggcccatctggagcttctggtgagagagggccacctggacctatgggacctcctgggcttgctggacctccaggggaatctggtagggagggtgctccaggtgctgaaggatcacctggtagagatggatcacctggagctaaaggtgatagaggggaaacaggtccagcaggtccacctggcgctcctggtgctccaggagcaccagggccagttggacctgctggaaagtctggagataggggagagactggaccagctggacctgctggaccaatcggtcctgttggcgctagaggtcctgctggaccacaaggtcctaggggagataaaggtgaaacaggtgaacaaggagatagaggaattaaaggtcatagagggttttctggtttgcaaggacctccaggacctcctggatctccaggagagcaaggaccatctggtgcaagcggacctgctggtcctagaggacctccaggttcagctggctcacctggtaaggatggattaaatggtttgcctggaccaataggtccaccaggacctagaggaaggacaggtgatgcaggaccagctggtccacctggtccaccaggaccaccaggaccaccaggtccaccttctggtggatatgatcttagttttcttcctcaacctccccaggagaaagctcatgatggtggtagatattatagggcttaaacccagctttcttgtacaaagtggtagctcgaatttccccgatcgttcaaacatttggcaataaagtttcttaagattgaatcctgttgccggtcttgcgatgattatcatataatttctgttgaattacgttaagcatgtaataattaacatgtaatgcatgacgttatttatgagatgggtttttatgattagagtcccgcaattatacatttaatacgcgatagaaaacaaaatatagcgcgcaaactaggataaattatcgcgcgcggtgtcatctatgttactagatcgggaaagcttttaaactatcagtgtttgacaggatatattggcgggtaaacctaagagaaaagagcgtttattagaataatcggatatttaaaagggcgtgaaaaggtttatccgttcgtccatttgtatgtgcatgccaaccacagggttcccctcgggatcaaagtactttgatccaacccctccgctgctatagtgcagtcggcttctgacgttcagtgcagccgtcttctgaaaacgacatgtcgcacaagtcctaagttacgcgacaggctgccgccctgcccttttcctggcgttttcttgtcgcgtgttttagtcgcataaagtagaatacttgcgactagaaccggagacattacgccatgaacaagagcgccgccgctggcctgctgggctatgcccgcgtcagcaccgacgaccaggacttgaccaaccaacgggccgaactgcacgcggccggctgcaccaagctgttttccgagaagatcaccggcaccaggcgcgaccgcccggagctggccaggatgcttgaccacctacgccctggcgacgttgtgacagtgaccaggctagaccgcctggcccgcagcacccgcgacctactggacattgccgagcgcatccaggaggccggcgcgggcctgcgtagcctggcagagccgtgggccgacaccaccacgccggccggccgcatggtgttgaccgtgttcgccggcattgccgagttcgagcgttccctaatcatcgaccgcacccggagcgggcgcgaggccgccaaggcccgaggcgtgaagtttggcccccgccctaccctcaccccggcacagatcgcgcacgcccgcgagctgatcgaccaggaaggccgcaccgtgaaagaggcggctgcactgcttggcgtgcatcgctcgaccctgtaccgcgcacttgagcgcagcgaggaagtgacgcccaccgaggccaggcggcgcggtgccttccgtgaggacgcattgaccgaggccgacgccctggcggccgccgagaatgaacgccaagaggaacaagcatgaaaccgcaccaggacggccaggacgaaccgtttttcattaccgaagagatcgaggcggagatgatcgcggccgggtacgtgttcgagccgcccgcgcacgtctcaaccgtgcggctgcatgaaatcctggccggtttgtctgatgccaagctggcggcctggccggccagcttggccgctgaagaaaccgagcgccgccgtctaaaaaggtgatgtgtatttgagtaaaacagcttgcgtcatgcggtcgctgcgtatatgatgcgatgagtaaataaacaaatacgcaaggggaacgcatgaaggttatcgctgtacttaaccagaaaggcgggtcaggcaagacgaccatcgcaacccatctagcccgcgccctgcaactcgccggggccgatgttctgttagtcgattccgatccccagggcagtgcccgcgattgggcggccgtgcgggaagatcaaccgctaaccgttgtcggcatcgaccgcccgacgattgaccgcgacgtgaaggccatcggccggcgcgacttcgtagtgatcgacggagcgccccaggcggcggacttggctgtgtccgcgatcaaggcagccgacttcgtgctgattccggtgcagccaagcccttacgacatatgggccaccgccgacctggtggagctggttaagcagcgcattgaggtcacggatggaaggctacaagcggcctttgtcgtgtcgcgggcgatcaaaggcacgcgcatcggcggtgaggttgccgaggcgctggccgggtacgagctgcccattcttgagtcccgtatcacgcagcgcgtgagctacccaggcactgccgccgccggcacaaccgttcttgaatcagaacccgagggcgacgctgcccgcgaggtccaggcgctggccgctgaaattaaatcaaaactcatttgagttaatgaggtaaagagaaaatgagcaaaagcacaaacacgctaagtgccggccgtccgagcgcacgcagcagcaaggctgcaacgttggccagcctggcagacacgccagccatgaagcgggtcaactttcagttgccggcggaggatcacaccaagctgaagatgtacgcggtacgccaaggcaagaccattaccgagctgctatctgaatacatcgcgcagctaccagagtaaatgagcaaatgaataaatgagtagatgaattttagcggctaaaggaggcggcatggaaaatcaagaacaaccaggcaccgacgccgtggaatgccccatgtgtggaggaacgggcggttggccaggcgtaagcggctgggttgcctgccggccctgcaatggcactggaacccccaagcccgaggaatcggcgtgagcggtcgcaaaccatccggcccggtacaaatcggcgcggcgctgggtgatgacctggtggagaagttgaaggccgcgcaggccgcccagcggcaacgcatcgaggcagaagcacgccccggtgaatcgtggcaagcggccgctgatcgaatccgcaaagaatcccggcaaccgccggcagccggtgcgccgtcgattaggaagccgcccaagggcgacgagcaaccagattttttcgttccgatgctctatgacgtgggcacccgcgatagtcgcagcatcatggacgtggccgttttccgtctgtcgaagcgtgaccgacgagctggcgaggtgatccgctacgagcttccagacgggcacgtagaggtttccgcagggccggccggcatggccagtgtgtgggattacgacctggtactgatggcggtttcccatctaaccgaatccatgaaccgataccgggaagggaagggagacaagcccggccgcgtgttccgtccacacgttgcggacgtactcaagttctgccggcgagccgatggcggaaagcagaaagacgacctggtagaaacctgcattcggttaaacaccacgcacgttgccatgcagcgtacgaagaaggccaagaacggccgcctggtgacggtatccgagggtgaagccttgattagccgctacaagatcgtaaagagcgaaaccgggcggccggagtacatcgagatcgagctagctgattggatgtaccgcgagatcacagaaggcaagaacccggacgtgctgacggttcaccccgattactttttgatcgatcccggcatcggccgttttctctaccgcctggcacgccgcgccgcaggcaaggcagaagccagatggttgttcaagacgatctacgaacgcagtggcagcgccggagagttcaagaagttctgtttcaccgtgcgcaagctgatcgggtcaaatgacctgccggagtacgatttgaaggaggaggcggggcaggctggcccgatcctagtcatgcgctaccgcaacctgatcgagggcgaagcatccgccggttcctaatgtacggagcagatgctagggcaaattgccctagcaggggaaaaaggtcgaaaaggtctctttcctgtggatagcacgtacattgggaacccaaagccgtacattgggaaccggaacccgtacattgggaacccaaagccgtacattgggaaccggtcacacatgtaagtgactgatataaaagagaaaaaaggcgatttttccgcctaaaactctttaaaacttattaaaactcttaaaacccgcctggcctgtgcataactgtctggccagcgcacagccgaagagctgcaaaaagcgcctacccttcggtcgctgcgctccctacgccccgccgcttcgcgtcggcctatcgcggccgctggccgctcaaaaatggctggcctacggccaggcaatctaccagggcgcggacaagccgcgccgtcgccactcgaccgccggcgcccacatcaaggcaccctgcctcgcgcgtttcggtgatgacggtgaaaacctctgacacatgcagctcccggagacggtcacagcttgtctgtaagcggatgccgggagcagacaagcccgtcagggcgcgtcagcgggtgttggcgggtgtcggggcgcagccatgacccagtcacgtagcgatagcggagtgtatactggcttaactatgcggcatcagagcagattgtactgagagtgcaccatatgcggtgtgaaataccgcacagatgcgtaaggagaaaataccgcatcaggcgctcttccgcttcctcgctcactgactcgctgcgctcggtcgttcggctgcggcgagcggtatcagctcactcaaaggcggtaatacggttatccacagaatcaggggataacgcaggaaagaacatgtgagcaaaaggccagcaaa

SEQ ID NO: 13 - protein, 1072 aa, synthetic construct
MHHHHHHGSENLYFQGQLSYGYDEKSTGISVPGPMGPSGPRGLPGPPGAPGPQGFQGPPGEPGEPGASGPMGPRGPPGPPGKNGDDGEAGKPGRPGERGPPGPQGARGLPGTAGLPGMKGHRGFSGLDGAKGDAGPAGPKGEPGSPGENGAPGQMGPRGLPGERGRPGAPGPAGARGNDGATGAAGPPGPTGPAGPPGFPGAVGAKGEGGPQGPRGSEGPQGVRGEPGPPGPAGAAGPAGNPGADGQPGAKGANGAPGIAGAPGFPGARGPSGPQGPSGPPGPKGNSGEPGAPGSKGDTGAKGEPGPTGIQGPPGPAGEEGKRGARGEPGPAGLPGPPGERGGPGSRGFPGADGVAGPKGPAGERGAPGPAGPKGSPGEAGRPGEAGLPGAKGLTGSPGSPGPDGKTGPPGPAGQDGRPGPPGPPGARGQAGVMGFPGPKGAAGEPGKAGERGVPGPPGAVGPAGKDGEAGAQGPPGPAGPAGERGEQGPAGSPGFQGLPGPAGPPGEAGKPGEQGVPGDLGAPGPSGARGERGFPGERGVQGPPGPAGPRGANGAPGNDGAKGDAGAPGAPGSQGAPGLQGMPGERGAAGLPGPKGDRGDAGPKGADGAPGKDGVRGLTGPIGPPGPAGAPGDKGEAGPSGPAGPTGARGAPGDRGEPGPPGPAGFAGPPGADGQPGAKGEPGDAGAKGDAGPPGPAGPAGPPGPIGNVGAPGPKGARGSAGPPGATGFPGAAGRVGPPGPSGNAGPPGPPGPAGKEGSKGPRGETGPAGRPGEVGPPGPPGPAGEKGAPGADGPAGAPGTPGPQGIAGQRGVVGLPGQRGERGFPGLPGPSGEPGKQGPSGASGERGPPGPMGPPGLAGPPGESGREGAPGAEGSPGRDGSPGAKGDRGETGPAGPPGAPGAPGAPGPVGPAGKSGDRGETGPAGPAGPIGPVGARGPAGPQGPRGDKGETGEQGDRGIKGHRGFSGLQGPPGPPGSPGEQGPSGASGPAGPRGPPGSAGSPGKDGLNGLPGPIGPPGPRGRTGDAGPAGPPGPPGPPGPPGPPSGGYDLSFLPQPPQEKAHDGGRYYRA

SEQ ID NO: 14 - protein, 1056 aa, synthetic construct; identical to SEQ ID NO: 2

SEQ ID NO: 15 - DNA, 12157 bp, synthetic construct
  source 1..12157: mol_type = other DNA
  repeat_region 1932..1956: function = plasmid transfer to host cells; note = LB T-DNA repeat
  regulatory 2040..2737: note = p19 suppressor; regulatory_class = other
  regulatory 2738..3083: note = p35S_short promotor; regulatory_class = promoter
  regulatory 3088..3543: note = pPD7; regulatory_class = promoter
  CDS 3560..7489: note = fuGFP-Col1-AFVY; protein_id = 16; translation = MVSSGEDIFSGLVPILIELEGDVNGHRFSVRGEGYGDASNGKLEIKFICTTGRLPVPWPTLVTTLSYGVQCFAKYPEHMRQNDFFKSAMPDGYVQERTISFKEDGTYKTRAEVKFEGEALVNRIDLKGLEFKEDGNILGHKLEYSFNSHYVYITADKNRNGLEAQFRIRHNVDDGSVQLADHYQQNTPIGEGPVLLPEQHYLTTNSVLSKDPQERRDHMVLVEFVTAAGLSLGMDELYKSGSENLYFQGQLSYGYDEKSTGISVPGPMGPSGPRGLPGPPGAPGPQGFQGPPGEPGEPGASGPMGPRGPPGPPGKNGDDGEAGKPGRPGERGPPGPQGARGLPGTAGLPGMKGHRGFSGLDGAKGDAGPAGPKGEPGSPGENGAPGQMGPRGLPGERGRPGAPGPAGARGNDGATGAAGPPGPTGPAGPPGFPGAVGAKGEGGPQGPRGSEGPQGVRGEPGPPGPAGAAGPAGNPGADGQPGAKGANGAPGIAGAPGFPGARGPSGPQGPSGPPGPKGNSGEPGAPGSKGDTGAKGEPGPTGIQGPPGPAGEEGKRGARGEPGPAGLPGPPGERGGPGSRGFPGADGVAGPKGPAGERGAPGPAGPKGSPGEAGRPGEAGLPGAKGLTGSPGSPGPDGKTGPPGPAGQDGRPGPPGPPGARGQAGVMGFPGPKGAAGEPGKAGERGVPGPPGAVGPAGKDGEAGAQGPPGPAGPAGERGEQGPAGSPGFQGLPGPAGPPGEAGKPGEQGVPGDLGAPGPSGARGERGFPGERGVQGPPGPAGPRGANGAPGNDGAKGDAGAPGAPGSQGAPGLQGMPGERGAAGLPGPKGDRGDAGPKGADGAPGKDGVRGLTGPIGPPGPAGAPGDKGEAGPSGPAGPTGARGAPGDRGEPGPPGPAGFAGPPGADGQPGAKGEPGDAGAKGDAGPPGPAGPAGPPGPIGNVGAPGPKGARGSAGPPGATGFPGAAGRVGPPGPSGNAGPPGPPGPAGKEGSKGPRGETGPAGRPGEVGPPGPPGPAGEKGAPGADGPAGAPGTPGPQGIAGQRGVVGLPGQRGERGFPGLPGPSGEPGKQGPSGASGERGPPGPMGPPGLAGPPGESGREGAPGAEGSPGRDGSPGAKGDRGETGPAGPPGAPGAPGAPGPVGPAGKSGDRGETGPAGPAGPIGPVGARGPAGPQGPRGDKGETGEQGDRGIKGHRGFSGLQGPPGPPGSPGEQGPSGASGPAGPRGPPGSAGSPGKDGLNGLPGPIGPPGPRGRTGDAGPAGPPGPPGPPGPPGPPSGGYDLSFLPQPPQEKAHDGGRYYRAAFVY
  CDS 3563..4279: gene = fuGFP_codon-opt. N. tabacum; protein_id = 17; translation = VSSGEDIFSGLVPILIELEGDVNGHRFSVRGEGYGDASNGKLEIKFICTTGRLPVPWPTLVTTLSYGVQCFAKYPEHMRQNDFFKSAMPDGYVQERTISFKEDGTYKTRAEVKFEGEALVNRIDLKGLEFKEDGNILGHKLEYSFNSHYVYITADKNRNGLEAQFRIRHNVDDGSVQLADHYQQNTPIGEGPVLLPEQHYLTTNSVLSKDPQERRDHMVLVEFVTAAGLSLGMDELYKS
  CDS 4307..7474: gene = Col1a; protein_id = 18; translation = QLSYGYDEKSTGISVPGPMGPSGPRGLPGPPGAPGPQGFQGPPGEPGEPGASGPMGPRGPPGPPGKNGDDGEAGKPGRPGERGPPGPQGARGLPGTAGLPGMKGHRGFSGLDGAKGDAGPAGPKGEPGSPGENGAPGQMGPRGLPGERGRPGAPGPAGARGNDGATGAAGPPGPTGPAGPPGFPGAVGAKGEGGPQGPRGSEGPQGVRGEPGPPGPAGAAGPAGNPGADGQPGAKGANGAPGIAGAPGFPGARGPSGPQGPSGPPGPKGNSGEPGAPGSKGDTGAKGEPGPTGIQGPPGPAGEEGKRGARGEPGPAGLPGPPGERGGPGSRGFPGADGVAGPKGPAGERGAPGPAGPKGSPGEAGRPGEAGLPGAKGLTGSPGSPGPDGKTGPPGPAGQDGRPGPPGPPGARGQAGVMGFPGPKGAAGEPGKAGERGVPGPPGAVGPAGKDGEAGAQGPPGPAGPAGERGEQGPAGSPGFQGLPGPAGPPGEAGKPGEQGVPGDLGAPGPSGARGERGFPGERGVQGPPGPAGPRGANGAPGNDGAKGDAGAPGAPGSQGAPGLQGMPGERGAAGLPGPKGDRGDAGPKGADGAPGKDGVRGLTGPIGPPGPAGAPGDKGEAGPSGPAGPTGARGAPGDRGEPGPPGPAGFAGPPGADGQPGAKGEPGDAGAKGDAGPPGPAGPAGPPGPIGNVGAPGPKGARGSAGPPGATGFPGAAGRVGPPGPSGNAGPPGPPGPAGKEGSKGPRGETGPAGRPGEVGPPGPPGPAGEKGAPGADGPAGAPGTPGPQGIAGQRGVVGLPGQRGERGFPGLPGPSGEPGKQGPSGASGERGPPGPMGPPGLAGPPGESGREGAPGAEGSPGRDGSPGAKGDRGETGPAGPPGAPGAPGAPGPVGPAGKSGDRGETGPAGPAGPIGPVGARGPAGPQGPRGDKGETGEQGDRGIKGHRGFSGLQGPPGPPGSPGEQGPSGASGPAGPRGPPGSAGSPGKDGLNGLPGPIGPPGPRGRTGDAGPAGPPGPPGPPGPPGPPSGGYDLSFLPQPPQEKAHDGGRYYRA
  misc_feature 4286..4303: function = TEV cleavage site
  sig_peptide 7475..7486: function = Vacuolar targeting signal; note = AFVY
  regulatory 7530..7785: note = Nos pA; regulatory_class = polyA_signal_sequence; regulatory_class = terminator
  misc_feature 7809..7833: function = plasmid transfer to host cells; note = RB T-DNA repeat
aggccaggaaccgtaaaaaggccgcgttgctggcgtttttccataggctccgcccccctgacgagcatcacaaaaatcgacgctcaagtcagaggtggcgaaacccgacaggactataaagataccaggcgtttccccctggaagctccctcgtgcgctctcctgttccgaccctgccgcttaccggatacctgtccgcctttctcccttcgggaagcgtggcgctttctcatagctcacgctgtaggtatctcagttcggtgtaggtcgttcgctccaagctgggctgtgtgcacgaaccccccgttcagcccgaccgctgcgccttatccggtaactatcgtcttgagtccaacccggtaagacacgacttatcgccactggcagcagccactggtaacaggattagcagagcgaggtatgtaggcggtgctacagagttcttgaagtggtggcctaactacggctacactagaaggacagtatttggtatctgcgctctgctgaagccagttaccttcggaaaaagagttggtagctcttgatccggcaaacaaaccaccgctggtagcggtggtttttttgtttgcaagcagcagattacgcgcagaaaaaaaggatctcaagaagatcctttgatcttttctacggggtctgacgctcagtggaacgaaaactcacgttaagggattttggtcatgcattctaggtactaaaacaattcatccagtaaaatataatattttattttctcccaatcaggcttgatccccagtaagtcaaaaaatagctcgacatactgttcttccccgatatcctccctgatcgaccggacgcagaaggcaatgtcataccacttgtccgccctgccgcttctcccaagatcaataaagccacttactttgccatctttcacaaagatgttgctgtctcccaggtcgccgtgggaaaagacaagttcctcttcgggcttttccgtctttaaaaaatcatacagctcgcgcggatctttaaatggagtgtcttcttcccagttttcgcaatccacatcggccagatcgttattcagtaagtaatccaattcggctaagcggctgtctaagctattcgtatagggacaatccgatatgtcgatggagtgaaagagcctgatgcactccgcatacagctcgataatcttttcagggctttgttcatcttcatactcttccgagcaaaggacgccatcggcctcactcatgagcagattgctccagccatcatgccgttcaaagtgcaggacctttggaacaggcagctttccttccagccatagcatcatgtccttttcccgttccacatcataggtggtccctttataccggctgtccgtcatttttaaatataggttttcattttctcccaccagcttatataccttagcaggagacattccttccgtatcttttacgcagcggtatttttcgatcagttttttcaattccggtgatattctcattttagccatttattatttccttcctcttttctacagtatttaaagataccccaagaagctaattataacaagacgaactccaattcactgttccttgcattctaaaaccttaaataccagaaaacagctttttcaaagttgttttcaaagttggcgtataacatagtatcgacggagccgattttgaaaccgcggtgatcacaggcagcaacgctctgtcatcgttacaatcaacatgctaccctccgcgagatcatccgtgtttcaaacccggcagcttagttgccgttcttccgaatagcatcggtaacatgagcaaagtctgccgccttacaacggctctcccgctgacgccgtcccggactgatgggctgcctgtatcgagtggtgattttgtgccgagctgccggtcggggagctgttggctggctggtggcaggatatattgtggtgtaaacaaattgacgcttagacaacttaataacacattgcggacgtttttaatgtactgaattaacgccgaattgaattcgagctcggtggaggatctggattttagtactggattttggttttaggaattagaaattttattgatagaagtattttacaaatacaaatacatactaagggtttcttatatgctcaacacatgagcgaaaccctataggaaccctaattcccttatctgggaactactcacacattattatggagaaactattcactctccttctcaaacgtttctgttccctctggacagccccgactgacgttggactcaacctcaatgggcgctaattgtaatagctcctgtttgcttcttatggccatttcgcaaaggtgttgcagtgttctgctaccaccactcactgtaattgacacacctctgaaacggatggagtaagtgcaaccaatttgatcaaatccaaagaaacgactagcagcgtaatttactgagtcaccagtccaggaacctagaactcgatggagagaggcctctgtccgatcatagcgtaggtagcgtttgaaaactaccttgccaaatccccaggactctttaaatcccagtgggttgtcctggttggagtttgtttcgtcattgtgtaaacgccattctgtccaagatgggctctcatcgggtaacttaaatgggctggtagtgccgccagaaccaccgtcccatctctctgaattggcctgctctcttgcatcattaccctggattgctctctccattgtcctctccaaatgaaatgaacttccttatatagaggaagggtcttgcgaaggatagtgggattgtgcgtcatcccttacgtcagtggagatgtcacatcaatccacttgctttgtagacgtggttggaacctcttctttttccacgatgctcctcgtgggtgggggtccatctttgggaccactgtcggcagagagatcttgaatgatagcctttcctttatcgcaatgatggcatttgtaggagccaccttccttttctactgtcctttcgatgaagtgacagatagctgggcaatggaatccgaggaggtttcccgaaattatcctttgttgaaaagtctcaaacaataggcaaccgtggacttcttcactagctcatcgagatagcaatgccactagctaatttcttacgttgtatcttatttgttttactttggggcatgacatggttaaaccccatcaaagagaaagtgtttcatccactagtcaatatacgaattcattcgaatttatccctgtaaatcctagttcttaggatgaactggtgtaataaacagcaaaaaaaaataaaaaaaaataaatctggaatcattcgaccacctcaataaactaaagctaccaattaccacaatatagtcatccatatccacttagatataaaagataaaagtaaacaaatattaaatttcatatgcacgcataggaaactcatgatcttatcttttaaatagacatctagttttcttaggttataaatagacattttgtcctagaacttcttcactactaaaacctagcctcaaaaagcaggctgccaccatggtgagcagtggtgaggacatcttttcaggcctagtcccgatacttattgaacttgaaggagacgtcaatgggcacagattctcagtacgaggcgagggatacggggatgcttccaatggaaagcttgagataaaatttatatgtacaactggaaggcttcctgtcccatggccaactttagttaccactcttagctacggtgtacaatgcttcgctaaatacccagaacatatgcgtcagaatgacttcttcaagtcagcaatgcctgatggatatgttcaagaaagaacaatctcttttaaagaggacggaacttataagaccagagctgaagtcaaattcgagggagaggccttggtgaacagaattgacttaaaaggactggaattcaaggaagatggcaatatcctcggtcacaagcttgaatacagttttaattcacactacgtgtatataaccgcggataagaacaggaatggtttagaagctcagtttagaataagacataacgtggacgatggatccgtgcagctagcagatcactatcagcaaaatacgccgataggggaaggccctgttcttttgccagagcagcattacctaactactaactctgttttgtctaaggacccacaagagcggagagatcatatggttttggttgagttcgttacggcagctggactctccctaggcatggatgaattatacaaatcaggatctgagaatttatattttcaaggtcaattgagttatggatacgacgaaaaatcaactggaatatcagtgccaggaccaatgggtccatcaggacctaggggtcttccagggccacctggcgctcctggtcctcagggatttcaaggtcctccaggtgaacctggagagcctggtgcttctggtccaatgggaccaagaggccctcctggtccacctggtaaaaatggtgatgatggtgaggctggaaagcctggtcgtcctggagaaagaggaccaccaggaccacagggagctagaggtttgccaggtacagccggtcttccaggaatgaaaggacacaggggtttttctggtcttgatggtgctaagggagacgcaggacctgctggaccaaagggtgaacctggatctcctggtgaaaatggtgctcctggacaaatgggacctagaggattgcctggcgaaagaggaagacctggtgctcctggaccagctggagctagaggaaatgatggagctactggtgctgccggaccaccaggaccaactggaccagctggaccacctggttttccaggagcagttggggctaagggagaaggtggaccacaaggacctagaggatcagaaggacctcaaggagttaggggagaaccaggtcctcctggtcctgctggagctgctggacccgctggtaacccaggagcagatggacaacctggagcaaaaggggctaatggtgctcctggtattgcaggtgctcctggattccctggtgctagaggaccttcaggacctcagggaccatccggtcctccaggaccaaagggaaactctggtgaaccaggggctcctggatctaagggagatactggagctaagggtgagccaggacctacaggaattcaaggaccaccaggacctgcaggagaggaaggtaagaggggtgctagaggtgaacctggaccagctggattgccaggcccacctggagagaggggtggtccaggttctagaggttttccaggagctgatggagttgctggtccaaagggtcctgctggtgagagaggtgcacctggaccagcaggacctaaaggatcacctggagaagctggtcgtcctggtgaggctggtcttccaggtgctaagggccttacaggatctccaggatcaccaggtccagatggaaagactggaccaccaggtcctgcaggacaagatggaaggcctggtccacctggaccacctggtgctaggggacaagctggtgttatgggattcccaggtccaaagggtgcagctggtgagcctggtaaagctggtgaaagaggagttccaggacctcctggtgctgttggacctgctggtaaagatggtgaagcaggtgctcagggtccaccaggtccagccggtccagctggtgagaggggagagcaaggtcctgctggatctcctggatttcaaggtttgcctggacctgctggacctccaggagaggctggtaaacctggtgagcagggtgtgcctggtgatcttggtgctcctggacctagtggcgcaagaggcgaaaggggatttccaggtgaaagaggagttcagggaccaccaggtccagctggtccaagaggcgctaatggagctccaggaaatgatggagcaaagggtgatgctggcgctccaggagctcctggttctcaaggtgcacctggattgcaaggaatgccaggagagagaggtgcagctggtttgccgggaccaaagggtgatagaggtgatgctggtcctaagggagctgatggagctccaggaaaggatggtgtgagaggattgactggtccaattggaccaccaggtcctgctggagcaccaggagataaaggagaagctggtccttcaggaccagccggtccaactggagctagaggagctccaggagatagaggtgaaccaggaccaccaggacctgctgggtttgcaggtccacctggtgctgatggacaacctggtgctaaaggagaaccaggcgatgctggtgctaagggagatgctggcccacctggtccagctggtcctgctgggccaccaggtcctatcggaaatgttggtgctccagggcctaaaggagctagaggatcagcaggtcccccaggtgctacaggttttccaggggctgctggaagagtgggtcccccaggtccttctgggaatgcaggaccaccaggtcctccaggaccagctggaaaagaaggaagtaagggaccaaggggagaaactggacctgcaggacgtccaggtgaagttggtccacctggacctccaggtccagctggagagaaaggagctccaggagctgatggtccagcaggtgctcctggtactccaggtccacaaggtattgctggtcaaaggggagtggttggtctcccaggtcagagaggtgaaagaggtttcccaggtttgcctggaccatctggagaaccaggtaagcagggcccatctggagcttctggtgagagagggccacctggacctatgggacctcctgggcttgctggacctccaggggaatctggtagggagggtgctccaggtgctgaaggatcacctggtagagatggatcacctggagctaaaggtgatagaggggaaacaggtccagcaggtccacctggcgctcctggtgctccaggagcaccagggccagttggacctgctggaaagtctggagataggggagagactggaccagctggacctgctggaccaatcggtcctgttggcgctagaggtcctgctggaccacaaggtcctaggggagataaaggtgaaacaggtgaacaaggagatagaggaattaaaggtcatagagggttttctggtttgcaaggacctccaggacctcctggatctccaggagagcaaggaccatctggtgcaagcggacctgctggtcctagaggacctccaggttcagctggctcacctggtaaggatggattaaatggtttgcctggaccaataggtccaccaggacctagaggaaggacaggtgatgcaggaccagctggtccacctggtccaccaggaccaccaggaccaccaggtccaccttctggtggatatgatcttagttttcttcctcaacctccccaggagaaagctcatgatggtggtagatattatagggctgcatttgtttattaaacccagctttcttgtacaaagtggtagctcgaatttccccgatcgttcaaacatttggcaataaagtttcttaagattgaatcctgttgccggtcttgcgatgattatcatataatttctgttgaattacgttaagcatgtaataattaacatgtaatgcatgacgttatttatgagatgggtttttatgattagagtcccgcaattatacatttaatacgcgatagaaaacaaaatatagcgcgcaaactaggataaattatcgcgcgcggtgtcatctatgttactagatcgggaaagcttttaaactatcagtgtttgacaggatatattggcgggtaaacctaagagaaaagagcgtttattagaataatcggatatttaaaagggcgtgaaaaggtttatccgttcgtccatttgtatgtgcatgccaaccacagggttcccctcgggatcaaagtactttgatccaacccctccgctgctatagtgcagtcggcttctgacgttcagtgcagccgtcttctgaaaacgacatgtcgcacaagtcctaagttacgcgacaggctgccgccctgcccttttcctggcgttttcttgtcgcgtgttttagtcgcataaagtagaatacttgcgactagaaccggagacattacgccatgaacaagagcgccgccgctggcctgctgggctatgcccgcgtcagcaccgacgaccaggacttgaccaaccaacgggccgaactgcacgcggccggctgcaccaagctgttttccgagaagatcaccggcaccaggcgcgaccgcccggagctggccaggatgcttgaccacctacgccctggcgacgttgtgacagtgaccaggctagaccgcctggcccgcagcacccgcgacctactggacattgccgagcgcatccaggaggccggcgcgggcctgcgtagcctggcagagccgtgggccgacaccaccacgccggccggccgcatggtgttgaccgtgttcgccggcattgccgagttcgagcgttccctaatcatcgaccgcacccggagcgggcgcgaggccgccaaggcccgaggcgtgaagtttggcccccgccctaccctcaccccggcacagatcgcgcacgcccgcgagctgatcgaccaggaaggccgcaccgtgaaagaggcggctgcactgcttggcgtgcatcgctcgaccctgtaccgcgcacttgagcgcagcgaggaagtgacgcccaccgaggccaggcggcgcggtgccttccgtgaggacgcattgaccgaggccgacgccctggcggccgccgagaatgaacgccaagaggaacaagcatgaaaccgcaccaggacggccaggacgaaccgtttttcattaccgaagagatcgaggcggagatgatcgcggccgggtacgtgttcgagccgcccgcgcacgtctcaaccgtgcggctgcatgaaatcctggccggtttgtctgatgccaagctggcggcctggccggccagcttggccgctgaagaaaccgagcgccgccgtctaaaaaggtgatgtgtatttgagtaaaacagcttgcgtcatgcggtcgctgcgtatatgatgcgatgagtaaataaacaaatacgcaaggggaacgcatgaaggttatcgctgtacttaaccagaaaggcgggtcaggcaagacgaccatcgcaacccatctagcccgcgccctgcaactcgccggggccgatgttctgttagtcgattccgatccccagggcagtgcccgcgattgggcggccgtgcgggaagatcaaccgctaaccgttgtcggcatcgaccgcccgacgattgaccgcgacgtgaaggccatcggccggcgcgacttcgtagtgatcgacggagcgccccaggcggcggacttggctgtgtccgcgatcaaggcagccgacttcgtgctgattccggtgcagccaagcccttacgacatatgggccaccgccgacctggtggagctggttaagcagcgcattgaggtcacggatggaaggctacaagcggcctttgtcgtgtcgcgggcgatcaaaggcacgcgcatcggcggtgaggttgccgaggcgctggccgggtacgagctgcccattcttgagtcccgtatcacgcagcgcgtgagctacccaggcactgccgccgccggcacaaccgttcttgaatcagaacccgagggcgacgctgcccgcgaggtccaggcgctggccgctgaaattaaatcaaaactcatttgagttaatgaggtaaagagaaaatgagcaaaagcacaaacacgctaagtgccggccgtccgagcgcacgcagcagcaaggctgcaacgttggccagcctggcagacacgccagccatgaagcgggtcaactttcagttgccggcggaggatcacaccaagctgaagatgtacgcggtacgccaaggcaagaccattaccgagctgctatctgaatacatcgcgcagctaccagagtaaatgagcaaatgaataaatgagtagatgaattttagcggctaaaggaggcggcatggaaaatcaagaacaaccaggcaccgacgccgtggaatgccccatgtgtggaggaacgggcggttggccaggcgtaagcggctgggttgcctgccggccctgcaatggcactggaacccccaagcccgaggaatcggcgtgagcggtcgcaaaccatccggcccggtacaaatcggcgcggcgctgggtgatgacctggtggagaagttgaaggccgcgcaggccgcccagcggcaacgcatcgaggcagaagcacgccccggtgaatcgtggcaagcggccgctgatcgaatccgcaaagaatcccggcaaccgccggcagccggtgcgccgtcgattaggaagccgcccaagggcgacgagcaaccagattttttcgttccgatgctctatgacgtgggcacccgcgatagtcgcagcatcatggacgtggccgttttccgtctgtcgaagcgtgaccgacgagctggcgaggtgatccgctacgagcttccagacgggcacgtagaggtttccgcagggccggccggcatggccagtgtgtgggattacgacctggtactgatggcggtttcccatctaaccgaatccatgaaccgataccgggaagggaagggagacaagcccggccgcgtgttccgtccacacgttgcggacgtactcaagttctgccggcgagccgatggcggaaagcagaaagacgacctggtagaaacctgcattcggttaaacaccacgcacgttgccatgcagcgtacgaagaaggccaagaacggccgcctggtgacggtatccgagggtgaagccttgattagccgctacaagatcgtaaagagcgaaaccgggcggccggagtacatcgagatcgagctagctgattggatgtaccgcgagatcacagaaggcaagaacccggacgtgctgacggttcaccccgattactttttgatcgatcccggcatcggccgttttctctaccgcctggcacgccgcgccgcaggcaaggcagaagccagatggttgttcaagacgatctacgaacgcagtggcagcgccggagagttcaagaagttctgtttcaccgtgcgcaagctgatcgggtcaaatgacctgccggagtacgatttgaaggaggaggcggggcaggctggcccgatcctagtcatgcgctaccgcaacctgatcgagggcgaagcatccgccggttcctaatgtacggagcagatgctagggcaaattgccctagcaggggaaaaaggtcgaaaaggtctctttcctgtggatagcacgtacattgggaacccaaagccgtacattgggaaccggaacccgtacattgggaacccaaagccgtacattgggaaccggtcacacatgtaagtgactgatataaaagagaaaaaaggcgatttttccgcctaaaactctttaaaacttattaaaactcttaaaacccgcctggcctgtgcataactgtctggccagcgcacagccgaagagctgcaaaaagcgcctacccttcggtcgctgcgctccctacgccccgccgcttcgcgtcggcctatcgcggccgctggccgctcaaaaatggctggcctacggccaggcaatctaccagggcgcggacaagccgcgccgtcgccactcgaccgccggcgcccacatcaaggcaccctgcctcgcgcgtttcggtgatgacggtgaaaacctctgacacatgcagctcccggagacggtcacagcttgtctgtaagcggatgccgggagcagacaagcccgtcagggcgcgtcagcgggtgttggcgggtgtcggggcgcagccatgacccagtcacgtagcgatagcggagtgtatactggcttaactatgcggcatcagagcagattgtactgagagtgcaccatatgcggtgtgaaataccgcacagatgcgtaaggagaaaataccgcatcaggcgctcttccgcttcctcgctcactgactcgctgcgctcggtcgttcggctgcggcgagcggtatcagctcactcaaaggcggtaatacggttatccacagaatcaggggataacgcaggaaagaacatgtgagcaaaaggccagcaaa

SEQ ID NO: 16 - protein, 1309 aa, synthetic construct
MVSSGEDIFSGLVPILIELEGDVNGHRFSVRGEGYGDASNGKLEIKFICTTGRLPVPWPTLVTTLSYGVQCFAKYPEHMRQNDFFKSAMPDGYVQERTISFKEDGTYKTRAEVKFEGEALVNRIDLKGLEFKEDGNILGHKLEYSFNSHYVYITADKNRNGLEAQFRIRHNVDDGSVQLADHYQQNTPIGEGPVLLPEQHYLTTNSVLSKDPQERRDHMVLVEFVTAAGLSLGMDELYKSGSENLYFQGQLSYGYDEKSTGISVPGPMGPSGPRGLPGPPGAPGPQGFQGPPGEPGEPGASGPMGPRGPPGPPGKNGDDGEAGKPGRPGERGPPGPQGARGLPGTAGLPGMKGHRGFSGLDGAKGDAGPAGPKGEPGSPGENGAPGQMGPRGLPGERGRPGAPGPAGARGNDGATGAAGPPGPTGPAGPPGFPGAVGAKGEGGPQGPRGSEGPQGVRGEPGPPGPAGAAGPAGNPGADGQPGAKGANGAPGIAGAPGFPGARGPSGPQGPSGPPGPKGNSGEPGAPGSKGDTGAKGEPGPTGIQGPPGPAGEEGKRGARGEPGPAGLPGPPGERGGPGSRGFPGADGVAGPKGPAGERGAPGPAGPKGSPGEAGRPGEAGLPGAKGLTGSPGSPGPDGKTGPPGPAGQDGRPGPPGPPGARGQAGVMGFPGPKGAAGEPGKAGERGVPGPPGAVGPAGKDGEAGAQGPPGPAGPAGERGEQGPAGSPGFQGLPGPAGPPGEAGKPGEQGVPGDLGAPGPSGARGERGFPGERGVQGPPGPAGPRGANGAPGNDGAKGDAGAPGAPGSQGAPGLQGMPGERGAAGLPGPKGDRGDAGPKGADGAPGKDGVRGLTGPIGPPGPAGAPGDKGEAGPSGPAGPTGARGAPGDRGEPGPPGPAGFAGPPGADGQPGAKGEPGDAGAKGDAGPPGPAGPAGPPGPIGNVGAPGPKGARGSAGPPGATGFPGAAGRVGPPGPSGNAGPPGPPGPAGKEGSKGPRGETGPAGRPGEVGPPGPPGPAGEKGAPGADGPAGAPGTPGPQGIAGQRGVVGLPGQRGERGFPGLPGPSGEPGKQGPSGASGERGPPGPMGPPGLAGPPGESGREGAPGAEGSPGRDGSPGAKGDRGETGPAGPPGAPGAPGAPGPVGPAGKSGDRGETGPAGPAGPIGPVGARGPAGPQGPRGDKGETGEQGDRGIKGHRGFSGLQGPPGPPGSPGEQGPSGASGPAGPRGPPGSAGSPGKDGLNGLPGPIGPPGPRGRTGDAGPAGPPGPPGPPGPPGPPSGGYDLSFLPQPPQEKAHDGGRYYRAAFVY

SEQ ID NO: 17 - protein, 239 aa, synthetic construct
VSSGEDIFSGLVPILIELEGDVNGHRFSVRGEGYGDASNGKLEIKFICTTGRLPVPWPTLVTTLSYGVQCFAKYPEHMRQNDFFKSAMPDGYVQERTISFKEDGTYKTRAEVKFEGEALVNRIDLKGLEFKEDGNILGHKLEYSFNSHYVYITADKNRNGLEAQFRIRHNVDDGSVQLADHYQQNTPIGEGPVLLPEQHYLTTNSVLSKDPQERRDHMVLVEFVTAAGLSLGMDELYKS

SEQ ID NO: 18 - protein, 1056 aa, synthetic construct; identical to SEQ ID NO: 2

SEQ ID NO: 19 - protein, 1463 aa, synthetic construct; identical to SEQ ID NO: 1

SEQ ID NO: 20 - protein, 1467 aa, synthetic construct
MFSFVDLRLLLLLAATALLTHGQEEGQEEGQEEDIPPVTCVQNGLRYHDRDVWKPVPCQICVCDNGNVLCDDVICDELKDCPNAKVPTDECCPVCPEGQESPTDQETTGVEGPKGDTGPRGPRGPAGPPGRDGIPGQPGLPGPPGPPGPPGPPGLGGNFAPQLSYGYDEKSTGISVPGPMGPSGPRGLPGPPGAPGPQGFQGPPGEPGEPGASGPMGPRGPPGPPGKNGDDGEAGKPGRPGERGPPGPQGARGLPGTAGLPGMKGHRGFSGLDGAKGDAGPAGPKGEPGSPGENGAPGQMGPRGLPGERGRPGAPGPAGARGNDGATGAAGPPGPTGPAGPPGFPGAVGAKGEGGPQGPRGSEGPQGVRGEPGPPGPAGAAGPAGNPGADGQPGAKGANGAPGIAGAPGFPGARGPSGPQGPSGPPGPKGNSGEPGAPGSKGDTGAKGEPGPTGIQGPPGPAGEEGKRGARGEPGPAGLPGPPGERGGPGSRGFPGADGVAGPKGPAGERGAPGPAGPKGSPGEAGRPGEAGLPGAKGLTGSPGSPGPDGKTGPPGPAGQDGRPGPPGPPGARGQAGVMGFPGPKGAAGEPGKAGERGVPGPPGAVGPAGKDGEAGAQGPPGPAGPAGERGEQGPAGSPGFQGLPGPAGPPGEAGKPGEQGVPGDLGAPGPSGARGERGFPGERGVQGPPGPAGPRGANGAPGNDGAKGDAGAPGAPGSQGAPGLQGMPGERGAAGLPGPKGDRGDAGPKGADGAPGKDGVRGLTGPIGPPGPAGAPGDKGEAGPSGPAGPTGARGAPGDRGEPGPPGPAGFAGPPGADGQPGAKGEPGDAGAKGDAGPPGPAGPAGPPGPIGNVGAPGPKGARGSAGPPGATGFPGAAGRVGPPGPSGNAGPPGPPGPAGKEGSKGPRGETGPAGRPGEVGPPGPPGPAGEKGAPGADGPAGAPGTPGPQGIAGQRGVVGLPGQRGERGFPGLPGPSGEPGKQGPSGASGERGPPGPMGPPGLAGPPGESGREGAPGAEGSPGRDGSPGAKGDRGETGPAGPPGAPGAPGAPGPVGPAGKSGDRGETGPAGPAGPIGPVGARGPAGPQGPRGDKGETGEQGDRGIKGHRGFSGLQGPPGPPGSPGEQGPSGASGPAGPRGPPGSAGSPGKDGLNGLPGPIGPPGPRGRTGDAGPAGPPGPPGPPGPPGPPSGGYDLSFLPQPPQEKAHDGGRYYRADDANVVRDRDLEVDTTLKSLSQQIENIRSPEGSRKNPARTCRDLKMCHSDWKSGEYWIDPNQGCNLDAIKVFCNMETGETCVYPTQPSVAQKNWYISKNPKEKRHVWYGESMTGGFQFEYGGQGSDPADVAIQLTFLRLMSTEASQNITYHCKNSVAYMDQQTGNLKKALLLQGSNEIEIRAEGNSRFTYSVTYDGCTSHTGAWGKTVIEYKTTKTSRLPIIDVAPLDVGAPDQEFGFDVGPACFLAFVY

SEQ ID NO: 21 - DNA, 12145 bp, synthetic construct
  source 1..12145: mol_type = other DNA
  misc_feature 1932..1956: function = plasmid transfer to host cells; note = LB T-DNA repeat
  regulatory 2040..2767: note = p19 suppressor; regulatory_class = other
  regulatory 2738..3083: note = p35S_short; regulatory_class = promoter
  regulatory 3088..3543: note = pPD7; regulatory_class = promoter
  CDS 3560..7477: gene = fuGFP-Col1a; protein_id = 22; translation = MVSSGEDIFSGLVPILIELEGDVNGHRFSVRGEGYGDASNGKLEIKFICTTGRLPVPWPTLVTTLSYGVQCFAKYPEHMRQNDFFKSAMPDGYVQERTISFKEDGTYKTRAEVKFEGEALVNRIDLKGLEFKEDGNILGHKLEYSFNSHYVYITADKNRNGLEAQFRIRHNVDDGSVQLADHYQQNTPIGEGPVLLPEQHYLTTNSVLSKDPQERRDHMVLVEFVTAAGLSLGMDELYKSGSENLYFQGQLSYGYDEKSTGISVPGPMGPSGPRGLPGPPGAPGPQGFQGPPGEPGEPGASGPMGPRGPPGPPGKNGDDGEAGKPGRPGERGPPGPQGARGLPGTAGLPGMKGHRGFSGLDGAKGDAGPAGPKGEPGSPGENGAPGQMGPRGLPGERGRPGAPGPAGARGNDGATGAAGPPGPTGPAGPPGFPGAVGAKGEGGPQGPRGSEGPQGVRGEPGPPGPAGAAGPAGNPGADGQPGAKGANGAPGIAGAPGFPGARGPSGPQGPSGPPGPKGNSGEPGAPGSKGDTGAKGEPGPTGIQGPPGPAGEEGKRGARGEPGPAGLPGPPGERGGPGSRGFPGADGVAGPKGPAGERGAPGPAGPKGSPGEAGRPGEAGLPGAKGLTGSPGSPGPDGKTGPPGPAGQDGRPGPPGPPGARGQAGVMGFPGPKGAAGEPGKAGERGVPGPPGAVGPAGKDGEAGAQGPPGPAGPAGERGEQGPAGSPGFQGLPGPAGPPGEAGKPGEQGVPGDLGAPGPSGARGERGFPGERGVQGPPGPAGPRGANGAPGNDGAKGDAGAPGAPGSQGAPGLQGMPGERGAAGLPGPKGDRGDAGPKGADGAPGKDGVRGLTGPIGPPGPAGAPGDKGEAGPSGPAGPTGARGAPGDRGEPGPPGPAGFAGPPGADGQPGAKGEPGDAGAKGDAGPPGPAGPAGPPGPIGNVGAPGPKGARGSAGPPGATGFPGAAGRVGPPGPSGNAGPPGPPGPAGKEGSKGPRGETGPAGRPGEVGPPGPPGPAGEKGAPGADGPAGAPGTPGPQGIAGQRGVVGLPGQRGERGFPGLPGPSGEPGKQGPSGASGERGPPGPMGPPGLAGPPGESGREGAPGAEGSPGRDGSPGAKGDRGETGPAGPPGAPGAPGAPGPVGPAGKSGDRGETGPAGPAGPIGPVGARGPAGPQGPRGDKGETGEQGDRGIKGHRGFSGLQGPPGPPGSPGEQGPSGASGPAGPRGPPGSAGSPGKDGLNGLPGPIGPPGPRGRTGDAGPAGPPGPPGPPGPPGPPSGGYDLSFLPQPPQEKAHDGGRYYRA
  CDS 3563..4279: gene = fuGFP_codon opt. N. tabacum; protein_id = 23; translation = VSSGEDIFSGLVPILIELEGDVNGHRFSVRGEGYGDASNGKLEIKFICTTGRLPVPWPTLVTTLSYGVQCFAKYPEHMRQNDFFKSAMPDGYVQERTISFKEDGTYKTRAEVKFEGEALVNRIDLKGLEFKEDGNILGHKLEYSFNSHYVYITADKNRNGLEAQFRIRHNVDDGSVQLADHYQQNTPIGEGPVLLPEQHYLTTNSVLSKDPQERRDHMVLVEFVTAAGLSLGMDELYKS
  CDS 4307..7477: gene = COL1A1; protein_id = 24; translation = QLSYGYDEKSTGISVPGPMGPSGPRGLPGPPGAPGPQGFQGPPGEPGEPGASGPMGPRGPPGPPGKNGDDGEAGKPGRPGERGPPGPQGARGLPGTAGLPGMKGHRGFSGLDGAKGDAGPAGPKGEPGSPGENGAPGQMGPRGLPGERGRPGAPGPAGARGNDGATGAAGPPGPTGPAGPPGFPGAVGAKGEGGPQGPRGSEGPQGVRGEPGPPGPAGAAGPAGNPGADGQPGAKGANGAPGIAGAPGFPGARGPSGPQGPSGPPGPKGNSGEPGAPGSKGDTGAKGEPGPTGIQGPPGPAGEEGKRGARGEPGPAGLPGPPGERGGPGSRGFPGADGVAGPKGPAGERGAPGPAGPKGSPGEAGRPGEAGLPGAKGLTGSPGSPGPDGKTGPPGPAGQDGRPGPPGPPGARGQAGVMGFPGPKGAAGEPGKAGERGVPGPPGAVGPAGKDGEAGAQGPPGPAGPAGERGEQGPAGSPGFQGLPGPAGPPGEAGKPGEQGVPGDLGAPGPSGARGERGFPGERGVQGPPGPAGPRGANGAPGNDGAKGDAGAPGAPGSQGAPGLQGMPGERGAAGLPGPKGDRGDAGPKGADGAPGKDGVRGLTGPIGPPGPAGAPGDKGEAGPSGPAGPTGARGAPGDRGEPGPPGPAGFAGPPGADGQPGAKGEPGDAGAKGDAGPPGPAGPAGPPGPIGNVGAPGPKGARGSAGPPGATGFPGAAGRVGPPGPSGNAGPPGPPGPAGKEGSKGPRGETGPAGRPGEVGPPGPPGPAGEKGAPGADGPAGAPGTPGPQGIAGQRGVVGLPGQRGERGFPGLPGPSGEPGKQGPSGASGERGPPGPMGPPGLAGPPGESGREGAPGAEGSPGRDGSPGAKGDRGETGPAGPPGAPGAPGAPGPVGPAGKSGDRGETGPAGPAGPIGPVGARGPAGPQGPRGDKGETGEQGDRGIKGHRGFSGLQGPPGPPGSPGEQGPSGASGPAGPRGPPGSAGSPGKDGLNGLPGPIGPPGPRGRTGDAGPAGPPGPPGPPGPPGPPSGGYDLSFLPQPPQEKAHDGGRYYRA
  misc_feature 4286..4303: function = cleavage site; note = TEV site
  regulatory 7517..7773: note = Nos pA; regulatory_class = terminator; regulatory_class = polyA_signal_sequence
  misc_feature 7797..7821: function = plasmid transfer to host cells; note = RB T-DNA repeat
aggccaggaaccgtaaaaaggccgcgttgctggcgtttttccataggctccgcccccctgacgagcatcacaaaaatcgacgctcaagtcagaggtggcgaaacccgacaggactataaagataccaggcgtttccccctggaagctccctcgtgcgctctcctgttccgaccctgccgcttaccggatacctgtccgcctttctcccttcgggaagcgtggcgctttctcatagctcacgctgtaggtatctcagttcggtgtaggtcgttcgctccaagctgggctgtgtgcacgaaccccccgttcagcccgaccgctgcgccttatccggtaactatcgtcttgagtccaacccggtaagacacgacttatcgccactggcagcagccactggtaacaggattagcagagcgaggtatgtaggcggtgctacagagttcttgaagtggtggcctaactacggctacactagaaggacagtatttggtatctgcgctctgctgaagccagttaccttcggaaaaagagttggtagctcttgatccggcaaacaaaccaccgctggtagcggtggtttttttgtttgcaagcagcagattacgcgcagaaaaaaaggatctcaagaagatcctttgatcttttctacggggtctgacgctcagtggaacgaaaactcacgttaagggattttggtcatgcattctaggtactaaaacaattcatccagtaaaatataatattttattttctcccaatcaggcttgatccccagtaagtcaaaaaatagctcgacatactgttcttccccgatatcctccctgatcgaccggacgcagaaggcaatgtcataccacttgtccgccctgccgcttctcccaagatcaataaagccacttactttgccatctttcacaaagatgttgctgtctcccaggtcgccgtgggaaaagacaagttcctcttcgggcttttccgtctttaaaaaatcatacagctcgcgcggatctttaaatggagtgtcttcttcccagttttcgcaatccacatcggccagatcgttattcagtaagtaatccaattcggctaagcggctgtctaagctattcgtatagggacaatccgatatgtcgatggagtgaaagagcctgatgcactccgcatacagctcgataatcttttcagggctttgttcatcttcatactcttccgagcaaaggacgccatcggcctcactcatgagcagattgctccagccatcatgccgttcaaagtgcaggacctttggaacaggcagctttccttccagccatagcatcatgtccttttcccgttccacatcataggtggtccctttataccggctgtccgtcatttttaaatataggttttcattttctcccaccagcttatataccttagcaggagacattccttccgtatcttttacgcagcggtatttttcgatcagttttttcaattccggtgatattctcattttagccatttattatttccttcctcttttctacagtatttaaagataccccaagaagctaattataacaagacgaactccaattcactgttccttgcattctaaaaccttaaataccagaaaacagctttttcaaagttgttttcaaagttggcgtataacatagtatcgacggagccgattttgaaaccgcggtgatcacaggcagcaacgctctgtcatcgttacaatcaacatgctaccctccgcgagatcatccgtgtttcaaacccggcagcttagttgccgttcttccgaatagcatcggtaacatgagcaaagtctgccgccttacaacggctctcccgctgacgccgtcccggactgatgggctgcctgtatcgagtggtgattttgtgccgagctgccggtcggggagctgttggctggctggtggcaggatatattgtggtgtaaacaaattgacgcttagacaacttaataacacattgcggacgtttttaatgtactgaattaacgccgaattgaattcgagctcggtggaggatctggattttagtactggattttggttttaggaattagaaattttattgatagaagtattttacaaatacaaatacatactaagggtttcttatatgctcaacacatgagcgaaaccctataggaaccctaattcccttatctgggaactactcacacattattatggagaaactattcactctccttctcaaacgtttctgttccctctggacagccccgactgacgttggactcaacctcaatgggcgctaattgtaatagctcctgtttgcttcttatggccatttcgcaaaggtgttgcagtgttctgctaccaccactcactgtaattgacacacctctgaaacggatggagtaagtgcaaccaatttgatcaaatccaaagaaacgactagcagcgtaatttactgagtcaccagtccaggaacctagaactcgatggagagaggcctctgtccgatcatagcgtaggtagcgtttgaaaactaccttgccaaatccccaggactctttaaatcccagtgggttgtcctggttggagtttgtttcgtcattgtgtaaacgccattctgtccaagatgggctctcatcgggtaacttaaatgggctggtagtgccgccagaaccaccgtcccatctctctgaattggcctgctctcttgcatcattaccctggattgctctctccattgtcctctccaaatgaaatgaacttccttatatagaggaagggtcttgcgaaggatagtgggattgtgcgtcatcccttacgtcagtggagatgtcacatcaatccacttgctttgtagacgtggttggaacctcttctttttccacgatgctcctcgtgggtgggggtccatctttgggaccactgtcggcagagagatcttgaatgatagcctttcctttatcgcaatgatggcatttgtaggagccaccttccttttctactgtcctttcgatgaagtgacagatagctgggcaatggaatccgaggaggtttcccgaaattatcctttgttgaaaagtctcaaacaataggcaaccgtggacttcttcactagctcatcgagatagcaatgccactagctaatttcttacgttgtatcttatttgttttactttggggcatgacatggttaaaccccatcaaagagaaagtgtttcatccactagtcaatatacgaattcattcgaatttatccctgtaaatcctagttcttaggatgaactggtgtaataaacagcaaaaaaaaataaaaaaaaataaatctggaatcattcgaccacctcaataaactaaagctaccaattaccacaatatagtcatccatatccacttagatataaaagataaaagtaaacaaatattaaatttcatatgcacgcataggaaactcatgatcttatcttttaaatagacatctagttttcttaggttataaatagacattttgtcctagaacttcttcactactaaaacctagcctcaaaaagcaggctgccaccatggtgagcagtggtgaggacatcttttcaggcctagtcccgatacttattgaacttgaaggagacgtcaatgggcacagattctcagtacgaggcgagggatacggggatgcttccaatggaaagcttgagataaaatttatatgtacaactggaaggcttcctgtcccatggccaactttagttaccactcttagctacggtgtacaatgcttcgctaaatacccagaacatatgcgtcagaatgacttcttcaagtcagcaatgcctgatggatatgttcaagaaagaacaatctcttttaaagaggacggaacttataagaccagagctgaagtcaaattcgagggagaggccttggtgaacagaattgacttaaaaggactggaattcaaggaagatggcaatatcctcggtcacaagcttgaatacagttttaattcacactacgtgtatataaccgcggataagaacaggaatggtttagaagctcagtttagaataagacataacgtggacgatggatccgtgcagctagcagatcactatcagcaaaatacgccgataggggaaggccctgttcttttgccagagcagcattacctaactactaactctgttttgtctaaggacccacaagagcggagagatcatatggttttggttgagttcgttacggcagctggactctccctaggcatggatgaattatacaaatcaggatctgagaatttatattttcaaggtcaattgagttatggatacgacgaaaaatcaactggaatatcagtgccaggaccaatgggtccatcaggacctaggggtcttccagggccacctggcgctcctggtcctcagggatttcaaggtcctccaggtgaacctggagagcctggtgcttctggtccaatgggaccaagaggccctcctggtccacctggtaaaaatggtgatgatggtgaggctggaaagcctggtcgtcctggagaaagaggaccaccaggaccacagggagctagaggtttgccaggtacagccggtcttccaggaatgaaaggacacaggggtttttctggtcttgatggtgctaagggagacgcaggacctgctggaccaaagggtgaacctggatctcctggtgaaaatggtgctcctggacaaatgggacctagaggattgcctggcgaaagaggaagacctggtgctcctggaccagctggagctagaggaaatgatggagctactggtgctgccggaccaccaggaccaactggaccagctggaccacctggttttccaggagcagttggggctaagggagaaggtggaccacaaggacctagaggatcagaaggacctcaaggagttaggggagaaccaggtcctcctggtcctgctggagctgctggacccgctggtaacccaggagcagatggacaacctggagcaaaaggggctaatggtgctcctggtattgcaggtgctcctggattccctggtgctagaggaccttcaggacctcagggaccatccggtcctccaggaccaaagggaaactctggtgaaccaggggctcctggatctaagggagatactggagctaagggtgagccaggacctacaggaattcaaggaccaccaggacctgcaggagaggaaggtaagaggggtgctagaggtgaacctggaccagctggattgccaggcccacctggagagaggggtggtccaggttctagaggttttccaggagctgatggagttgctggtccaaagggtcctgctggtgagagaggtgcacctggaccagcaggacctaaaggatcacctggagaagctggtcgtcctggtgaggctggtcttccaggtgctaagggccttacaggatctccaggatcaccaggtccagatggaaagactggaccaccaggtcctgcaggacaagatggaaggcctggtccacctggaccacctggtgctaggggacaagctggtgttatgggattcccaggtccaaagggtgcagctggtgagcctggtaaagctggtgaaagaggagttccaggacctcctggtgctgttggacctgctggtaaagatggtgaagcaggtgctcagggtccaccaggtccagccggtccagctggtgagaggggagagcaaggtcctgctggatctcctggatttcaaggtttgcctggacctgctggacctccaggagaggctggtaaacctggtgagcagggtgtgcctggtgatcttggtgctcctggacctagtggcgcaagaggcgaaaggggatttccaggtgaaagaggagttcagggaccaccaggtccagctggtccaagaggcgctaatggagctccaggaaatgatggagcaaagggtgatgctggcgctccaggagctcctggttctcaaggtgcacctggattgcaaggaatgccaggagagagaggtgcagctggtttgccgggaccaaagggtgatagaggtgatgctggtcctaagggagctgatggagctccaggaaaggatggtgtgagaggattgactggtccaattggaccaccaggtcctgctggagcaccaggagataaaggagaagctggtccttcaggaccagccggtccaactggagctagaggagctccaggagatagaggtgaaccaggaccaccaggacctgctgggtttgcaggtccacctggtgctgatggacaacctggtgctaaaggagaaccaggcgatgctggtgctaagggagatgctggcccacctggtccagctggtcctgctgggccaccaggtcctatcggaaatgttggtgctccagggcctaaaggagctagaggatcagcaggtcccccaggtgctacaggttttccaggggctgctggaagagtgggtcccccaggtccttctgggaatgcaggaccaccaggtcctccaggaccagctggaaaagaaggaagtaagggaccaaggggagaaactggacctgcaggacgtccaggtgaagttggtccacctggacctccaggtccagctggagagaaaggagctccaggagctgatggtccagcaggtgctcctggtactccaggtccacaaggtattgctggtcaaaggggagtggttggtctcccaggtcagagaggtgaaagaggtttcccaggtttgcctggaccatctggagaaccaggtaagcagggcccatctggagcttctggtgagagagggccacctggacctatgggacctcctgggcttgctggacctccaggggaatctggtagggagggtgctccaggtgctgaaggatcacctggtagagatggatcacctggagctaaaggtgatagaggggaaacaggtccagcaggtccacctggcgctcctggtgctccaggagcaccagggccagttggacctgctggaaagtctggagataggggagagactggaccagctggacctgctggaccaatcggtcctgttggcgctagaggtcctgctggaccacaaggtcctaggggagataaaggtgaaacaggtgaacaaggagatagaggaattaaaggtcatagagggttttctggtttgcaaggacctccaggacctcctggatctccaggagagcaaggaccatctggtgcaagcggacctgctggtcctagaggacctccaggttcagctggctcacctggtaaggatggattaaatggtttgcctggaccaataggtccaccaggacctagaggaaggacaggtgatgcaggaccagctggtccacctggtccaccaggaccaccaggaccaccaggtccaccttctggtggatatgatcttagttttcttcctcaacctccccaggagaaagctcatgatggtggtagatattatagggcttaaacccagctttcttgtacaaagtggtagctcgaatttccccgatcgttcaaacatttggcaataaagtttcttaagattgaatcctgttgccggtcttgcgatgattatcatataatttctgttgaattacgttaagcatgtaataattaacatgtaatgcatgacgttatttatgagatgggtttttatgattagagtcccgcaattatacatttaatacgcgatagaaaacaaaatatagcgcgcaaactaggataaattatcgcgcgcggtgtcatctatgttactagatcgggaaagcttttaaactatcagtgtttgacaggatatattggcgggtaaacctaagagaaaagagcgtttattagaataatcggatatttaaaagggcgtgaaaaggtttatccgttcgtccatttgtatgtgcatgccaaccacagggttcccctcgggatcaaagtactttgatccaacccctccgctgctatagtgcagtcggcttctgacgttcagtgcagccgtcttctgaaaacgacatgtcgcacaagtcctaagttacgcgacaggctgccgccctgcccttttcctggcgttttcttgtcgcgtgttttagtcgcataaagtagaatacttgcgactagaaccggagacattacgccatgaacaagagcgccgccgctggcctgctgggctatgcccgcgtcagcaccgacgaccaggacttgaccaaccaacgggccgaactgcacgcggccggctgcaccaagctgttttccgagaagatcaccggcaccaggcgcgaccgcccggagctggccaggatgcttgaccacctacgccctggcgacgttgtgacagtgaccaggctagaccgcctggcccgcagcacccgcgacctactggacattgccgagcgcatccaggaggccggcgcgggcctgcgtagcctggcagagccgtgggccgacaccaccacgccggccggccgcatggtgttgaccgtgttcgccggcattgccgagttcgagcgttccctaatcatcgaccgcacccggagcgggcgcgaggccgccaaggcccgaggcgtgaagtttggcccccgccctaccctcaccccggcacagatcgcgcacgcccgcgagctgatcgaccaggaaggccgcaccgtgaaagaggcggctgcactgcttggcgtgcatcgctcgaccctgtaccgcgcacttgagcgcagcgaggaagtgacgcccaccgaggccaggcggcgcggtgccttccgtgaggacgcattgaccgaggccgacgccctggcggccgccgagaatgaacgccaagaggaacaagcatgaaaccgcaccaggacggccaggacgaaccgtttttcattaccgaagagatcgaggcggagatgatcgcggccgggtacgtgttcgagccgcccgcgcacgtctcaaccgtgcggctgcatgaaatcctggccggtttgtctgatgccaagctggcggcctggccggccagcttggccgctgaagaaaccgagcgccgccgtctaaaaaggtgatgtgtatttgagtaaaacagcttgcgtcatgcggtcgctgcgtatatgatgcgatgagtaaataaacaaatacgcaaggggaacgcatgaaggttatcgctgtacttaaccagaaaggcgggtcaggcaagacgaccatcgcaacccatctagcccgcgccctgcaactcgccggggccgatgttctgttagtcgattccgatccccagggcagtgcccgcgattgggcggccgtgcgggaagatcaaccgctaaccgttgtcggcatcgaccgcccgacgattgaccgcgacgtgaaggccatcggccggcgcgacttcgtagtgatcgacggagcgccccaggcggcggacttggctgtgtccgcgatcaaggcagccgacttcgtgctgattccggtgcagccaagcccttacgacatatgggccaccgccgacctggtggagctggttaagcagcgcattgaggtcacggatggaaggctacaagcggcctttgtcgtgtcgcgggcgatcaaaggcacgcgcatcggcggtgaggttgccgaggcgctggccgggtacgagctgcccattcttgagtcccgtatcacgcagcgcgtgagctacccaggcactgccgccgccggcacaaccgttcttgaatcagaacccgagggcgacgctgcccgcgaggtccaggcgctggccgctgaaattaaatcaaaactcatttgagttaatgaggtaaagagaaaatgagcaaaagcacaaacacgctaagtgccggccgtccgagcgcacgcagcagcaaggctgcaacgttggccagcctggcagacacgccagccatgaagcgggtcaactttcagttgccggcggaggatcacaccaagctgaagatgtacgcggtacgccaaggcaagaccattaccgagctgctatctgaatacatcgcgcagctaccagagtaaatgagcaaatgaataaatgagtagatgaattttagcggctaaaggaggcggcatggaaaatcaagaacaaccaggcaccgacgccgtggaatgccccatgtgtggaggaacgggcggttggccaggcgtaagcggctgggttgcctgccggccctgcaatggcactggaacccccaagcccgaggaatcggcgtgagcggtcgcaaaccatccggcccggtacaaatcggcgcggcgctgggtgatgacctggtggagaagttgaaggccgcgcaggccgcccagcggcaacgcatcgaggcagaagcacgccccggtgaatcgtggcaagcggccgctgatcgaatccgcaaagaatcccggcaaccgccggcagccggtgcgccgtcgattaggaagccgcccaagggcgacgagcaaccagattttttcgttccgatgctctatgacgtgggcacccgcgatagtcgcagcatcatggacgtggccgttttccgtctgtcgaagcgtgaccgacgagctggcgaggtgatccgctacgagcttccagacgggcacgtagaggtttccgcagggccggccggcatggccagtgtgtgggattacgacctggtactgatggcggtttcccatctaaccgaatccatgaaccgataccgggaagggaagggagacaagcccggccgcgtgttccgtccacacgttgcggacgtactcaagttctgccggcgagccgatggcggaaagcagaaagacgacctggtagaaacctgcattcggttaaacaccacgcacgttgccatgcagcgtacgaagaaggccaagaacggccgcctggtgacggtatccgagggtgaagccttgattagccgctacaagatcgtaaagagcgaaaccgggcggccggagtacatcgagatcgagctagctgattggatgtaccgcgagatcacagaaggcaagaacccggacgtgctgacggttcaccccgattactttttgatcgatcccggcatcggccgttttctctaccgcctggcacgccgcgccgcaggcaaggcagaagccagatggttgttcaagacgatctacgaacgcagtggcagcgccggagagttcaagaagttctgtttcaccgtgcgcaagctgatcgggtcaaatgacctgccggagtacgatttgaaggaggaggcggggcaggctggcccgatcctagtcatgcgctaccgcaacctgatcgagggcgaagcatccgccggttcctaatgtacggagcagatgctagggcaaattgccctagcaggggaaaaaggtcgaaaaggtctctttcctgtggatagcacgtacattgggaacccaaagccgtacattgggaaccggaacccgtacattgggaacccaaagccgtacattgggaaccggtcacacatgtaagtgactgatataaaagagaaaaaaggcgatttttccgcctaaaactctttaaaacttattaaaactcttaaaacccgcctggcctgtgcataactgtctggccagcgcacagccgaagagctgcaaaaagcgcctacccttcggtcgctgcgctccctacgccccgccgcttcgcgtcggcctatcgcggccgctggccgctcaaaaatggctggcctacggccaggcaatctaccagggcgcggacaagccgcgccgtcgccactcgaccgccggcgcccacatcaaggcaccctgcctcgcgcgtttcggtgatgacggtgaaaacctctgacacatgcagctcccggagacggtcacagcttgtctgtaagcggatgccgggagcagacaagcccgtcagggcgcgtcagcgggtgttggcgggtgtcggggcgcagccatgacccagtcacgtagcgatagcggagtgtatactggcttaactatgcggcatcagagcagattgtactgagagtgcaccatatgcggtgtgaaataccgcacagatgcgtaaggagaaaataccgcatcaggcgctcttccgcttcctcgctcactgactcgctgcgctcggtcgttcggctgcggcgagcggtatcagctcactcaaaggcggtaatacggttatccacagaatcaggggataacgcaggaaagaacatgtgagcaaaaggccagcaaa

SEQ ID NO: 22 - protein, 1305 aa, synthetic construct
MVSSGEDIFSGLVPILIELEGDVNGHRFSVRGEGYGDASNGKLEIKFICTTGRLPVPWPTLVTTLSYGVQCFAKYPEHMRQNDFFKSAMPDGYVQERTISFKEDGTYKTRAEVKFEGEALVNRIDLKGLEFKEDGNILGHKLEYSFNSHYVYITADKNRNGLEAQFRIRHNVDDGSVQLADHYQQNTPIGEGPVLLPEQHYLTTNSVLSKDPQERRDHMVLVEFVTAAGLSLGMDELYKSGSENLYFQGQLSYGYDEKSTGISVPGPMGPSGPRGLPGPPGAPGPQGFQGPPGEPGEPGASGPMGPRGPPGPPGKNGDDGEAGKPGRPGERGPPGPQGARGLPGTAGLPGMKGHRGFSGLDGAKGDAGPAGPKGEPGSPGENGAPGQMGPRGLPGERGRPGAPGPAGARGNDGATGAAGPPGPTGPAGPPGFPGAVGAKGEGGPQGPRGSEGPQGVRGEPGPPGPAGAAGPAGNPGADGQPGAKGANGAPGIAGAPGFPGARGPSGPQGPSGPPGPKGNSGEPGAPGSKGDTGAKGEPGPTGIQGPPGPAGEEGKRGARGEPGPAGLPGPPGERGGPGSRGFPGADGVAGPKGPAGERGAPGPAGPKGSPGEAGRPGEAGLPGAKGLTGSPGSPGPDGKTGPPGPAGQDGRPGPPGPPGARGQAGVMGFPGPKGAAGEPGKAGERGVPGPPGAVGPAGKDGEAGAQGPPGPAGPAGERGEQGPAGSPGFQGLPGPAGPPGEAGKPGEQGVPGDLGAPGPSGARGERGFPGERGVQGPPGPAGPRGANGAPGNDGAKGDAGAPGAPGSQGAPGLQGMPGERGAAGLPGPKGDRGDAGPKGADGAPGKDGVRGLTGPIGPPGPAGAPGDKGEAGPSGPAGPTGARGAPGDRGEPGPPGPAGFAGPPGADGQPGAKGEPGDAGAKGDAGPPGPAGPAGPPGPIGNVGAPGPKGARGSAGPPGATGFPGAAGRVGPPGPSGNAGPPGPPGPAGKEGSKGPRGETGPAGRPGEVGPPGPPGPAGEKGAPGADGPAGAPGTPGPQGIAGQRGVVGLPGQRGERGFPGLPGPSGEPGKQGPSGASGERGPPGPMGPPGLAGPPGESGREGAPGAEGSPGRDGSPGAKGDRGETGPAGPPGAPGAPGAPGPVGPAGKSGDRGETGPAGPAGPIGPVGARGPAGPQGPRGDKGETGEQGDRGIKGHRGFSGLQGPPGPPGSPGEQGPSGASGPAGPRGPPGSAGSPGKDGLNGLPGPIGPPGPRGRTGDAGPAGPPGPPGPPGPPGPPSGGYDLSFLPQPPQEKAHDGGRYYRA

SEQ ID NO: 23 - protein, 239 aa, synthetic construct; identical to SEQ ID NO: 17

SEQ ID NO: 24 - protein, 1056 aa, synthetic construct; identical to SEQ ID NO: 2

SEQ ID NO: 25 - DNA, 12157 bp, synthetic construct
  source 1..12157: mol_type = other DNA
  misc_feature 1932..1956: function = plasmid transfer to host cells; note = LB T-DNA repeat
  regulatory 2040..2737: note = p19 Suppressor; regulatory_class = other
  regulatory 2738..3083: note = p35S_short; regulatory_class = promoter
  regulatory 3088..3543: note = pPD7; regulatory_class = promoter
  CDS 3560..7489: note = fuGFP-Col1a; protein_id = 26; translation = MVSSGEDIFSGLVPILIELEGDVNGHRFSVRGEGYGDASNGKLEIKFICTTGRLPVPWPTLVTTLSYGVQCFAKYPEHMRQNDFFKSAMPDGYVQERTISFKEDGTYKTRAEVKFEGEALVNRIDLKGLEFKEDGNILGHKLEYSFNSHYVYITADKNRNGLEAQFRIRHNVDDGSVQLADHYQQNTPIGEGPVLLPEQHYLTTNSVLSKDPQERRDHMVLVEFVTAAGLSLGMDELYKSGSENLYFQGQLSYGYDEKSTGISVPGPMGPSGPRGLPGPPGAPGPQGFQGPPGEPGEPGASGPMGPRGPPGPPGKNGDDGEAGKPGRPGERGPPGPQGARGLPGTAGLPGMKGHRGFSGLDGAKGDAGPAGPKGEPGSPGENGAPGQMGPRGLPGERGRPGAPGPAGARGNDGATGAAGPPGPTGPAGPPGFPGAVGAKGEGGPQGPRGSEGPQGVRGEPGPPGPAGAAGPAGNPGADGQPGAKGANGAPGIAGAPGFPGARGPSGPQGPSGPPGPKGNSGEPGAPGSKGDTGAKGEPGPTGIQGPPGPAGEEGKRGARGEPGPAGLPGPPGERGGPGSRGFPGADGVAGPKGPAGERGAPGPAGPKGSPGEAGRPGEAGLPGAKGLTGSPGSPGPDGKTGPPGPAGQDGRPGPPGPPGARGQAGVMGFPGPKGAAGEPGKAGERGVPGPPGAVGPAGKDGEAGAQGPPGPAGPAGERGEQGPAGSPGFQGLPGPAGPPGEAGKPGEQGVPGDLGAPGPSGARGERGFPGERGVQGPPGPAGPRGANGAPGNDGAKGDAGAPGAPGSQGAPGLQGMPGERGAAGLPGPKGDRGDAGPKGADGAPGKDGVRGLTGPIGPPGPAGAPGDKGEAGPSGPAGPTGARGAPGDRGEPGPPGPAGFAGPPGADGQPGAKGEPGDAGAKGDAGPPGPAGPAGPPGPIGNVGAPGPKGARGSAGPPGATGFPGAAGRVGPPGPSGNAGPPGPPGPAGKEGSKGPRGETGPAGRPGEVGPPGPPGPAGEKGAPGADGPAGAPGTPGPQGIAGQRGVVGLPGQRGERGFPGLPGPSGEPGKQGPSGASGERGPPGPMGPPGLAGPPGESGREGAPGAEGSPGRDGSPGAKGDRGETGPAGPPGAPGAPGAPGPVGPAGKSGDRGETGPAGPAGPIGPVGARGPAGPQGPRGDKGETGEQGDRGIKGHRGFSGLQGPPGPPGSPGEQGPSGASGPAGPRGPPGSAGSPGKDGLNGLPGPIGPPGPRGRTGDAGPAGPPGPPGPPGPPGPPSGGYDLSFLPQPPQEKAHDGGRYYRAKDEL
  CDS 3563..4279: gene = fuGFP codon opt. N. tabacum; protein_id = 27; translation = VSSGEDIFSGLVPILIELEGDVNGHRFSVRGEGYGDASNGKLEIKFICTTGRLPVPWPTLVTTLSYGVQCFAKYPEHMRQNDFFKSAMPDGYVQERTISFKEDGTYKTRAEVKFEGEALVNRIDLKGLEFKEDGNILGHKLEYSFNSHYVYITADKNRNGLEAQFRIRHNVDDGSVQLADHYQQNTPIGEGPVLLPEQHYLTTNSVLSKDPQERRDHMVLVEFVTAAGLSLGMDELYKS
  misc_feature 4286..4303: function = TEV cleavage site
  CDS 4307..7474: gene = Collagen alpha-1(I) chain; protein_id = 28; translation = QLSYGYDEKSTGISVPGPMGPSGPRGLPGPPGAPGPQGFQGPPGEPGEPGASGPMGPRGPPGPPGKNGDDGEAGKPGRPGERGPPGPQGARGLPGTAGLPGMKGHRGFSGLDGAKGDAGPAGPKGEPGSPGENGAPGQMGPRGLPGERGRPGAPGPAGARGNDGATGAAGPPGPTGPAGPPGFPGAVGAKGEGGPQGPRGSEGPQGVRGEPGPPGPAGAAGPAGNPGADGQPGAKGANGAPGIAGAPGFPGARGPSGPQGPSGPPGPKGNSGEPGAPGSKGDTGAKGEPGPTGIQGPPGPAGEEGKRGARGEPGPAGLPGPPGERGGPGSRGFPGADGVAGPKGPAGERGAPGPAGPKGSPGEAGRPGEAGLPGAKGLTGSPGSPGPDGKTGPPGPAGQDGRPGPPGPPGARGQAGVMGFPGPKGAAGEPGKAGERGVPGPPGAVGPAGKDGEAGAQGPPGPAGPAGERGEQGPAGSPGFQGLPGPAGPPGEAGKPGEQGVPGDLGAPGPSGARGERGFPGERGVQGPPGPAGPRGANGAPGNDGAKGDAGAPGAPGSQGAPGLQGMPGERGAAGLPGPKGDRGDAGPKGADGAPGKDGVRGLTGPIGPPGPAGAPGDKGEAGPSGPAGPTGARGAPGDRGEPGPPGPAGFAGPPGADGQPGAKGEPGDAGAKGDAGPPGPAGPAGPPGPIGNVGAPGPKGARGSAGPPGATGFPGAAGRVGPPGPSGNAGPPGPPGPAGKEGSKGPRGETGPAGRPGEVGPPGPPGPAGEKGAPGADGPAGAPGTPGPQGIAGQRGVVGLPGQRGERGFPGLPGPSGEPGKQGPSGASGERGPPGPMGPPGLAGPPGESGREGAPGAEGSPGRDGSPGAKGDRGETGPAGPPGAPGAPGAPGPVGPAGKSGDRGETGPAGPAGPIGPVGARGPAGPQGPRGDKGETGEQGDRGIKGHRGFSGLQGPPGPPGSPGEQGPSGASGPAGPRGPPGSAGSPGKDGLNGLPGPIGPPGPRGRTGDAGPAGPPGPPGPPGPPGPPSGGYDLSFLPQPPQEKAHDGGRYYRA
  sig_peptide 7475..7486: function = ER-retention signal
  regulatory 7530..7783: note = Nos pA; regulatory_class = polyA_signal_sequence; regulatory_class = terminator
  misc_feature 7809..7833: function = plasmid transfer to host cells; note = RB T-DNA repeat
aggccaggaaccgtaaaaaggccgcgttgctggcgtttttccataggctccgcccccctgacgagcatcacaaaaatcgacgctcaagtcagaggtggcgaaacccgacaggactataaagataccaggcgtttccccctggaagctccctcgtgcgctctcctgttccgaccctgccgcttaccggatacctgtccgcctttctcccttcgggaagcgtggcgctttctcatagctcacgctgtaggtatctcagttcggtgtaggtcgttcgctccaagctgggctgtgtgcacgaaccccccgttcagcccgaccgctgcgccttatccggtaactatcgtcttgagtccaacccggtaagacacgacttatcgccactggcagcagccactggtaacaggattagcagagcgaggtatgtaggcggtgctacagagttcttgaagtggtggcctaactacggctacactagaaggacagtatttggtatctgcgctctgctgaagccagttaccttcggaaaaagagttggtagctcttgatccggcaaacaaaccaccgctggtagcggtggtttttttgtttgcaagcagcagattacgcgcagaaaaaaaggatctcaagaagatcctttgatcttttctacggggtctgacgctcagtggaacgaaaactcacgttaagggattttggtcatgcattctaggtactaaaacaattcatccagtaaaatataatattttattttctcccaatcaggcttgatccccagtaagtcaaaaaatagctcgacatactgttcttccccgatatcctccctgatcgaccggacgcagaaggcaatgtcataccacttgtccgccctgccgcttctcccaagatcaataaagccacttactttgccatctttcacaaagatgttgctgtctcccaggtcgccgtgggaaaagacaagttcctcttcgggcttttccgtctttaaaaaatcatacagctcgcgcggatctttaaatggagtgtcttcttcccagttttcgcaatccacatcggccagatcgttattcagtaagtaatccaattcggctaagcggctgtctaagctattcgtatagggacaatccgatatgtcgatggagtgaaagagcctgatgcactccgcatacagctcgataatcttttcagggctttgttcatcttcatactcttccgagcaaaggacgccatcggcctcactcatgagcagattgctccagccatcatgccgttcaaagtgcaggacctttggaacaggcagctttccttccagccatagcatcatgtccttttcccgttccacatcataggtggtccctttataccggctgtccgtcatttttaaatataggttttcattttctcccaccagcttatataccttagcaggagacattccttccgtatcttttacgcagcggtatttttcgatcagttttttcaattccggtgatattctcattttagccatttattatttccttcctcttttctacagtatttaaagataccccaagaagctaattataacaagacgaactccaattcactgttccttgcattctaaaaccttaaataccagaaaacagctttttcaaagttgttttcaaagttggcgtataacatagtatcgacggagccgattttgaaaccgcggtgatcacaggcagcaacgctctgtcatcgttacaatcaacatgctaccctccgcgagatcatccgtgtttcaaacccggcagcttagttgccgttcttccgaatagcatcggtaacatgagcaaagtctgccgccttacaacggctctcccgctgacgccgtcccggactgatgggctgcctgtatcgagtggtgattttgtgccgagctgccggtcggggagctgttggctggctggtggcaggatatattgtggtgtaaacaaattgacgcttagacaacttaataacacattgcggacgtttttaatgtactgaattaacgccgaattgaattcgagctcggtggaggatctggattttagtactggattttggttttaggaattagaaattttattgatagaagtattttacaaatacaaatacatactaagggtttcttatatgctcaacacatgagcgaaaccctataggaaccctaattcccttatctgggaactactcacacattattatggagaaactattcactctccttctcaaacgtttctgttccctctggacagccccgactgacgttggactcaacctcaatgggcgctaattgtaatagctcctgtttgcttcttatggccatttcgcaaaggtgttgcagtgttctgctaccaccactcactgtaattgacacacctctgaaacggatggagtaagtgcaaccaatttgatcaaatccaaagaaacgactagcagcgtaatttactgagtcaccagtccaggaacctagaactcgatggagagaggcctctgtccgatcatagcgtaggtagcgtttgaaaactaccttgccaaatccccaggactctttaaatcccagtgggttgtcctggttggagtttgtttcgtcattgtgtaaacgccattctgtccaagatgggctctcatcgggtaacttaaatgggctggtagtgccgccagaaccaccgtcccatctctctgaattggcctgctctcttgcatcattaccctggattgctctctccattgtcctctccaaatgaaatgaacttccttatatagaggaagggtcttgcgaaggatagtgggattgtgcgtcatcccttacgtcagtggagatgtcacatcaatccacttgctttgtagacgtggttggaacctcttctttttccacgatgctcctcgtgggtgggggtccatctttgggaccactgtcggcagagagatcttgaatgatagcctttcctttatcgcaatgatggcatttgtaggagccaccttccttttctactgtcctttcgatgaagtgacagatagctgggcaatggaatccgaggaggtttcccgaaattatcctttgttgaaaagtctcaaacaataggcaaccgtggacttcttcactagctcatcgagatagcaatgccactagctaatttcttacgttgtatcttatttgttttactttggggcatgacatggttaaaccccatcaaagagaaagtgtttcatccactagtcaatatacgaattcattcgaatttatccctgtaaatcctagttcttaggatgaactggtgtaataaacagcaaaaaaaaataaaaaaaaataaatctggaatcattcgaccacctcaataaactaaagctaccaattaccacaatatagtcatccatatccacttagatataaaagataaaagtaaacaaatattaaatttcatatgcacgcataggaaactcatgatcttatcttttaaatagacatctagttttcttaggttataaatagacattttgtcctagaacttcttcactactaaaacctagcctcaaaaagcaggctgccaccatggtgagcagtggtgaggacatcttttcaggcctagtcccgatacttattgaacttgaaggagacgtcaatgggcacagattctcagtacgaggcgagggatacggggatgcttccaatggaaagcttgagataaaatttatatgtacaactggaaggcttcctgtcccatggccaactttagttaccactcttagctacggtgtacaatgcttcgctaaatacccagaacatatgcgtcagaatgacttcttcaagtcagcaatgcctgatggatatgttcaagaaagaacaatctcttttaaagaggacggaacttataagaccagagctgaagtcaaattcgagggagaggccttggtgaacagaattgacttaaaaggactggaattcaaggaagatggcaatatcctcggtcacaagcttgaatacagttttaattcacactacgtgtatataaccgcggataagaacaggaatggtttagaagctcagtttagaataagacataacgtggacgatggatccgtgcagctagcagatcactatcagcaaaatacgccgataggggaaggccctgttcttttgccagagcagcattacctaactactaactctgttttgtctaaggacccacaagagcggagagatcatatggttttggttgagttcgttacggcagctggactctccctaggcatggatgaattatacaaatcaggatctgagaatttatattttcaaggtcaattgagttatggatacgacgaaaaatcaactggaatatcagtgccaggaccaatgggtccatcaggacctaggggtcttccagggccacctggcgctcctggtcctcagggatttcaaggtcctccaggtgaacctggagagcctggtgcttctggtccaatgggaccaagaggccctcctggtccacctggtaaaaatggtgatgatggtgaggctggaaagcctggtcgtcctggagaaagaggaccaccaggaccacagggagctagaggtttgccaggtacagccggtcttccaggaatgaaaggacacaggggtttttctggtcttgatggtgctaagggagacgcaggacctgctggaccaaagggtgaacctggatctcctggtgaaaatggtgctcctggacaaatgggacctagaggattgcctggcgaaagaggaagacctggtgctcctggaccagctggagctagaggaaatgatggagctactggtgctgccggaccaccaggaccaactggaccagctggaccacctggttttccaggagcagttggggctaagggagaaggtggaccacaaggacctagaggatcagaaggacctcaaggagttaggggagaaccaggtcctcctggtcctgctggagctgctggacccgctggtaacccaggagcagatggacaacctggagcaaaaggggctaatggtgctcctggtattgcaggtgctcctggattccctggtgctagaggaccttcaggacctcagggaccatccggtcctccaggaccaaagggaaactctggtgaaccaggggctcctggatctaagggagatactggagctaagggtgagccaggacctacaggaattcaaggaccaccaggacctgcaggagaggaaggtaagaggggtgctagaggtgaacctggaccagctggattgccaggcccacctggagagaggggtggtccaggttctagaggttttccaggagctgatggagttgctggtccaaagggtcctgctggtgagagaggtgcacctggaccagcaggacctaaaggatcacctggagaagctggtcgtcctggtgaggctggtcttccaggtgctaagggccttacaggatctccaggatcaccaggtccagatggaaagactggaccaccaggtcctgcaggacaagatggaaggcctggtccacctggaccacctggtgctaggggacaagctggtgttatgggattcccaggtccaaagggtgcagctggtgagcctggtaaagctggtgaaagaggagttccaggacctcctggtgctgttggacctgctggtaaagatggtgaagcaggtgctcagggtccaccaggtccagccggtccagctggtgagaggggagagcaaggtcctgctggatctcctggatttcaaggtttgcctggacctgctggacctccaggagaggctggtaaacctggtgagcagggtgtgcctggtgatcttggtgctcctggacctagtggcgcaagaggcgaaaggggatttccaggtgaaagaggagttcagggaccaccaggtccagctggtccaagaggcgctaatggagctccaggaaatgatggagcaaagggtgatgctggcgctccaggagctcctggttctcaaggtgcacctggattgcaaggaatgccaggagagagaggtgcagctggtttgccgggaccaaagggtgatagaggtgatgctggtcctaagggagctgatggagctccaggaaaggatggtgtgagaggattgactggtccaattggaccaccaggtcctgctggagcaccaggagataaaggagaagctggtccttcaggaccagccggtccaactggagctagaggagctccaggagatagaggtgaaccaggaccaccaggacctgctgggtttgcaggtccacctggtgctgatggacaacctggtgctaaaggagaaccaggcgatgctggtgctaagggagatgctggcccacctggtccagctggtcctgctgggccaccaggtcctatcggaaatgttggtgctccagggcctaaaggagctagaggatcagcaggtcccccaggtgctacaggttttccaggggctgctggaagagtgggtcccccaggtccttctgggaatgcaggaccaccaggtcctccaggaccagctggaaaagaaggaagtaagggaccaaggggagaaactggacctgcaggacgtccaggtgaagttggtccacctggacctccaggtccagctggagagaaaggagctccaggagctgatggtccagcaggtgctcctggtactccaggtccacaaggtattgctggtcaaaggggagtggttggtctcccaggtcagagaggtgaaagaggtttcccaggtttgcctggaccatctggagaaccaggtaagcagggcccatctggagcttctggtgagagagggccacctggacctatgggacctcctgggcttgctggacctccaggggaatctggtagggagggtgctccaggtgctgaaggatcacctggtagagatggatcacctggagctaaaggtgatagaggggaaacaggtccagcaggtccacctggcgctcctggtgctccaggagcaccagggccagttggacctgctggaaagtctggagataggggagagactggaccagctggacctgctggaccaatcggtcctgttggcgctagaggtcctgctggaccacaaggtcctaggggagataaaggtgaaacaggtgaacaaggagatagaggaattaaaggtcatagagggttttctggtttgcaaggacctccaggacctcctggatctccaggagagcaaggaccatctggtgcaagcggacctgctggtcctagaggacctccaggttcagctggctcacctggtaaggatggattaaatggtttgcctggaccaataggtccaccaggacctagaggaaggacaggtgatgcaggaccagctggtccacctggtccaccaggaccaccaggaccaccaggtccaccttctggtggatatgatcttagttttcttcctcaacctccccaggagaaagctcatgatggtggtagatattatagggctaaggatgagctttaaacccagctttcttgtacaaagtggtagctcgaatttccccgatcgttcaaacatttggcaataaagtttcttaagattgaatcctgttgccggtcttgcgatgattatcatataatttctgttgaattacgttaagcatgtaataattaacatgtaatgcatgacgttatttatgagatgggtttttatgattagagtcccgcaattatacatttaatacgcgatagaaaacaaaatatagcgcgcaaactaggataaattatcgcgcgcggtgtcatctatgttactagatcgggaaagcttttaaactatcagtgtttgacaggatatattggcgggtaaacctaagagaaaagagcgtttattagaataatcggatatttaaaagggcgtgaaaaggtttatccgttcgtccatttgtatgtgcatgccaaccacagggttcccctcgggatcaaagtactttgatccaacccctccgctgctatagtgcagtcggcttctgacgttcagtgcagccgtcttctgaaaacgacatgtcgcacaagtcctaagttacgcgacaggctgccgccctgcccttttcctggcgttttcttgtcgcgtgttttagtcgcataaagtagaatacttgcgactagaaccggagacattacgccatgaacaagagcgccgccgctggcctgctgggctatgcccgcgtcagcaccgacgaccaggacttgaccaaccaacgggccgaactgcacgcggccggctgcaccaagctgttttccgagaagatcaccggcaccaggcgcgaccgcccggagctggccaggatgcttgaccacctacgccctggcgacgttgtgacagtgaccaggctagaccgcctggcccgcagcacccgcgacctactggacattgccgagcgcatccaggaggccggcgcgggcctgcgtagcctggcagagccgtgggccgacaccaccacgccggccggccgcatggtgttgaccgtgttcgccggcattgccgagttcgagcgttccctaatcatcgaccgcacccggagcgggcgcgaggccgccaaggcccgaggcgtgaagtttggcccccgccctaccctcaccccggcacagatcgcgcacgcccgcgagctgatcgaccaggaaggccgcaccgtgaaagaggcggctgcactgcttggcgtgcatcgctcgaccctgtaccgcgcacttgagcgcagcgaggaagtgacgcccaccgaggccaggcggcgcggtgccttccgtgaggacgcattgaccgaggccgacgccctggcggccgccgagaatgaacgccaagaggaacaagcatgaaaccgcaccaggacggccaggacgaaccgtttttcattaccgaagagatcgaggcggagatgatcgcggccgggtacgtgttcgagccgcccgcgcacgtctcaaccgtgcggctgcatgaaatcctggccggtttgtctgatgccaagctggcggcctggccggccagcttggccgctgaagaaaccgagcgccgccgtctaaaaaggtgatgtgtatttgagtaaaacagcttgcgtcatgcggtcgctgcgtatatgatgcgatgagtaaataaacaaatacgcaaggggaacgcatgaaggttatcgctgtacttaaccagaaaggcgggtcaggcaagacgaccatcgcaacccatctagcccgcgccctgcaactcgccggggccgatgttctgttagtcgattccgatccccagggcagtgcccgcgattgggcggccgtgcgggaagatcaaccgctaaccgttgtcggcatcgaccgcccgacgattgaccgcgacgtgaaggccatcggccggcgcgacttcgtagtgatcgacggagcgccccaggcggcggacttggctgtgtccgcgatcaaggcagccgacttcgtgctgattccggtgcagccaagcccttacgacatatgggccaccgccgacctggtggagctggttaagcagcgcattgaggtcacggatggaaggctacaagcggcctttgtcgtgtcgcgggcgatcaaaggcacgcgcatcggcggtgaggttgccgaggcgctggccgggtacgagctgcccattcttgagtcccgtatcacgcagcgcgtgagctacccaggcactgccgccgccggcacaaccgttcttgaatcagaacccgagggcgacgctgcccgcgaggtccaggcgctggccgctgaaattaaatcaaaactcatttgagttaatgaggtaaagagaaaatgagcaaaagcacaaacacgctaagtgccggccgtccgagcgcacgcagcagcaaggctgcaacgttggccagcctggcagacacgccagccatgaagcgggtcaactttcagttgccggcggaggatcacaccaagctgaagatgtacgcggtacgccaaggcaagaccattaccgagctgctatctgaatacatcgcgcagctaccagagtaaatgagcaaatgaataaatgagtagatgaattttagcggctaaaggaggcggcatggaaaatcaagaacaaccaggcaccgacgccgtggaatgccccatgtgtggaggaacgggcggttggccaggcgtaagcggctgggttgcctgccggccctgcaatggcactggaacccccaagcccgaggaatcggcgtgagcggtcgcaaaccatccggcccggtacaaatcggcgcggcgctgggtgatgacctggtggagaagttgaaggccgcgcaggccgcccagcggcaacgcatcgaggcagaagcacgccccggtgaatcgtggcaagcggccgctgatcgaatccgcaaagaatcccggcaaccgccggcagccggtgcgccgtcgattaggaagccgcccaagggcgacgagcaaccagattttttcgttccgatgctctatgacgtgggcacccgcgatagtcgcagcatcatggacgtggccgttttccgtctgtcgaagcgtgaccgacgagctggcgaggtgatccgctacgagcttccagacgggcacgtagaggtttccgcagggccggccggcatggccagtgtgtgggattacgacctggtactgatggcggtttcccatctaaccgaatccatgaaccgataccgggaagggaagggagacaagcccggccgcgtgttccgtccacacgttgcggacgtactcaagttctgccggcgagccgatggcggaaagcagaaagacgacctggtagaaacctgcattcggttaaacaccacgcacgttgccatgcagcgtacgaagaaggccaagaacggccgcctggtgacggtatccgagggtgaagccttgattagccgctacaagatcgtaaagagcgaaaccgggcggccggagtacatcgagatcgagctagctgattggatgtaccgcgagatcacagaaggcaagaacccggacgtgctgacggttcaccccgattactttttgatcgatcccggcatcggccgttttctctaccgcctggcacgccgcgccgcaggcaaggcagaagccagatggttgttcaagacgatctacgaacgcagtggcagcgccggagagttcaagaagttctgtttcaccgtgcgcaagctgatcgggtcaaatgacctgccggagtacgatttgaaggaggaggcggggcaggctggcccgatcctagtcatgcgctaccgcaacctgatcgagggcgaagcatccgccggttcctaatgtacggagcagatgctagggcaaattgccctagcaggggaaaaaggtcgaaaaggtctctttcctgtggatagcacgtacattgggaacccaaagccgtacattgggaaccggaacccgtacattgggaacccaaagccgtacattgggaaccggtcacacatgtaagtgactgatataaaagagaaaaaaggcgatttttccgcctaaaactctttaaaacttattaaaactcttaaaacccgcctggcctgtgcataactgtctggccagcgcacagccgaagagctgcaaaaagcgcctacccttcggtcgctgcgctccctacgccccgccgcttcgcgtcggcctatcgcggccgctggccgctcaaaaatggctggcctacggccaggcaatctaccagggcgcggacaagccgcgccgtcgccactcgaccgccggcgcccacatcaaggcaccctgcctcgcgcgtttcggtgatgacggtgaaaacctctgacacatgcagctcccggagacggtcacagcttgtctgtaagcggatgccgggagcagacaagcccgtcagggcgcgtcagcgggtgttggcgggtgtcggggcgcagccatgacccagtcacgtagcgatagcggagtgtatactggcttaactatgcggcatcagagcagattgtactgagagtgcaccatatgcggtgtgaaataccgcacagatgcgtaaggagaaaataccgcatcaggcgctcttccgcttcctcgctcactgactcgctgcgctcggtcgttcggctgcggcgagcggtatcagctcactcaaaggcggtaatacggttatccacagaatcaggggataacgcaggaaagaacatgtgagcaaaaggccagcaaa

SEQ ID NO: 26 - protein, 1309 aa, synthetic construct
MVSSGEDIFSGLVPILIELEGDVNGHRFSVRGEGYGDASNGKLEIKFICTTGRLPVPWPTLVTTLSYGVQCFAKYPEHMRQNDFFKSAMPDGYVQERTISFKEDGTYKTRAEVKFEGEALVNRIDLKGLEFKEDGNILGHKLEYSFNSHYVYITADKNRNGLEAQFRIRHNVDDGSVQLADHYQQNTPIGEGPVLLPEQHYLTTNSVLSKDPQERRDHMVLVEFVTAAGLSLGMDELYKSGSENLYFQGQLSYGYDEKSTGISVPGPMGPSGPRGLPGPPGAPGPQGFQGPPGEPGEPGASGPMGPRGPPGPPGKNGDDGEAGKPGRPGERGPPGPQGARGLPGTAGLPGMKGHRGFSGLDGAKGDAGPAGPKGEPGSPGENGAPGQMGPRGLPGERGRPGAPGPAGARGNDGATGAAGPPGPTGPAGPPGFPGAVGAKGEGGPQGPRGSEGPQGVRGEPGPPGPAGAAGPAGNPGADGQPGAKGANGAPGIAGAPGFPGARGPSGPQGPSGPPGPKGNSGEPGAPGSKGDTGAKGEPGPTGIQGPPGPAGEEGKRGARGEPGPAGLPGPPGERGGPGSRGFPGADGVAGPKGPAGERGAPGPAGPKGSPGEAGRPGEAGLPGAKGLTGSPGSPGPDGKTGPPGPAGQDGRPGPPGPPGARGQAGVMGFPGPKGAAGEPGKAGERGVPGPPGAVGPAGKDGEAGAQGPPGPAGPAGERGEQGPAGSPGFQGLPGPAGPPGEAGKPGEQGVPGDLGAPGPSGARGERGFPGERGVQGPPGPAGPRGANGAPGNDGAKGDAGAPGAPGSQGAPGLQGMPGERGAAGLPGPKGDRGDAGPKGADGAPGKDGVRGLTGPIGPPGPAGAPGDKGEAGPSGPAGPTGARGAPGDRGEPGPPGPAGFAGPPGADGQPGAKGEPGDAGAKGDAGPPGPAGPAGPPGPIGNVGAPGPKGARGSAGPPGATGFPGAAGRVGPPGPSGNAGPPGPPGPAGKEGSKGPRGETGPAGRPGEVGPPGPPGPAGEKGAPGADGPAGAPGTPGPQGIAGQRGVVGLPGQRGERGFPGLPGPSGEPGKQGPSGASGERGPPGPMGPPGLAGPPGESGREGAPGAEGSPGRDGSPGAKGDRGETGPAGPPGAPGAPGAPGPVGPAGKSGDRGETGPAGPAGPIGPVGARGPAGPQGPRGDKGETGEQGDRGIKGHRGFSGLQGPPGPPGSPGEQGPSGASGPAGPRGPPGSAGSPGKDGLNGLPGPIGPPGPRGRTGDAGPAGPPGPPGPPGPPGPPSGGYDLSFLPQPPQEKAHDGGRYYRAKDEL

SEQ ID NO: 27 - protein, 239 aa, synthetic construct; identical to SEQ ID NO: 17

SEQ ID NO: 28 - protein, 1056 aa, synthetic construct; identical to SEQ ID NO: 2

SEQ ID NO: 29 - DNA, 10736 bp, synthetic construct
  source 1..10736: mol_type = other DNA
  misc_feature 9022..9046: function = plasmid transfer to host cells; note = LB T-DNA repeat
  misc_feature 7128..7716: function = plasmid transfer to host cells; note = RB T-DNA repeat
  regulatory 9137..9311: note = CaMV 35S pA; regulatory_class = polyA_signal_sequence
  misc_feature 9331..9882: note = Bar resistance
  regulatory 9940..10693: note = CaMV35S (enhanced); regulatory_class = promoter
  regulatory 22..775: note = CaMV35S (enhanced); regulatory_class = promoter
  gene 806..2407: gene = Prolyl 4-hydroxylase subunit alpha-1 Protein
  regulatory 2463..2716: note = Nos pA; regulatory_class = terminator; regulatory_class = polyA_signal_sequence
caactttgtatagaaaagttggccaacatggtggagcacgacactctcgtctactccaagaatatcaaagatacagtctcagaagaccaaagggctattgagacttttcaacaaagggtaatatcgggaaacctcctcggattccattgcccagctatctgtcacttcatcaaaaggacagtagaaaaggaaggtggcacctacaaatgccatcattgcgataaaggaaaggctatcgttcaagatgcctctgccgacagtggtcccaaagatggacccccacccacgaggagcatcgtggaaaaagaagacgttccaaccacgtcttcaaagcaagtggattgatgtgaacatggtggagcacgacactctcgtctactccaagaatatcaaagatacagtctcagaagaccaaagggctattgagacttttcaacaaagggtaatatcgggaaacctcctcggattccattgcccagctatctgtcacttcatcaaaaggacagtagaaaaggaaggtggcacctacaaatgccatcattgcgataaaggaaaggctatcgttcaagatgcctctgccgacagtggtcccaaagatggacccccacccacgaggagcatcgtggaaaaagaagacgttccaaccacgtcttcaaagcaagtggattgatgtgatatctccactgacgtaagggatgacgcacaatcccactatccttcgcaagacccttcctctatataaggaagttcatttcatttggagaggacacgctgacaagtttgtacaaaaaagcaggctgccaccatgatttggtatattttggtggttggaattttattgcctcaatctcttgcacaccccggattttttacctctattggacaaatgacggatcttattcatactgaaaaggatttggttactagccttaaagattacattaaagctgaggaggataaacttgaacagattaagaagtgggcagaaaagttggatagacttacctctactgctactaaggatccagagggcttcgtcggacaccctgttaacgcattcaagttaatgaagagattgaacactgaatggtctgaacttgaaaatcttgtgttgaaggacatgtcagatggtttcatttctaatcttacaatacagcgacaatattttccaaacgatgaagatcaagttggcgcagctaaggcacttttgagactccaagatacttataacctcgatactgatacaatttctaaaggtgatttgccaggtgttaagcataagagttttttgactgttgaagattgtttcgagcttggtaaggttgcatatactgaggctgattactatcatactgagttgtggatggaacaagcactgaggcagctagatgagggtgaagtttctacagttgacaaggtttctgttcttgattacctttcttatgctgtttatcaacaaggagatttggataaagctttgcttcttacaaaaaagcttttggaacttgatccagaacaccagagagctaacggtaatctcaaatactttgaatatattatggcaaaagaaaaagatgctaacaagtcttcatctgatgatcaatctgatcaaaagactactcttaagaagaagggtgctgcagttgattatctccctgagagacagaagtatgaaatgctttgtaggggagaaggaattaaaatgacacctagaagacagaagaaacttttttgtaggtatcatgatggtaacaggaatccaaaatttattctcgctcctgctaaacaagaggatgagtgggacaagccaaggatcattcgttttcacgacattatatctgacgctgagatcgaagttgtgaaggatttagctaagcctaggctttcaagagctacagttcatgatccagaaactggaaaattgactactgctcaatacagagtttcaaagtctgcttggctttcaggatatgagaaccctgttgtgtctaggattaatatgagaatccaagatttgactggacttgatgtttcaactgcagaagaattgcaggttgctaactatggtgtgggaggacaatatgagcctcatttcgattttgctcggaaggatgaaccagatgcttttaaagaactcgggactggtaacagaattgccacttggcttttttatatgtcagatgtgcttgctggtggtgctactgtttttcctgaagtgggagcttctgtttggccaaagaaaggtaccgccgtcttttggtataatctttttgcaagtggtgaaggtgactattcaacaaggcatgctgcatgccctgtgttggttggtaataagtgggtgtctaataaatggcttcatgagcgtggccaggaatttagaagaccatgcactctgtcagagcttgaagcttttgtttattagacccagctttcttgtacaaagtggtagctcgaatttccccgatcgttcaaacatttggcaataaagtttcttaagattgaatcctgttgccggtcttgcgatgattatcatataatttctgttgaattacgttaagcatgtaataattaacatgtaatgcatgacgttatttatgagatgggtttttatgattagagtcccgcaattatacatttaatacgcgatagaaaacaaaatatagcgcgcaaactaggataaattatcgcgcgcggtgtcatctatgttactagatcgggaaagcttttaaactatcagtgtttgacaggatatattggcgggtaaacctaagagaaaagagcgtttattagaataatcggatatttaaaagggcgtgaaaaggtttatccgttcgtccatttgtatgtgcatgccaaccacagggttcccctcgggatcaaagtactttgatccaacccctccgctgctatagtgcagtcggcttctgacgttcagtgcagccgtcttctgaaaacgacatgtcgcacaagtcctaagttacgcgacaggctgccgccctgcccttttcctggcgttttcttgtcgcgtgttttagtcgcataaagtagaatacttgcgactagaaccggagacattacgccatgaacaagagcgccgccgctggcctgctgggctatgcccgcgtcagcaccgacgaccaggacttgaccaaccaacgggccgaactgcacgcggccggctgcaccaagctgttttccgagaagatcaccggcaccaggcgcgaccgcccggagctggccaggatgcttgaccacctacgccctggcgacgttgtgacagtgaccaggctagaccgcctggcccgcagcacccgcgacctactggacattgccgagcgcatccaggaggccggcgcgggcctgcgtagcctggcagagccgtgggccgacaccaccacgccggccggccgcatggtgttgaccgtgttcgccggcattgccgagttcgagcgttccctaatcatcgaccgcacccggagcgggcgcgaggccgccaaggcccgaggcgtgaagtttggcccccgccctaccctcaccccggcacagatcgcgcacgcccgcgagctgatcgaccaggaaggccgcaccgtgaaagaggcggctgcactgcttggcgtgcatcgctcgaccctgtaccgcgcacttgagcgcagcgaggaagtgacgcccaccgaggccaggcggcgcggtgccttccgtgaggacgcattgaccgaggccgacgccctggcggccgccgagaatgaacgccaagaggaacaagcatgaaaccgcaccaggacggccaggacgaaccgtttttcattaccgaagagatcgaggcggagatgatcgcggccgggtacgtgttcgagccgcccgcgcacgtctcaaccgtgcggctgcatgaaatcctggccggtttgtctgatgccaagctggcggcctggccggccagcttggccgctgaagaaaccgagcgccgccgtctaaaaaggtgatgtgtatttgagtaaaacagcttgcgtcatgcggtcgctgcgtatatgatgcgatgagtaaataaacaaatacgcaaggggaacgcatgaaggttatcgctgtacttaaccagaaaggcgggtcaggcaagacgaccatcgcaacccatctagcccgcgccctgcaactcgccggggccgatgttctgttagtcgattccgatccccagggcagtgcccgcgattgggcggccgtgcgggaagatcaaccgctaaccgttgtcggcatcgaccgcccgacgattgaccgcgacgtgaaggccatcggccggcgcgacttcgtagtgatcgacggagcgccccaggcggcggacttggctgtgtccgcgatcaaggcagccgacttcgtgctgattccggtgcagccaagcccttacgacatatgggccaccgccgacctggtggagctggttaagcagcgcattgaggtcacggatggaaggctacaagcggcctttgtcgtgtcgcgggcgatcaaaggcacgcgcatcggcggtgaggttgccgaggcgctggccgggtacgagctgcccattcttgagtcccgtatcacgcagcgcgtgagctacccaggcactgccgccgccggcacaaccgttcttgaatcagaacccgagggcgacgctgcccgcgaggtccaggcgctggccgctgaaattaaatcaaaactcatttgagttaatgaggtaaagagaaaatgagcaaaagcacaaacacgctaagtgccggccgtccgagcgcacgcagcagcaaggctgcaacgttggccagcctggcagacacgccagccatgaagcgggtcaactttcagttgccggcggaggatcacaccaagctgaagatgtacgcggtacgccaaggcaagaccattaccgagctgctatctgaatacatcgcgcagctaccagagtaaatgagcaaatgaataaatgagtagatgaattttagcggctaaaggaggcggcatggaaaatcaagaacaaccaggcaccgacgccgtggaatgccccatgtgtggaggaacgggcggttggccaggcgtaagcggctgggttgcctgccggccctgcaatggcactggaacccccaagcccgaggaatcggcgtgagcggtcgcaaaccatccggcccggtacaaatcggcgcggcgctgggtgatgacctggtggagaagttgaaggccgcgcaggccgcccagcggcaacgcatcgaggcagaagcacgccccggtgaatcgtggcaagcggccgctgatcgaatccgcaaagaatcccggcaaccgccggcagccggtgcgccgtcgattaggaagccgcccaagggcgacgagcaaccagattttttcgttccgatgctctatgacgtgggcacccgcgatagtcgcagcatcatggacgtggccgttttccgtctgtcgaagcgtgaccgacgagctggcgaggtgatccgctacgagcttccagacgggcacgtagaggtttccgcagggccggccggcatggccagtgtgtgggattacgacctggtactgatggcggtttcccatctaaccgaatccatgaaccgataccgggaagggaagggagacaagcccggccgcgtgttccgtccacacgttgcggacgtactcaagttctgccggcgagccgatggcggaaagcagaaagacgacctggtagaaacctgcattcggttaaacaccacgcacgttgccatgcagcgtacgaagaaggccaagaacggccgcctggtgacggtatccgagggtgaagccttgattagccgctacaagatcgtaaagagcgaaaccgggcggccggagtacatcgagatcgagctagctgattggatgtaccgcgagatcacagaaggcaagaacccggacgtgctgacggttcaccccgattactttttgatcgatcccggcatcggccgttttctctaccgcctggcacgccgcgccgcaggcaaggcagaagccagatggttgttcaagacgatctacgaacgcagtggcagcgccggagagttcaagaagttctgtttcaccgtgcgcaagctgatcgggtcaaatgacctgccggagtacgatttgaaggaggaggcggggcaggctggcccgatcctagtcatgcgctaccgcaacctgatcgagggcgaagcatccgccggttcctaatgtacggagcagatgctagggcaaattgccctagcaggggaaaaaggtcgaaaaggtctctttcctgtggatagcacgtacattgggaacccaaagccgtacattgggaaccggaacccgtacattgggaacccaaagccgtacattgggaaccggtcacacatgtaagtgactgatataaaagagaaaaaaggcgatttttccgcctaaaactctttaaaacttattaaaactcttaaaacccgcctggcctgtgcataactgtctggccagcgcacagccgaagagctgcaaaaagcgcctacccttcggtcgctgcgctccctacgccccgccgcttcgcgtcggcctatcgcggccgctggccgctcaaaaatggctggcctacggccaggcaatctaccagggcgcggacaagccgcgccgtcgccactcgaccgccggcgcccacatcaaggcaccctgcctcgcgcgtttcggtgatgacggtgaaaacctctgacacatgcagctcccggagacggtcacagcttgtctgtaagcggatgccgggagcagacaagcccgtcagggcgcgtcagcgggtgttggcgggtgtcggggcgcagccatgacccagtcacgtagcgatagcggagtgtatactggcttaactatgcggcatcagagcagattgtactgagagtgcaccatatgcggtgtgaaataccgcacagatgcgtaaggagaaaataccgcatcaggcgctcttccgcttcctcgctcactgactcgctgcgctcggtcgttcggctgcggcgagcggtatcagctcactcaaaggcggtaatacggttatccacagaatcaggggataacgcaggaaagaacatgtgagcaaaaggccagcaaaaggccaggaaccgtaaaaaggccgcgttgctggcgtttttccataggctccgcccccctgacgagcatcacaaaaatcgacgctcaagtcagaggtggcgaaacccgacaggactataaagataccaggcgtttccccctggaagctccctcgtgcgctctcctgttccgaccctgccgcttaccggatacctgtccgcctttctcccttcgggaagcgtggcgctttctcatagctcacgctgtaggtatctcagttcggtgtaggtcgttcgctccaagctgggctgtgtgcacgaaccccccgttcagcccgaccgctgcgccttatccggtaactatcgtcttgagtccaacccggtaagacacgacttatcgccactggcagcagccactggtaacaggattagcagagcgaggtatgtaggcggtgctacagagttcttgaagtggtggcctaactacggctacactagaaggacagtatttggtatctgcgctctgctgaagccagttaccttcggaaaaagagttggtagctcttgatccggcaaacaaaccaccgctggtagcggtggtttttttgtttgcaagcagcagattacgcgcagaaaaaaaggatctcaagaagatcctttgatcttttctacggggtctgacgctcagtggaacgaaaactcacgttaagggattttggtcatgcattctaggtactaaaacaattcatccagtaaaatataatattttattttctcccaatcaggcttgatccccagtaagtcaaaaaatagctcgacatactgttcttccccgatatcctccctgatcgaccggacgcagaaggcaatgtcataccacttgtccgccctgccgcttctcccaagatcaataaagccacttactttgccatctttcacaaagatgttgctgtctcccaggtcgccgtgggaaaagacaagttcctcttcgggcttttccgtctttaaaaaatcatacagctcgcgcggatctttaaatggagtgtcttcttcccagttttcgcaatccacatcggccagatcgttattcagtaagtaatccaattcggctaagcggctgtctaagctattcgtatagggacaatccgatatgtcgatggagtgaaagagcctgatgcactccgcatacagctcgataatcttttcagggctttgttcatcttcatactcttccgagcaaaggacgccatcggcctcactcatgagcagattgctccagccatcatgccgttcaaagtgcaggacctttggaacaggcagctttccttccagccatagcatcatgtccttttcccgttccacatcataggtggtccctttataccggctgtccgtcatttttaaatataggttttcattttctcccaccagcttatataccttagcaggagacattccttccgtatcttttacgcagcggtatttttcgatcagttttttcaattccggtgatattctcattttagccatttattatttccttcctcttttctacagtatttaaagataccccaagaagctaattataacaagacgaactccaattcactgttccttgcattctaaaaccttaaataccagaaaacagctttttcaaagttgttttcaaagttggcgtataacatagtatcgacggagccgattttgaaaccgcggtgatcacaggcagcaacgctctgtcatcgttacaatcaacatgctaccctccgcgagatcatccgtgtttcaaacccggcagcttagttgccgttcttccgaatagcatcggtaacatgagcaaagtctgccgccttacaacggctctcccgctgacgccgtcccggactgatgggctgcctgtatcgagtggtgattttgtgccgagctgccggtcggggagctgttggctggctggtggcaggatatattgtggtgtaaacaaattgacgcttagacaacttaataacacattgcggacgtttttaatgtactgaattaacgccgaattgaattcgagctcggtaccgggggatctggattttagtactggattttggttttaggaattagaaattttattgatagaagtattttacaaatacaaatacatactaagggtttcttatatgctcaacacatgagcgaaaccctataggaaccctaattcccttatctgggaactactcacacattattatggagaaactcgagcttgtcgatcgactcaaatctcggtgacgggcaggaccggacggggcggtaccggcaggctgaagtccagctgccagaaacccacgtcatgccagttcccgtgcttgaagccggccgcccgcagcatgccgcggggggcatatccgagcgcctcgtgcatgcgcacgctcgggtcgttgggcagcccgatgacagcgaccacgctcttgaagccctgtgcctccagggacttcagcaggtgggtgtagagcgtggagcccagtcccgtccgctggtggcggggggagacgtacacggtcgactcggccgtccagtcgtaggcgttgcgtgccttccaggggcccgcgtaggcgatgccggcgacctcgccgtccacctcggcgacgagccagggatagcgctcccgcagacggacgaggtcgtccgtccactcctgcggttcctgcggctcggtacggaagttgaccgtgcttgtctcgatgtagtggttgacgatggtgcagaccgccggcatgtccgcctcggtggcacggcggatgtcggccgggcgtcgttctgggctcatggtagacgatctgcgaaagctcgagagagatagatttgtagagagagactggtgatttcagcgtgtcctctccaaatgaaatgaacttccttatatagaggaagggtcttgcgaaggatagtgggattgtgcgtcatcccttacgtcagtggagatatcacatcaatccacttgctttgaagacgtggttggaacgtcttctttttccacgatgctcctcgtgggtgggggtccatctttgggaccactgtcggcagaggcatcttgaacgatagcctttcctttatcgcaatgatggcatttgtaggtgccaccttccttttctactgtccttttgatgaagtgacagatagctgggcaatggaatccgaggaggtttcccgatattaccctttgttgaaaagtctcaatagccctttggtcttctgagactgtatctttgatattcttggagtagacgagagtgtcgtgctccaccatgttcacatcaatccacttgctttgaagacgtggttggaacgtcttctttttccacgatgctcctcgtgggtgggggtccatctttgggaccactgtcggcagaggcatcttgaacgatagcctttcctttatcgcaatgatggcatttgtaggtgccaccttccttttctactgtccttttgatgaagtgacagatagctgggcaatggaatccgaggaggtttcccgatattaccctttgttgaaaagtctcaatagccctttggtcttctgagactgtatctttgatattcttggagtagacgagagtgtcgtgctccaccatgttggcgtacccggggatcctctagagtcgacctgcaggcatgcaagct

SEQ ID NO: 30 - DNA, 10829 bp, synthetic construct
  source 1..10829: mol_type = other DNA
  misc_feature 9115..9139: function = plasmid transfer to host cells; note = LB T-DNA repeat
  misc_feature 2835..2959: function = plasmid transfer to host cells; note = RB T-DNA repeat
  regulatory 9230..9404: note = CaMV 35S pA; regulatory_class = terminator; regulatory_class = polyA_signal_sequence
  misc_feature 9424..9975: function = Bar resistance
  regulatory 10033..10786: note = CaMV35S(enhanced); regulatory_class = promoter
  regulatory 22..775: note = CaMV35S(enhanced); regulatory_class = promoter
  gene 971..2500: gene = Protein disulfide-isomerase; note = P4Hb
  regulatory 2556..2809: note = Nos pA; regulatory_class = terminator; regulatory_class = polyA_signal_sequence
caactttgtatagaaaagttggccaacatggtggagcacgacactctcgtctactccaagaatatcaaagatacagtctcagaagaccaaagggctattgagacttttcaacaaagggtaatatcgggaaacctcctcggattccattgcccagctatctgtcacttcatcaaaaggacagtagaaaaggaaggtggcacctacaaatgccatcattgcgataaaggaaaggctatcgttcaagatgcctctgccgacagtggtcccaaagatggacccccacccacgaggagcatcgtggaaaaagaagacgttccaaccacgtcttcaaagcaagtggattgatgtgaacatggtggagcacgacactctcgtctactccaagaatatcaaagatacagtctcagaagaccaaagggctattgagacttttcaacaaagggtaatatcgggaaacctcctcggattccattgcccagctatctgtcacttcatcaaaaggacagtagaaaaggaaggtggcacctacaaatgccatcattgcgataaaggaaaggctatcgttcaagatgcctctgccgacagtggtcccaaagatggacccccacccacgaggagcatcgtggaaaaagaagacgttccaaccacgtcttcaaagcaagtggattgatgtgatatctccactgacgtaagggatgacgcacaatcccactatccttcgcaagacccttcctctatataaggaagttcatttcatttggagaggacacgctgacaagtttgtacaaaaaagcaggctgccaccatgagagtacaaagaaggagggctccagatcctccaggtcagtctgaggttgggacaggaggaagggctagaggaggaagaacttataaatctaggaccggaggtgctaggtcaagaggacttcttagctggaggagacagcttaagaggagggtttgcgctgatatgcttagaagggcacttctttgcttggctcttactgctctttttcgtgctggagctggagctccagatgaggaggatcatgttttggttcttcataagggtaatttcgatgaagctcttgcagctcataagtatttgcttgttgagttttatgctccatggtgtgggcactgtaaggcacttgctccagagtacgctaaagctgctggcaaacttaaggccgagggttcagaaattagacttgcaaaggtggatgctacagaggaatcagatttggctcaacagtatggtgttaggggttatcctactatcaagttttttaaaaatggtgatacagcttcaccaaaggaatatacagctggaagggaagctgatgatattgttaattggttgaagaaaagaactggtccagctgcttctacactttcagatggagctgctgctgaagctcttgttgaaagttccgaggttgctgttattggcttttttaaggatatggaatccgattcagctaagcagtttttgttggcagctgaagctattgatgatattccttttggaattacttctaattctgacgttttctctaaataccaattggataaagacggtgtggttcttttcaagaagtttgacgaaggaagaaacaattttgagggtgaggttaccaaggagaagcttcttgattttatcaaacataaccaacttccacttgttattgaatttactgaacaaactgcacctaagatttttggtggagaaattaaaactcatattctccttttcctccctaagagcgttagcgattatgagggtaagctgtcaaattttaagaaggctgcagaatcatttaagggtaagattttgttcatctttatcgattctgatcatactgataatcaaaggattttggagtttttcggtttgaagaaggaagagtgtcctgctgttagacttattactttggaagaggagatgacaaaatataaacctgagtctgatgaacttacagcagagaaaattactgaattttgccacaggtttcttgaaggaaagattaagcctcatttgatgagtcaagaattgcctgacgattgggataaacaacctgttaaggttttggttggtaaaaacttcgaggaggttgcttttgatgagaagaagaacgtgtttgttgaattttatgctccttggtgcggacattgtaagcagcttgctccaatctgggataagttgggagagacctataaagatcatgagaatattgttattgctaaaatggattctactgcaaacgaggttgaggcagttaaggttcatagtttccctactctcaagttttttcctgcttctgctgatagaactgttattgattataatggtgaaagaacactcgatggttttaagaaattccttgaatcaggaggacaagatggtgctggtgacgatgatgatcttgaagatctcgaagaagctgaagagccagatttggaagaagatgatgatcagaaggctgttaaggatgagttggcatttgtgtattaaacccagctttcttgtacaaagtggtagctcgaatttccccgatcgttcaaacatttggcaataaagtttcttaagattgaatcctgttgccggtcttgcgatgattatcatataatttctgttgaattacgttaagcatgtaataattaacatgtaatgcatgacgttatttatgagatgggtttttatgattagagtcccgcaattatacatttaatacgcgatagaaaacaaaatatagcgcgcaaactaggataaattatcgcgcgcggtgtcatctatgttactagatcgggaaagcttttaaactatcagtgtttgacaggatatattggcgggtaaacctaagagaaaagagcgtttattagaataatcggatatttaaaagggcgtgaaaaggtttatccgttcgtccatttgtatgtgcatgccaaccacagggttcccctcgggatcaaagtactttgatccaacccctccgctgctatagtgcagtcggcttctgacgttcagtgcagccgtcttctgaaaacgacatgtcgcacaagtcctaagttacgcgacaggctgccgccctgcccttttcctggcgttttcttgtcgcgtgttttagtcgcataaagtagaatacttgcgactagaaccggagacattacgccatgaacaagagcgccgccgctggcctgctgggctatgcccgcgtcagcaccgacgaccaggacttgaccaaccaacgggccgaactgcacgcggccggctgcaccaagctgttttccgagaagatcaccggcaccaggcgcgaccgcccggagctggccaggatgcttgaccacctacgccctggcgacgttgtgacagtgaccaggctagaccgcctggcccgcagcacccgcgacctactggacattgccgagcgcatccaggaggccggcgcgggcctgcgtagcctggcagagccgtgggccgacaccaccacgccggccggccgcatggtgttgaccgtgttcgccggcattgccgagttcgagcgttccctaatcatcgaccgcacccggagcgggcgcgaggccgccaaggcccgaggcgtgaagtttggcccccgccctaccctcaccccggcacagatcgcgcacgcccgcgagctgatcgaccaggaaggccgcaccgtgaaagaggcggctgcactgcttggcgtgcatcgctcgaccctgtaccgcgcacttgagcgcagcgaggaagtgacgcccaccgaggccaggcggcgcggtgccttccgtgaggacgcattgaccgaggccgacgccctggcggccgccgagaatgaacgccaagaggaacaagcatgaaaccgcaccaggacggccaggacgaaccgtttttcattaccgaagagatcgaggcggagatgatcgcggccgggtacgtgttcgagccgcccgcgcacgtctcaaccgtgcggctgcatgaaatcctggccggtttgtctgatgccaagctggcggcctggccggccagcttggccgctgaagaaaccgagcgccgccgtctaaaaaggtgatgtgtatttgagtaaaacagcttgcgtcatgcggtcgctgcgtatatgatgcgatgagtaaataaacaaatacgcaaggggaacgcatgaaggttatcgctgtacttaaccagaaaggcgggtcaggcaagacgaccatcgcaacccatctagcccgcgccctgcaactcgccggggccgatgttctgttagtcgattccgatccccagggcagtgcccgcgattgggcggccgtgcgggaagatcaaccgctaaccgttgtcggcatcgaccgcccgacgattgaccgcgacgtgaaggccatcggccggcgcgacttcgtagtgatcgacggagcgccccaggcggcggacttggctgtgtccgcgatcaaggcagccgacttcgtgctgattccggtgcagccaagcccttacgacatatgggccaccgccgacctggtggagctggttaagcagcgcattgaggtcacggatggaaggctacaagcggcctttgtcgtgtcgcgggcgatcaaaggcacgcgcatcggcggtgaggttgccgaggcgctggccgggtacgagctgcccattcttgagtcccgtatcacgcagcgcgtgagctacccaggcactgccgccgccggcacaaccgttcttgaatcagaacccgagggcgacgctgcccgcgaggtccaggcgctggccgctgaaattaaatcaaaactcatttgagttaatgaggtaaagagaaaatgagcaaaagcacaaacacgctaagtgccggccgtccgagcgcacgcagcagcaaggctgcaacgttggccagcctggcagacacgccagccatgaagcgggtcaactttcagttgccggcggaggatcacaccaagctgaagatgtacgcggtacgccaaggcaagaccattaccgagctgctatctgaatacatcgcgcagctaccagagtaaatgagcaaatgaataaatgagtagatgaattttagcggctaaaggaggcggcatggaaaatcaagaacaaccaggcaccgacgccgtggaatgccccatgtgtggaggaacgggcggttggccaggcgtaagcggctgggttgcctgccggccctgcaatggcactggaacccccaagcccgaggaatcggcgtgagcggtcgcaaaccatccggcccggtacaaatcggcgcggcgctgggtgatgacctggtggagaagttgaaggccgcgcaggccgcccagcggcaacgcatcgaggcagaagcacgccccggtgaatcgtggcaagcggccgctgatcgaatccgcaaagaatcccggcaaccgccggcagccggtgcgccgtcgattaggaagccgcccaagggcgacgagcaaccagattttttcgttccgatgctctatgacgtgggcacccgcgatagtcgcagcatcatggacgtggccgttttccgtctgtcgaagcgtgaccgacgagctggcgaggtgatccgctacgagcttccagacgggcacgtagaggtttccgcagggccggccggcatggccagtgtgtgggattacgacctggtactgatggcggtttcccatctaaccgaatccatgaaccgataccgggaagggaagggagacaagcccggccgcgtgttccgtccacacgttgcggacgtactcaagttctgccggcgagccgatggcggaaagcagaaagacgacctggtagaaacctgcattcggttaaacaccacgcacgttgccatgcagcgtacgaagaaggccaagaacggccgcctggtgacggtatccgagggtgaagccttgattagccgctacaagatcgtaaagagcgaaaccgggcggccggagtacatcgagatcgagctagctgattggatgtaccgcgagatcacagaaggcaagaacccggacgtgctgacggttcaccccgattactttttgatcgatcccggcatcggccgttttctctaccgcctggcacgccgcgccgcaggcaaggcagaagccagatggttgttcaagacgatctacgaacgcagtggcagcgccggagagttcaagaagttctgtttcaccgtgcgcaagctgatcgggtcaaatgacctgccggagtacgatttgaaggaggaggcggggcaggctggcccgatcctagtcatgcgctaccgcaacctgatcgagggcgaagcatccgccggttcctaatgtacggagcagatgctagggcaaattgccctagcaggggaaaaaggtcgaaaaggtctctttcctgtggatagcacgtacattgggaacccaaagccgtacattgggaaccggaacccgtacattgggaacccaaagccgtacattgggaaccggtcacacatgtaagtgactgatataaaagagaaaaaaggcgatttttccgcctaaaactctttaaaacttattaaaactcttaaaacccgcctggcctgtgcataactgtctggccagcgcacagccgaagagctgcaaaaagcgcctacccttcggtcgctgcgctccctacgccccgccgcttcgcgtcggcctatcgcggccgctggccgctcaaaaatggctggcctacggccaggcaatctaccagggcgcggacaagccgcgccgtcgccactcgaccgccggcgcccacatcaaggcaccctgcctcgcgcgtttcggtgatgacggtgaaaacctctgacacatgcagctcccggagacggtcacagcttgtctgtaagcggatgccgggagcagacaagcccgtcagggcgcgtcagcgggtgttggcgggtgtcggggcgcagccatgacccagtcacgtagcgatagcggagtgtatactggcttaactatgcggcatcagagcagattgtactgagagtgcaccatatgcggtgtgaaataccgcacagatgcgtaaggagaaaataccgcatcaggcgctcttccgcttcctcgctcactgactcgctgcgctcggtcgttcggctgcggcgagcggtatcagctcactcaaaggcggtaatacggttatccacagaatcaggggataacgcaggaaagaacatgtgagcaaaaggccagcaaaaggccaggaaccgtaaaaaggccgcgttgctggcgtttttccataggctccgcccccctgacgagcatcacaaaaatcgacgctcaagtcagaggtggcgaaacccgacaggactataaagataccaggcgtttccccctggaagctccctcgtgcgctctcctgttccgaccctgccgcttaccggatacctgtccgcctttctcccttcgggaagcgtggcgctttctcatagctcacgctgtaggtatctcagttcggtgtaggtcgttcgctccaagctgggctgtgtgcacgaaccccccgttcagcccgaccgctgcgccttatccggtaactatcgtcttgagtccaacccggtaagacacgacttatcgccactggcagcagccactggtaacaggattagcagagcgaggtatgtaggcggtgctacagagttcttgaagtggtggcctaactacggctacactagaaggacagtatttggtatctgcgctctgctgaagccagttaccttcggaaaaagagttggtagctcttgatccggcaaacaaaccaccgctggtagcggtggtttttttgtttgcaagcagcagattacgcgcagaaaaaaaggatctcaagaagatcctttgatcttttctacggggtctgacgctcagtggaacgaaaactcacgttaagggattttggtcatgcattctaggtactaaaacaattcatccagtaaaatataatattttattttctcccaatcaggcttgatccccagtaagtcaaaaaatagctcgacatactgttcttccccgatatcctccctgatcgaccggacgcagaaggcaatgtcataccacttgtccgccctgccgcttctcccaagatcaataaagccacttactttgccatctttcacaaagatgttgctgtctcccaggtcgccgtgggaaaagacaagttcctcttcgggcttttccgtctttaaaaaatcatacagctcgcgcggatctttaaatggagtgtcttcttcccagttttcgcaatccacatcggccagatcgttattcagtaagtaatccaattcggctaagcggctgtctaagctattcgtatagggacaatccgatatgtcgatggagtgaaagagcctgatgcactccgcatacagctcgataatcttttcagggctttgttcatcttcatactcttccgagcaaaggacgccatcggcctcactcatgagcagattgctccagccatcatgccgttcaaagtgcaggacctttggaacaggcagctttccttccagccatagcatcatgtccttttcccgttccacatcataggtggtccctttataccggctgtccgtcatttttaaatataggttttcattttctcccaccagcttatataccttagcaggagacattccttccgtatcttttacgcagcggtatttttcgatcagttttttcaattccggtgatattctcattttagccatttattatttccttcctcttttctacagtatttaaagataccccaagaagctaattataacaagacgaactccaattcactgttccttgcattctaaaaccttaaataccagaaaacagctttttcaaagttgttttcaaagttggcgtataacatagtatcgacggagccgattttgaaaccgcggtgatcacaggcagcaacgctctgtcatcgttacaatcaacatgctaccctccgcgagatcatccgtgtttcaaacccggcagcttagttgccgttcttccgaatagcatcggtaacatgagcaaagtctgccgccttacaacggctctcccgctgacgccgtcccggactgatgggctgcctgtatcgagtggtgattttgtgccgagctgccggtcggggagctgttggctggctggtggcaggatatattgtggtgtaaacaaattgacgcttagacaacttaataacacattgcggacgtttttaatgtactgaattaacgccgaattgaattcgagctcggtaccgggggatctggattttagtactggattttggttttaggaattagaaattttattgatagaagtattttacaaatacaaatacatactaagggtttcttatatgctcaacacatgagcgaaaccctataggaaccctaattcccttatctgggaactactcacacattattatggagaaactcgagcttgtcgatcgactcaaatctcggtgacgggcaggaccggacggggcggtaccggcaggctgaagtccagctgccagaaacccacgtcatgccagttcccgtgcttgaagccggccgcccgcagcatgccgcggggggcatatccgagcgcctcgtgcatgcgcacgctcgggtcgttgggcagcccgatgacagcgaccacgctcttgaagccctgtgcctccagggacttcagcaggtgggtgtagagcgtggagcccagtcccgtccgctggtggcggggggagacgtacacggtcgactcggccgtccagtcgtaggcgttgcgtgccttccaggggcccgcgtaggcgatgccggcgacctcgccgtccacctcggcgacgagccagggatagcgctcccgcagacggacgaggtcgtccgtccactcctgcggttcctgcggctcggtacggaagttgaccgtgcttgtctcgatgtagtggttgacgatggtgcagaccgccggcatgtccgcctcggtggcacggcggatgtcggccgggcgtcgttctgggctcatggtagacgatctgcgaaagctcgagagagatagatttgtagagagagactggtgatttcagcgtgtcctctccaaatgaaatgaacttccttatatagaggaagggtcttgcgaaggatagtgggattgtgcgtcatcccttacgtcagtggagatatcacatcaatccacttgctttgaagacgtggttggaacgtcttctttttccacgatgctcctcgtgggtgggggtccatctttgggaccactgtcggcagaggcatcttgaacgatagcctttcctttatcgcaatgatggcatttgtaggtgccaccttccttttctactgtccttttgatgaagtgacagatagctgggcaatggaatccgaggaggtttcccgatattaccctttgttgaaaagtctcaatagccctttggtcttctgagactgtatctttgatattcttggagtagacgagagtgtcgtgctccaccatgttcacatcaatccacttgctttgaagacgtggttggaacgtcttctttttccacgatgctcctcgtgggtgggggtccatctttgggaccactgtcggcagaggcatcttgaacgatagcctttcctttatcgcaatgatggcatttgtaggtgccaccttccttttctactgtccttttgatgaagtgacagatagctgggcaatggaatccgaggaggtttcccgatattaccctttgttgaaaagtctcaatagccctttggtcttctgagactgtatctttgatattcttggagtagacgagagtgtcgtgctccaccatgttggcgtacccggggatcctctagagtcgacctgcaggcatgcaagct

SEQ ID NO: 31 - DNA, 11458 bp, synthetic construct
  source 1..11458: mol_type = other DNA
  misc_feature 1932..1956: function = plasmid transfer to host cells; note = LB T-DNA repeat
  misc_RNA 2040..2737: function = RNA silencing suppressor; note = p19 Suppressor
  regulatory 2738..3083: note = p35S_short; regulatory_class = promoter
  regulatory 3088..3543: note = pPD7; regulatory_class = promoter
  misc_feature 3525..11458: gene = 35S-His-TEV-Col1a
  misc_feature 3563..3580: note = 6xHis Tag
  misc_feature 3587..3604: note = TEV cleavage site
  gene 3608..6775: gene = Collagen alpha-1(I) chain
  sig_peptide 6776..6787: function = Vacuolar targeting signal
  regulatory 6831..7084: note = Nos pA; regulatory_class = terminator; regulatory_class = polyA_signal_sequence
  misc_feature 7110..7134: function = plasmid transfer to host cells; note = RB T-DNA repeat
aggccaggaaccgtaaaaaggccgcgttgctggcgtttttccataggctccgcccccctgacgagcatcacaaaaatcgacgctcaagtcagaggtggcgaaacccgacaggactataaagataccaggcgtttccccctggaagctccctcgtgcgctctcctgttccgaccctgccgcttaccggatacctgtccgcctttctcccttcgggaagcgtggcgctttctcatagctcacgctgtaggtatctcagttcggtgtaggtcgttcgctccaagctgggctgtgtgcacgaaccccccgttcagcccgaccgctgcgccttatccggtaactatcgtcttgagtccaacccggtaagacacgacttatcgccactggcagcagccactggtaacaggattagcagagcgaggtatgtaggcggtgctacagagttcttgaagtggtggcctaactacggctacactagaaggacagtatttggtatctgcgctctgctgaagccagttaccttcggaaaaagagttggtagctcttgatccggcaaacaaaccaccgctggtagcggtggtttttttgtttgcaagcagcagattacgcgcagaaaaaaaggatctcaagaagatcctttgatcttttctacggggtctgacgctcagtggaacgaaaactcacgttaagggattttggtcatgcattctaggtactaaaacaattcatccagtaaaatataatattttattttctcccaatcaggcttgatccccagtaagtcaaaaaatagctcgacatactgttcttccccgatatcctccctgatcgaccggacgcagaaggcaatgtcataccacttgtccgccctgccgcttctcccaagatcaataaagccacttactttgccatctttcacaaagatgttgctgtctcccaggtcgccgtgggaaaagacaagttcctcttcgggcttttccgtctttaaaaaatcatacagctcgcgcggatctttaaatggagtgtcttcttcccagttttcgcaatccacatcggccagatcgttattcagtaagtaatccaattcggctaagcggctgtctaagctattcgtatagggacaatccgatatgtcgatggagtgaaagagcctgatgcactccgcatacagctcgataatcttttcagggctttgttcatcttcatactcttccgagcaaaggacgccatcggcctcactcatgagcagattgctccagccatcatgccgttcaaagtgcaggacctttggaacaggcagctttccttccagccatagcatcatgtccttttcccgttccacatcataggtggtccctttataccggctgtccgtcatttttaaatataggttttcattttctcccaccagcttatataccttagcaggagacattccttccgtatcttttacgcagcggtatttttcgatcagttttttcaattccggtgatattctcattttagccatttattatttccttcctcttttctacagtatttaaagataccccaagaagctaattataacaagacgaactccaattcactgttccttgcattctaaaaccttaaataccagaaaacagctttttcaaagttgttttcaaagttggcgtataacatagtatcgacggagccgattttgaaaccgcggtgatcacaggcagcaacgctctgtcatcgttacaatcaacatgctaccctccgcgagatcatccgtgtttcaaacccggcagcttagttgccgttcttccgaatagcatcggtaacatgagcaaagtctgccgccttacaacggctctcccgctgacgccgtcccggactgatgggctgcctgtatcgagtggtgattttgtgccgagctgccggtcggggagctgttggctggctggtggcaggatatattgtggtgtaaacaaattgacgcttagacaacttaataacacattgcggacgtttttaatgtactgaattaacgccgaattgaattcgagctcggtggaggatctggattttagtactggattttggttttaggaattagaaattttattgatagaagtattttacaaatacaaatacatactaagggtttcttatatgctcaacacatgagcgaaaccctataggaaccctaattcccttatctgggaactactcacacattattatggagaaactattcactctccttctcaaacgtttctgttccctctggacagccccgactgacgttggactcaacctcaatgggcgctaattgtaatagctcctgtttgcttcttatggccatttcgcaaaggtgttgcagtgttctgctaccaccactcactgtaattgacacacctctgaaacggatggagtaagtgcaaccaatttgatcaaatccaaagaaacgactagcagcgtaatttactgagtcaccagtccaggaacctagaactcgatggagagaggcctctgtccgatcatagcgtaggtagcgtttgaaaactaccttgccaaatccccaggactctttaaatcccagtgggttgtcctggttggagtttgtttcgtcattgtgtaaacgccattctgtccaagatgggctctcatcgggtaacttaaatgggctggtagtgccgccagaaccaccgtcccatctctctgaattggcctgctctcttgcatcattaccctggattgctctctccattgtcctctccaaatgaaatgaacttccttatatagaggaagggtcttgcgaaggatagtgggattgtgcgtcatcccttacgtcagtggagatgtcacatcaatccacttgctttgtagacgtggttggaacctcttctttttccacgatgctcctcgtgggtgggggtccatctttgggaccactgtcggcagagagatcttgaatgatagcctttcctttatcgcaatgatggcatttgtaggagccaccttccttttctactgtcctttcgatgaagtgacagatagctgggcaatggaatccgaggaggtttcccgaaattatcctttgttgaaaagtctcaaacaataggcaaccgtggacttcttcactagctcatcgagatagcaatgccactagctaatttcttacgttgtatcttatttgttttactttggggcatgacatggttaaaccccatcaaagagaaagtgtttcatccactagtcaatatacgaattcattcgaatttatccctgtaaatcctagttcttaggatgaactggtgtaataaacagcaaaaaaaaataaaaaaaaataaatctggaatcattcgaccacctcaataaactaaagctaccaattaccacaatatagtcatccatatccacttagatataaaagataaaagtaaacaaatattaaatttcatatgcacgcataggaaactcatgatcttatcttttaaatagacatctagttttcttaggttataaatagacattttgtcctagaacttcttcactactaaaacctagcctcaaaaagcaggctgccaccatgcatcaccatcatcatcatggatctgagaatttatattttcaaggtcaattgagttatggatacgacgaaaaatcaactggaatatcagtgccaggaccaatgggtccatcaggacctaggggtcttccagggccacctggcgctcctggtcctcagggatttcaaggtcctccaggtgaacctggagagcctggtgcttctggtccaatgggaccaagaggccctcctggtccacctggtaaaaatggtgatgatggtgaggctggaaagcctggtcgtcctggagaaagaggaccaccaggaccacagggagctagaggtttgccaggtacagccggtcttccaggaatgaaaggacacaggggtttttctggtcttgatggtgctaagggagacgcaggacctgctggaccaaagggtgaacctggatctcctggtgaaaatggtgctcctggacaaatgggacctagaggattgcctggcgaaagaggaagacctggtgctcctggaccagctggagctagaggaaatgatggagctactggtgctgccggaccaccaggaccaactggaccagctggaccacctggttttccaggagcagttggggctaagggagaaggtggaccacaaggacctagaggatcagaaggacctcaaggagttaggggagaaccaggtcctcctggtcctgctggagctgctggacccgctggtaacccaggagcagatggacaacctggagcaaaaggggctaatggtgctcctggtattgcaggtgctcctggattccctggtgctagaggaccttcaggacctcagggaccatccggtcctccaggaccaaagggaaactctggtgaaccaggggctcctggatctaagggagatactggagctaagggtgagccaggacctacaggaattcaaggaccaccaggacctgcaggagaggaaggtaagaggggtgctagaggtgaacctggaccagctggattgccaggcccacctggagagaggggtggtccaggttctagaggttttccaggagctgatggagttgctggtccaaagggtcctgctggtgagagaggtgcacctggaccagcaggacctaaaggatcacctggagaagctggtcgtcctggtgaggctggtcttccaggtgctaagggccttacaggatctccaggatcaccaggtccagatggaaagactggaccaccaggtcctgcaggacaagatggaaggcctggtccacctggaccacctggtgctaggggacaagctggtgttatgggattcccaggtccaaagggtgcagctggtgagcctggtaaagctggtgaaagaggagttccaggacctcctggtgctgttggacctgctggtaaagatggtgaagcaggtgctcagggtccaccaggtccagccggtccagctggtgagaggggagagcaaggtcctgctggatctcctggatttcaaggtttgcctggacctgctggacctccaggagaggctggtaaacctggtgagcagggtgtgcctggtgatcttggtgctcctggacctagtggcgcaagaggcgaaaggggatttccaggtgaaagaggagttcagggaccaccaggtccagctggtccaagaggcgctaatggagctccaggaaatgatggagcaaagggtgatgctggcgctccaggagctcctggttctcaaggtgcacctggattgcaaggaatgccaggagagagaggtgcagctggtttgccgggaccaaagggtgatagaggtgatgctggtcctaagggagctgatggagctccaggaaaggatggtgtgagaggattgactggtccaattggaccaccaggtcctgctggagcaccaggagataaaggagaagctggtccttcaggaccagccggtccaactggagctagaggagctccaggagatagaggtgaaccaggaccaccaggacctgctgggtttgcaggtccacctggtgctgatggacaacctggtgctaaaggagaaccaggcgatgctggtgctaagggagatgctggcccacctggtccagctggtcctgctgggccaccaggtcctatcggaaatgttggtgctccagggcctaaaggagctagaggatcagcaggtcccccaggtgctacaggttttccaggggctgctggaagagtgggtcccccaggtccttctgggaatgcaggaccaccaggtcctccaggaccagctggaaaagaaggaagtaagggaccaaggggagaaactggacctgcaggacgtccaggtgaagttggtccacctggacctccaggtccagctggagagaaaggagctccaggagctgatggtccagcaggtgctcctggtactccaggtccacaaggtattgctggtcaaaggggagtggttggtctcccaggtcagagaggtgaaagaggtttcccaggtttgcctggaccatctggagaaccaggtaagcagggcccatctggagcttctggtgagagagggccacctggacctatgggacctcctgggcttgctggacctccaggggaatctggtagggagggtgctccaggtgctgaaggatcacctggtagagatggatcacctggagctaaaggtgatagaggggaaacaggtccagcaggtccacctggcgctcctggtgctccaggagcaccagggccagttggacctgctggaaagtctggagataggggagagactggaccagctggacctgctggaccaatcggtcctgttggcgctagaggtcctgctggaccacaaggtcctaggggagataaaggtgaaacaggtgaacaaggagatagaggaattaaaggtcatagagggttttctggtttgcaaggacctccaggacctcctggatctccaggagagcaaggaccatctggtgcaagcggacctgctggtcctagaggacctccaggttcagctggctcacctggtaaggatggattaaatggtttgcctggaccaataggtccaccaggacctagaggaaggacaggtgatgcaggaccagctggtccacctggtccaccaggaccaccaggaccaccaggtccaccttctggtggatatgatcttagttttcttcctcaacctccccaggagaaagctcatgatggtggtagatattatagggctgcatttgtttattaaacccagctttcttgtacaaagtggtagctcgaatttccccgatcgttcaaacatttggcaataaagtttcttaagattgaatcctgttgccggtcttgcgatgattatcatataatttctgttgaattacgttaagcatgtaataattaacatgtaatgcatgacgttatttatgagatgggtttttatgattagagtcccgcaattatacatttaatacgcgatagaaaacaaaatatagcgcgcaaactaggataaattatcgcgcgcggtgtcatctatgttactagatcgggaaagcttttaaactatcagtgtttgacaggatatattggcgggtaaacctaagagaaaagagcgtttattagaataatcggatatttaaaagggcgtgaaaaggtttatccgttcgtccatttgtatgtgcatgccaaccacagggttcccctcgggatcaaagtactttgatccaacccctccgctgctatagtgcagtcggcttctgacgttcagtgcagccgtcttctgaaaacgacatgtcgcacaagtcctaagttacgcgacaggctgccgccctgcccttttcctggcgttttcttgtcgcgtgttttagtcgcataaagtagaatacttgcgactagaaccggagacattacgccatgaacaagagcgccgccgctggcctgctgggctatgcccgcgtcagcaccgacgaccaggacttgaccaaccaacgggccgaactgcacgcggccggctgcaccaagctgttttccgagaagatcaccggcaccaggcgcgaccgcccggagctggccaggatgcttgaccacctacgccctggcgacgttgtgacagtgaccaggctagaccgcctggcccgcagcacccgcgacctactggacattgccgagcgcatccaggaggccggcgcgggcctgcgtagcctggcagagccgtgggccgacaccaccacgccggccggccgcatggtgttgaccgtgttcgccggcattgccgagttcgagcgttccctaatcatcgaccgcacccggagcgggcgcgaggccgccaaggcccgaggcgtgaagtttggcccccgccctaccctcaccccggcacagatcgcgcacgcccgcgagctgatcgaccaggaaggccgcaccgtgaaagaggcggctgcactgcttggcgtgcatcgctcgaccctgtaccgcgcacttgagcgcagcgaggaagtgacgcccaccgaggccaggcggcgcggtgccttccgtgaggacgcattgaccgaggccgacgccctggcggccgccgagaatgaacgccaagaggaacaagcatgaaaccgcaccaggacggccaggacgaaccgtttttcattaccgaagagatcgaggcggagatgatcgcggccgggtacgtgttcgagccgcccgcgcacgtctcaaccgtgcggctgcatgaaatcctggccggtttgtctgatgccaagctggcggcctggccggccagcttggccgctgaagaaaccgagcgccgccgtctaaaaaggtgatgtgtatttgagtaaaacagcttgcgtcatgcggtcgctgcgtatatgatgcgatgagtaaataaacaaatacgcaaggggaacgcatgaaggttatcgctgtacttaaccagaaaggcgggtcaggcaagacgaccatcgcaacccatctagcccgcgccctgcaactcgccggggccgatgttctgttagtcgattccgatccccagggcagtgcccgcgattgggcggccgtgcgggaagatcaaccgctaaccgttgtcggcatcgaccgcccgacgattgaccgcgacgtgaaggccatcggccggcgcgacttcgtagtgatcgacggagcgccccaggcggcggacttggctgtgtccgcgatcaaggcagccgacttcgtgctgattccggtgcagccaagcccttacgacatatgggccaccgccgacctggtggagctggttaagcagcgcattgaggtcacggatggaaggctacaagcggcctttgtcgtgtcgcgggcgatcaaaggcacgcgcatcggcggtgaggttgccgaggcgctggccgggtacgagctgcccattcttgagtcccgtatcacgcagcgcgtgagctacccaggcactgccgccgccggcacaaccgttcttgaatcagaacccgagggcgacgctgcccgcgaggtccaggcgctggccgctgaaattaaatcaaaactcatttgagttaatgaggtaaagagaaaatgagcaaaagcacaaacacgctaagtgccggccgtccgagcgcacgcagcagcaaggctgcaacgttggccagcctggcagacacgccagccatgaagcgggtcaactttcagttgccggcggaggatcacaccaagctgaagatgtacgcggtacgccaaggcaagaccattaccgagctgctatctgaatacatcgcgcagctaccagagtaaatgagcaaatgaataaatgagtagatgaattttagcggctaaaggaggcggcatggaaaatcaagaacaaccaggcaccgacgccgtggaatgccccatgtgtggaggaacgggcggttggccaggcgtaagcggctgggttgcctgccggccctgcaatggcactggaacccccaagcccgaggaatcggcgtgagcggtcgcaaaccatccggcccggtacaaatcggcgcggcgctgggtgatgacctggtggagaagttgaaggccgcgcaggccgcccagcggcaacgcatcgaggcagaagcacgccccggtgaatcgtggcaagcggccgctgatcgaatccgcaaagaatcccggcaaccgccggcagccggtgcgccgtcgattaggaagccgcccaagggcgacgagcaaccagattttttcgttccgatgctctatgacgtgggcacccgcgatagtcgcagcatcatggacgtggccgttttccgtctgtcgaagcgtgaccgacgagctggcgaggtgatccgctacgagcttccagacgggcacgtagaggtttccgcagggccggccggcatggccagtgtgtgggattacgacctggtactgatggcggtttcccatctaaccgaatccatgaaccgataccgggaagggaagggagacaagcccggccgcgtgttccgtccacacgttgcggacgtactcaagttctgccggcgagccgatggcggaaagcagaaagacgacctggtagaaacctgcattcggttaaacaccacgcacgttgccatgcagcgtacgaagaaggccaagaacggccgcctggtgacggtatccgagggtgaagccttgattagccgctacaagatcgtaaagagcgaaaccgggcggccggagtacatcgagatcgagctagctgattggatgtaccgcgagatcacagaaggcaagaacccggacgtgctgacggttcaccccgattactttttgatcgatcccggcatcggccgttttctctaccgcctggcacgccgcgccgcaggcaaggcagaagccagatggttgttcaagacgatctacgaacgcagtggcagcgccggagagttcaagaagttctgtttcaccgtgcgcaagctgatcgggtcaaatgacctgccggagtacgatttgaaggaggaggcggggcaggctggcccgatcctagtcatgcgctaccgcaacctgatcgagggcgaagcatccgccggttcctaatgtacggagcagatgctagggcaaattgccctagcaggggaaaaaggtcgaaaaggtctctttcctgtggatagcacgtacattgggaacccaaagccgtacattgggaaccggaacccgtacattgggaacccaaagccgtacattgggaaccggtcacacatgtaagtgactgatataaaagagaaaaaaggcgatttttccgcctaaaactctttaaaacttattaaaactcttaaaacccgcctggcctgtgcataactgtctggccagcgcacagccgaagagctgcaaaaagcgcctacccttcggtcgctgcgctccctacgccccgccgcttcgcgtcggcctatcgcggccgctggccgctcaaaaatggctggcctacggccaggcaatctaccagggcgcggacaagccgcgccgtcgccactcgaccgccggcgcccacatcaaggcaccctgcctcgcgcgtttcggtgatgacggtgaaaacctctgacacatgcagctcccggagacggtcacagcttgtctgtaagcggatgccgggagcagacaagcccgtcagggcgcgtcagcgggtgttggcgggtgtcggggcgcagccatgacccagtcacgtagcgatagcggagtgtatactggcttaactatgcggcatcagagcagattgtactgagagtgcaccatatgcggtgtgaaataccgcacagatgcgtaaggagaaaataccgcatcaggcgctcttccgcttcctcgctcactgactcgctgcgctcggtcgttcggctgcggcgagcggtatcagctcactcaaaggcggtaatacggttatccacagaatcaggggataacgcaggaaagaacatgtgagcaaaaggccagcaaa

SEQ ID NO: 32 - DNA, 1326 bp, Arabidopsis thaliana
  source 1..1326: mol_type = genomic DNA
  regulatory 1..1326: note = UBQ10; regulatory_class = promoter
tcgagctgcaggtcaacggatcaggatattcttgtttaagatgttgaactctatggaggtttgtatgaactgatgatctaggaccggataagttcccttcttcatagcgaacttattcaaagaatgttttgtgtatcattcttgttacattgttattaatgaaaaaatattattggtcattggactgaacacgagtgttaaatatggaccaggccccaaataagatccattgatatatgaattaaataacaagaataaatcgagtcaccaaaccacttgccttttttaacgagacttgttcaccaacttgatacaaaagtcattatcctatgcaaatcaataatcatacaaaaatatccaataacactaaaaaattaaaagaaatggataatttcacaatatgttatacgataaagaagttacttttccaagaaattcactgattttataagcccacttgcattagataaatggcaaaaaaaaacaaaaaggaaaagaaataaagcacgaagaattctagaaaatacgaaatacgcttcaatgcagtgggacccacggttcaattattgccaattttcagctccaccgtatatttaaaaaataaaacgataatgctaaaaaaatataaatcgtaacgatcgttaaatctcaacggctggatcttatgacgaccgttagaaattgtggttgtcgacgagtcagtaataaacggcgtcaaagtggttgcagccggcacacacgagtcgtgtttatcaactcaaagcacaaatacttttcctcaacctaaaaataaggcaattagccaaaaacaactttgcgtgtaaacaacgctcaatacacgtgtcattttattattagctattgcttcaccgccttagctttctcgtgacctagtcgtcctcgtcttttcttcttcttcttctataaaacaatacccaaagagctcttcttcttcacaattcagatttcaatttctcaaaatcttaaaaactttctctcaattctctctaccgtgatcaaggtaaatttctgtgttccttattctctcaaaatcttcgattttgttttcgttcgatcccaatttcgtatatgttctttggtttagattctgttaatcttagatcgaacacgattttctgggtttgatcgttagatatcatcttaattctcgattagggtttcatagatatcatccgatttgttcaaataatttgagttttgtcgaataattactcttcgatttgtgatttctatctagatctggtgttagtttctagtttgtgcgatcgaatttgtcgattaatctgagtttttctgattaacagg

SEQ ID NO: 33 - DNA, 8913 bp, synthetic construct
  source 1..8913: mol_type = other DNA
  regulatory 4105..5187: note = Lac repressor; regulatory_class = replication_regulatory_region
  regulatory 5574..5591: note = T7; regulatory_class = promoter
  misc_feature 5597..5613: function = operator; note = LacO
  regulatory 5637..5663: note = T7 translation enhancer RBS; regulatory_class = enhancer
  gene 5662..8913: gene = Col1A1
taaaagggcgagctcagatccggctgctaacaaagcccgaaaggaagctgagttggctgctgccaccgctgagcaataactagcataaccccttggggcctctaaacgggtcttgaggggttttttgctgaaaggaggaactatatccggatatcccgcaagaggcccggcagtaccggcataaccaagcctatgcctacagcatccagggtgacggtgccgaggatgacgatgagcgcattgttagatttcatacacggtgcctgactgcgttagcaatttaactgtgataaactaccgcattaaagctagcttatcgatgataagctgtcaaacatgagaattaattcttgaagacgaaagggcctcgtgatacgcctatttttataggttaatgtcatgataataatggtttcttagacgtcaggtggcacttttcggggaaatgtgcgcggaacccctatttgtttatttttctaaatacattcaaatatgtatccgctcatgagacaataaccctgataaatgcttcaataatattgaaaaaggaagagtatgagtattcaacatttccgtgtcgcccttattcccttttttgcggcattttgccttcctgtttttgctcacccagaaacgctggtgaaagtaaaagatgctgaagatcagttgggtgcacgagtgggttacatcgaactggatctcaacagcggtaagatccttgagagttttcgccccgaagaacgttttccaatgatgagcacttttaaagttctgctatgtggcgcggtattatcccgtgttgacgccgggcaagagcaactcggtcgccgcatacactattctcagaatgacttggttgagtactcaccagtcacagaaaagcatcttacggatggcatgacagtaagagaattatgcagtgctgccataaccatgagtgataacactgcggccaacttacttctgacaacgatcggaggaccgaaggagctaaccgcttttttgcacaacatgggggatcatgtaactcgccttgatcgttgggaaccggagctgaatgaagccataccaaacgacgagcgtgacaccacgatgcctgcagcaatggcaacaacgttgcgcaaactattaactggcgaactacttactctagcttcccggcaacaattaatagactggatggaggcggataaagttgcaggaccacttctgcgctcggcccttccggctggctggtttattgctgataaatctggagccggtgagcgtgggtctcgcggtatcattgcagcactggggccagatggtaagccctcccgtatcgtagttatctacacgacggggagtcaggcaactatggatgaacgaaatagacagatcgctgagataggtgcctcactgattaagcattggtaactgtcagaccaagtttactcatatatactttagattgatttaaaacttcatttttaatttaaaaggatctaggtgaagatcctttttgataatctcatgaccaaaatcccttaacgtgagttttcgttccactgagcgtcagaccccgtagaaaagatcaaaggatcttcttgagatcctttttttctgcgcgtaatctgctgcttgcaaacaaaaaaaccaccgctaccagcggtggtttgtttgccggatcaagagctaccaactctttttccgaaggtaactggcttcagcagagcgcagataccaaatactgtccttctagtgtagccgtagttaggccaccacttcaagaactctgtagcaccgcctacatacctcgctctgctaatcctgttaccagtggctgctgccagtggcgataagtcgtgtcttaccgggttggactcaagacgatagttaccggataaggcgcagcggtcgggctgaacggggggttcgtgcacacagcccagcttggagcgaacgacctacaccgaactgagatacctacagcgtgagctatgagaaagcgccacgcttcccgaagggagaaaggcggacaggtatccggtaagcggcagggtcggaacaggagagcgcacgagggagcttccagggggaaacgcctggtatctttatagtcctgtcgggtttcgccacctctgacttgagcgtcgatttttgtgatgctcgtcaggggggcggagcctatggaaaaacgccagcaacgcggcctttttacggttcctggccttttgctggccttttgctcacatgttctttcctgcgttatcccctgattctgtggataaccgtattaccgcctttgagtgagctgataccgctcgccgcagccgaacgaccgagcgcagcgagtcagtgagcgaggaagcggaagagcgcctgatgcggtattttctccttacgcatctgtgcggtatttcacaccgcaatggtgcactctcagtacaatctgctctgatgccgcatagttaagccagtatacactccgctatcgctacgtgactgggtcatggctgcgccccgacacccgccaacacccgctgacgcgccctgacgggcttgtctgctcccggcatccgcttacagacaagctgtgaccgtctccgggagctgcatgtgtcagaggttttcaccgtcatcaccgaaacgcgcgaggcagctgcggtaaagctcatcagcgtggtcgtgaagcgattcacagatgtctgcctgttcatccgcgtccagctcgttgagtttctccagaagcgttaatgtctggcttctgataaagcgggccatgttaagggcggttttttcctgtttggtcactgatgcctccgtgtaagggggatttctgttcatgggggtaatgataccgatgaaacgagagaggatgctcacgatacgggttactgatgatgaacatgcccggttactggaacgttgtgagggtaaacaactggcggtatggatgcggcgggaccagagaaaaatcactcagggtcaatgccagcgcttcgttaatacagatgtaggtgttccacagggtagccagcagcatcctgcgatgcagatccggaacataatggtgcagggcgctgacttccgcgtttccagactttacgaaacacggaaaccgaagaccattcatgttgttgctcaggtcgcagacgttttgcagcagcagtcgcttcacgttcgctcgcgtatcggtgattcattctgctaaccagtaaggcaaccccgccagcctagccgggtcctcaacgacaggagcacgatcatgcgcacccgtggccaggacccaacgctgcccgagatgcgccgcgtgcggctgctggagatggcggacgcgatggatatgttctgccaagggttggtttgcgcattcacagttctccgcaagaattgattggctccaattcttggagtggtgaatccgttagcgaggtgccgccggcttccattcaggtcgaggtggcccggctccatgcaccgcgacgcaacgcggggaggcagacaaggtatagggcggcgcctacaatccatgccaacccgttccatgtgctcgccgaggcggcataaatcgccgtgacgatcagcggtccaatgatcgaagttaggctggtaagagccgcgagcgatccttgaagctgtccctgatggtcgtcatctacctgcctggacagcatggcctgcaacgcgggcatcccgatgccgccggaagcgagaagaatcataatggggaaggccatccagcctcgcgtcgcgaacgccagcaagacgtagcccagcgcgtcggccgccatgccggcgataatggcctgcttctcgccgaaacgtttggtggcgggaccagtgacgaaggcttgagcgagggcgtgcaagattccgaataccgcaagcgacaggccgatcatcgtcgcgctccagcgaaagcggtcctcgccgaaaatgacccagagcgctgccggcacctgtcctacgagttgcatgataaagaagacagtcataagtgcggcgacgatagtcatgccccgcgcccaccggaaggagctgactgggttgaaggctctcaagggcatcggtcgagatcccggtgcctaatgagtgagctaacttacattaattgcgttgcgctcactgcccgctttccagtcgggaaacctgtcgtgccagctgcattaatgaatcggccaacgcgcggggagaggcggtttgcgtattgggcgccagggtggtttttcttttcaccagtgagacgggcaacagctgattgcccttcaccgcctggccctgagagagttgcagcaagcggtccacgctggtttgccccagcaggcgaaaatcctgtttgatggtggttaacggcgggatataacatgagctgtcttcggtatcgtcgtatcccactaccgagatatccgcaccaacgcgcagcccggactcggtaatggcgcgcattgcgcccagcgccatctgatcgttggcaaccagcatcgcagtgggaacgatgccctcattcagcatttgcatggtttgttgaaaaccggacatggcactccagtcgccttcccgttccgctatcggctgaatttgattgcgagtgagatatttatgccagccagccagacgcagacgcgccgagacagaacttaatgggcccgctaacagcgcgatttgctggtgacccaatgcgaccagatgctccacgcccagtcgcgtaccgtcttcatgggagaaaataatactgttgatgggtgtctggtcagagacatcaagaaataacgccggaacattagtgcaggcagcttccacagcaatggcatcctggtcatccagcggatagttaatgatcagcccactgacgcgttgcgcgagaagattgtgcaccgccgctttacaggcttcgacgccgcttcgttctaccatcgacaccaccacgctggcacccagttgatcggcgcgagatttaatcgccgcgacaatttgcgacggcgcgtgcagggccagactggaggtggcaacgccaatcagcaacgactgtttgcccgccagttgttgtgccacgcggttgggaatgtaattcagctccgccatcgccgcttccactttttcccgcgttttcgcagaaacgtggctggcctggttcaccacgcgggaaacggtctgataagagacaccggcatactctgcgacatcgtataacgttactggtttcacattcaccaccctgaattgactctcttccgggcgctatcatgccataccgcgaaaggttttgcgccattcgatggtgtccgggatctcgacgctctcccttatgcgactcctgcattaggaagcagcccagtagtaggttgaggccgttgagcaccgccgccgcaaggaatggtgcatgcaaggagatggcgcccaacagtcccccggccacggggcctgccaccatacccacgccgaaacaagcgctcatgagcccgaagtggcgagcccgatcttccccatcggtgatgtcggcgatataggcgccagcaaccgcacctgtggcgccggtgatgccggccacgatgcgtccggcgtagaggatcgagatctcgatcccgcgaaattaatacgactcactataggggaattgtgagcggataacaattcccctctagaaataattttgtttaactttaagaaggagatatacatatgcatcatcaccatcaccatggtaagcctatccctaaccctctcctcggtctcgattctacggaaaacctgtattttcagggacaattgagttatggatacgacgaaaaatcaactggaatatcagtgccaggaccaatgggtccatcaggacctaggggtcttccagggccacctggcgctcctggtcctcagggatttcaaggtcctccaggtgaacctggagagcctggtgcttctggtccaatgggaccaagaggccctcctggtccacctggtaaaaatggtgatgatggtgaggctggaaagcctggtcgtcctggagaaagaggaccaccaggaccacagggagctagaggtttgccaggtacagccggtcttccaggaatgaaaggacacaggggtttttctggtcttgatggtgctaagggagacgcaggacctgctggaccaaagggtgaacctggatctcctggtgaaaatggtgctcctggacaaatgggacctagaggattgcctggcgaaagaggaagacctggtgctcctggaccagctggagctagaggaaatgatggagctactggtgctgccggaccaccaggaccaactggaccagctggaccacctggttttccaggagcagttggggctaagggagaaggtggaccacaaggacctagaggatcagaaggacctcaaggagttaggggagaaccaggtcctcctggtcctgctggagctgctggacccgctggtaacccaggagcagatggacaacctggagcaaaaggggctaatggtgctcctggtattgcaggtgctcctggattccctggtgctagaggaccttcaggacctcagggaccatccggtcctccaggaccaaagggaaactctggtgaaccaggggctcctggatctaagggagatactggagctaagggtgagccaggacctacaggaattcaaggaccaccaggacctgcaggagaggaaggtaagaggggtgctagaggtgaacctggaccagctggattgccaggcccacctggagagaggggtggtccaggttctagaggttttccaggagctgatggagttgctggtccaaagggtcctgctggtgagagaggtgcacctggaccagcaggacctaaaggatcacctggagaagctggtcgtcctggtgaggctggtcttccaggtgctaagggccttacaggatctccaggatcaccaggtccagatggaaagactggaccaccaggtcctgcaggacaagatggaaggcctggtccacctggaccacctggtgctaggggacaagctggtgttatgggattcccaggtccaaagggtgcagctggtgagcctggtaaagctggtgaaagaggagttccaggacctcctggtgctgttggacctgctggtaaagatggtgaagcaggtgctcagggtccaccaggtccagccggtccagctggtgagaggggagagcaaggtcctgctggatctcctggatttcaaggtttgcctggacctgctggacctccaggagaggctggtaaacctggtgagcagggtgtgcctggtgatcttggtgctcctggacctagtggcgcaagaggcgaaaggggatttccaggtgaaagaggagttcagggaccaccaggtccagctggtccaagaggcgctaatggagctccaggaaatgatggagcaaagggtgatgctggcgctccaggagctcctggttctcaaggtgcacctggattgcaaggaatgccaggagagagaggtgcagctggtttgccgggaccaaagggtgatagaggtgatgctggtcctaagggagctgatggagctccaggaaaggatggtgtgagaggattgactggtccaattggaccaccaggtcctgctggagcaccaggagataaaggagaagctggtccttcaggaccagccggtccaactggagctagaggagctccaggagatagaggtgaaccaggaccaccaggacctgctgggtttgcaggtccacctggtgctgatggacaacctggtgctaaaggagaaccaggcgatgctggtgctaagggagatgctggcccacctggtccagctggtcctgctgggccaccaggtcctatcggaaatgttggtgctccagggcctaaaggagctagaggatcagcaggtcccccaggtgctacaggttttccaggggctgctggaagagtgggtcccccaggtccttctgggaatgcaggaccaccaggtcctccaggaccagctggaaaagaaggaagtaagggaccaaggggagaaactggacctgcaggacgtccaggtgaagttggtccacctggacctccaggtccagctggagagaaaggagctccaggagctgatggtccagcaggtgctcctggtactccaggtccacaaggtattgctggtcaaaggggagtggttggtctcccaggtcagagaggtgaaagaggtttcccaggtttgcctggaccatctggagaaccaggtaagcagggcccatctggagcttctggtgagagagggccacctggacctatgggacctcctgggcttgctggacctccaggggaatctggtagggagggtgctccaggtgctgaaggatcacctggtagagatggatcacctggagctaaaggtgatagaggggaaacaggtccagcaggtccacctggcgctcctggtgctccaggagcaccagggccagttggacctgctggaaagtctggagataggggagagactggaccagctggacctgctggaccaatcggtcctgttggcgctagaggtcctgctggaccacaaggtcctaggggagataaaggtgaaacaggtgaacaaggagatagaggaattaaaggtcatagagggttttctggtttgcaaggacctccaggacctcctggatctccaggagagcaaggaccatctggtgcaagcggacctgctggtcctagaggacctccaggttcagctggctcacctggtaaggatggattaaatggtttgcctggaccaataggtccaccaggacctagaggaaggacaggtgatgcaggaccagctggtccacctggtccaccaggaccaccaggaccaccaggtccaccttctggtggatatgatcttagttttcttcctcaacctccccaggagaaagctcatgatggtggtagatattatagggct

SEQ ID NO: 34 - DNA, 6748 bp, synthetic construct
  source 1..6748: mol_type = other DNA
  regulatory 22..962: note = AOX1; regulatory_class = promoter
  gene 993..4469: gene = Col1A1 without propeptides
  regulatory 4502..4830: note = AOX1 TT; regulatory_class = promoter
caactttgtatagaaaagttgagatctaacatccaaagacgaaaggttgaatgaaacctttttgccatccgacatccacaggtccattctcacacataagtgccaaacgcaacaggaggggatacactagcagcagaccgttgcaaacgcaggacctccactcctcttctcctcaacacccacttttgccatcgaaaaaccagcccagttattgggcttgattggagctcgctcattccaattccttctattaggctactaacaccatgactttattagcctgtctatcctggcccccctggcgaggttcatgtttgtttatttccgaatgcaacaagctccgcattacacccgaacatcactccagatgagggctttctgagtgtggggtcaaatagtttcatgttccccaaatggcccaaaactgacagtttaaacgctgtcttggaacctaatatgacaaaagcgtgatctcatccaagatgaactaagtttggttcgttgaaatgctaacggccagttggtcaaaaagaaacttccaaaagtcggcataccgtttgtcttgtttggtattgattgacgaatgctcaaaaataatctcattaatgcttagcgcagtctctctatcgcttctgaaccccggtgcacctgtgccgaaacgcaaatggggaaacacccgctttttggatgattatgcattgtctccacattgtatgcttccaagattctggtgggaatactgctgatagcctaacgttcatgatcaaaatttaactgttctaacccctacttgacagcaatatataaacagaaggaagctgccctgtcttaaacctttttttttatcatcattattagcttactttcataattgcgactggttccaattgacaagcttttgattttaacgacttttaacgacaacttgagaagatcaaaaaacaactaattattcgaaacgacaagtttgtacaaaaaagcaggctgccaccatgagatttccttcaatttttactgctgttttattcgcagcatcctccgcattagctgctccagtcaacactacaacagaagatgaaacggcacaaattccggctgaagctgtcatcggttactcagatttagaaggggatttcgatgttgctgttttgccattttccaacagcacaaataacgggttattgtttataaatactactattgccagcattgctgctaaagaagaaggggtatctctcgagaaaagagaggctgaagctcatcaccatcaccatcacgaaaacctgtattttcagggccaattgtcttatggttacgatgaaaagtccactggtatttctgtccctggaccaatgggtccatcaggtcctagaggtttgccaggtcctccaggtgctccaggtccacaaggttttcaaggtccaccaggtgaaccaggagaacccggtgcttctggtccaatgggtccaagaggtccacctggacctcctggtaagaacggtgatgatggtgaggctggtaagccaggaagacctggagaaagaggaccacctggtccacaaggagctagaggtttacccggtacagctggtttgcctggtatgaagggtcatagaggtttctccggtttggatggagctaagggtgatgctggacctgctggtcctaagggagagccaggatctccaggtgagaacggagctcctggacaaatgggaccaagaggtctgcctggtgaaagaggtagaccaggtgctcctggtcctgccggagccagaggtaatgatggtgctactggtgctgctggtcctccaggtccaactggtcctgctggtcctccaggttttccaggtgctgttggagccaaaggtgaaggtggcccacaaggtcctagaggatctgaaggtccacagggtgttagaggtgaaccaggtccaccaggtccagctggagctgctggtcctgctggtaacccaggtgcagatggtcaaccaggtgctaagggtgccaacggtgctccaggcattgctggagctccaggttttccaggagctagaggtccttctggacctcaaggaccatctggtccacctggaccaaaaggtaactctggagaaccaggtgctcctggttccaaaggtgataccggtgctaaaggagagccaggtcctactggtattcaaggtcctcctggtcctgctggtgaagagggtaaaagaggagccagaggtgaacctggtccagccggtttgccaggtccaccaggtgaaagaggaggtccaggatctagaggttttccaggtgctgacggtgttgctggtccaaagggtcctgctggtgagagaggagccccaggtccagctggacctaaaggatctccaggagaagctggtcgtcctggtgaagctggtcttccaggtgctaagggtttgacaggctccccaggatcccctggtccagatggtaagactggaccacctggaccagctggtcaagatggaagaccaggtcctccaggaccacctggagccagaggccaagctggtgttatgggtttccctggtccaaaaggtgctgctggagaaccgggtaaagccggtgaaagaggtgttccaggtcctccaggtgctgttggtcctgctggtaaagatggagaagccggtgctcaaggaccaccaggtccagctggtccagctggagagagaggtgaacaaggtcctgctggatccccaggtttccaaggtttgcctggtcctgctggaccaccaggtgaagctggtaagccaggtgaacaaggagttccaggtgatttgggtgctcctggtccatccggtgctagaggtgaaagaggatttccaggagagagaggtgttcaaggaccacctggtcctgctggaccaagaggagcaaacggtgctccaggaaacgatggtgctaaaggtgatgctggtgctccaggagctccaggttcacaaggtgctccaggtttgcaaggaatgcctggagaaagaggtgctgctggattaccaggtccaaaaggagacagaggtgatgccggtccaaagggtgctgatggtgctccaggtaaggacggtgtgcgaggtttgactggaccaattggacctccaggtccagctggagccccaggagataagggtgaagctggtccatcgggtcctgctggtcctactggtgctagaggagctccaggagatagaggtgaacctggtccacctggacccgctggatttgctggtccaccaggtgctgatggtcaaccaggggctaaaggtgaaccaggtgacgctggagctaaaggagatgccggtccaccaggtccagccggtccagctggtcctcctggtccaattggtaatgttggcgctcctggtcctaagggtgccagaggttcagctggaccaccaggtgctactggtttcccaggtgctgccggtagagttggtccaccaggtccatctggtaacgctggtcctccaggtccaccaggtcctgctggaaaggagggatctaagggaccaagaggtgaaactggtccagctggaagacctggtgaagttggtcctccaggaccaccaggtcctgctggagaaaaaggtgctccaggtgctgatggaccagctggtgctcctggtaccccaggtccacaaggtattgctggtcaaagaggtgtggttggtcttcctggacaaagaggtgagagaggttttcctggtttgccaggtccttctggagaacctggaaaacagggtccctctggtgcttctggtgagagaggtcctccaggaccaatgggacctccaggtttggctggtccaccaggtgagtctggtagagagggtgctccaggtgctgagggttctccaggtagagatggtagtccaggtgctaaaggagacagaggagagactggtccagctggtcctccaggtgctcctggtgctcccggtgctcctggtcctgtcggtcctgctggaaagtctggtgatagaggtgagactggtccagctggaccagctggtccaatcggaccagttggagctagaggtcctgctggtcctcaaggtccaagaggtgacaagggtgaaacaggtgagcaaggtgacagaggtattaaaggacatagaggtttctctggtctacagggacctcctggtcctccaggttccccaggtgagcaaggtccttctggtgcttcaggtcctgctggtccaagaggtccaccaggttctgctggttctccaggaaaggatggtttgaatggtttgcctggacctattggtcctcctggacctagaggtagaacaggtgatgctggtcctgctggtccacctggtcctcctggtcctcctggtccccctggacctccatctggaggttacgatttgtcttttttgccacaacctccacaggaaaaagcccatgacggtggaagatattatagagcttaaacccagctttcttgtacaaagtggtgtttgtagccttagacatgactgttcctcagttcaagttgggcacttacgagaagaccggtcttgctagattctaatcaagaggatgtcagaatgccatttgcctgagagatgcaggcttcatttttgatacttttttatttgtaacctatatagtataggattttttttgtcattttgtttcttctcgtacgagcttgctcctgatcagcctatctcgcagctgatgaatatcttgtggtaggggtttgggaaaatcattcgagtttgatgtttttcttggtatttcccactcctcttcagagtacagaagattaagtgagaccttcgtttgtgcggatcccccacacaccatagcttcaaaatgtttctactccttttttactcttccagattttctcggactccgcgcatcgccgtaccacttcaaaacacccaagcacagcatactaaattccccctctttcttcctctagggtgtcgttaattacccgtactaaaggtttggaaaagaaaaaagagaccgcctcgtttctttttcttcgtcgaaaaaggcaataaaaatttttatcacgtttctttttcttgaaaatttttttttttgatttttttctctttcgatgacctcccattgatatttaagttaataaatggtcttcaatttctcaagtttcagtttcatttttcttgttctattacaactttttttacttcttgctcattagaaagaaagcatagcaatctaatctaagggcggtgttgacaattaatcatcggcatagtatatcggcatagtataatacgacaaggtgaggaactaaaccatggccaagttgaccagtgccgttccggtgctcaccgcgcgcgacgtcgccggagcggtcgagttctggaccgaccggctcgggttctcccgggacttcgtggaggacgacttcgccggtgtggtccgggacgacgtgaccctgttcatcagcgcggtccaggaccaggtggtgccggacaacaccctggcctgggtgtgggtgcgcggcctggacgagctgtacgccgagtggtcggaggtcgtgtccacgaacttccgggacgcctccgggccggccatgaccgagatcggcgagcagccgtgggggcgggagttcgccctgcgcgacccggccggcaactgcgtgcacttcgtggccgaggagcaggactgacacgtccgacgcggcccgacgggtccgaggcctcggagatccgtcccccttttcctttgtcgatatcatgtaattagttatgtcacgcttacattcacgccctccccccacatccgctctaaccgaaaaggaaggagttagacaacctgaagtctaggtccctatttatttttttatagttatgttagtattaagaacgttatttatatttcaaatttttcttttttttctgtacagacgcgtgtacgcatgtaacattatactgaaaaccttgcttgagaaggttttgggacgctcgaaggctttaatttgcaagctggagaccaacatgtgagcaaaaggccagcaaaaggccaggaaccgtaaaaaggccgcgttgctggcgtttttccataggctccgcccccctgacgagcatcacaaaaatcgacgctcaagtcagaggtggcgaaacccgacaggactataaagataccaggcgtttccccctggaagctccctcgtgcgctctcctgttccgaccctgccgcttaccggatacctgtccgcctttctcccttcgggaagcgtggcgctttctcatagctcacgctgtaggtatctcagttcggtgtaggtcgttcgctccaagctgggctgtgtgcacgaaccccccgttcagcccgaccgctgcgccttatccggtaactatcgtcttgagtccaacccggtaagacacgacttatcgccactggcagcagccactggtaacaggattagcagagcgaggtatgtaggcggtgctacagagttcttgaagtggtggcctaactacggctacactagaagaacagtatttggtatctgcgctctgctgaagccagttaccttcggaaaaagagttggtagctcttgatccggcaaacaaaccaccgctggtagcggtggtttttttgtttgcaagcagcagattacgcgcagaaaaaaaggatctcaagaagatcctttgatcttttctacggggtctgacgctcagtggaacgaaaactcacgttaagggattttggtcatgagatc